European Patent Application EP 4 541 824 A1, published April 23, 2025. Title: Linker peptide, FVIII Protein or variant thereof containing linker peptide, and use thereof. Applicant: Shenzhen Syno Minicircle Biotechnology Co., Ltd. Application CN PCT/CN2023/104477, filed June 30, 2023. The sequence listing filed with the application follows.

SEQUENCE LISTING (62 sequences)

SEQ ID NO: 1 - protein, 72 aa, synthetic construct
SFSQNSRHPSTRQKQFNATNVSNNSNTSNDSNVSNKTSNNSNATNKTNNTNDSTNRTNQTNTSPPVLKRHQR

SEQ ID NO: 2 - protein, 74 aa, synthetic construct
SFSQNSRHPSTRQKQFNATNVSNNSNTSNDSNVSNKTSNNSNATNKTNNTNDSTNRTNQTNTSQQNFVTQRSKR

SEQ ID NO: 3 - DNA, 216 bp, synthetic construct
  source 1..216: mol_type = other DNA
agcttcagccagaatagcagacaccctagcaccagacagaaacagtttaatgccactaatgtgagcaacaacagcaacaccagcaatgacagcaatgtgtctaacaagacatctaacaacagcaatgccacaaacaagaccaacaacacaaatgatagcacaaacaggaccaaccagaccaataccagcccccctgtgctgaagagacatcagagg

SEQ ID NO: 4 - DNA, 222 bp, synthetic construct
  source 1..222: mol_type = other DNA
agcttcagccagaattctagacaccctagcaccagacagaaacagtttaatgccactaatgtgtctaacaacagcaacaccagcaatgacagcaatgtgtctaacaagacatctaacaacagcaacgccacaaacaagaccaacaacacaaatgatagcacaaaccggaccaaccagaccaataccagccagcagaacttcgtgacccagagaagtaagaga

SEQ ID NO: 5 - protein, 1496 aa, synthetic construct
ATRRYYLGAVELSWDYMQSDLGELPVDARFPPRVPKSFPFNTSVVYKKTLFVEFTDHLFNIAKPRPPWMGLLGPTIQAEVYDTVVITLKNMASHPVSLHAVGVSYWKASEGAEYDDQTSQREKEDDKVFPGGSHTYVWQVLKENGPMASDPLCLTYSYLSHVDLVKDLNSGLIGALLVCREGSLAKEKTQTLHKFILLFAVFDEGKSWHSETKNSLMQDRDAASARAWPKMHTVNGYVNRSLPGLIGCHRKSVYWHVIGMGTTPEVHSIFLEGHTFLVRNHRQASLEISPITFLTAQTLLMDLGQFLLFCHISSHQHDGMEAYVKVDSCPEEPQLRMKNNEEAEDYDDDLTDSEMDVVRFDDDNSPSFIQIRSVAKKHPKTWVHYIAAEEEDWDYAPLVLAPDDRSYKSQYLNNGPQRIGRKYKKVRFMAYTDETFKTREAIQHESGILGPLLYGEVGDTLLIIFKNQASRPYNIYPHGITDVRPLYSRRLPKGVKHLKDFPILPGEIFKYKWTVTVEDGPTKSDPRCLTRYYSSFVNMERDLASGLIGPLLICYKESVDQRGNQIMSDKRNVILFSVFDENRSWYLTENIQRFLPNPAGVQLEDPEFQASNIMHSINGYVFDSLQLSVCLHEVAYWYILSIGAQTDFLSVFFSGYTFKHKMVYEDTLTLFPFSGETVFMSMENPGLWILGCHNSDFRNRGMTALLKVSSCDKNTGDYYEDSYEDISAYLLSKNNAIEPRSFSQNSRHPSTRQKQFNATNVSNNSNTSNDSNVSNKTSNNSNATNKTNNTNDSTNRTNQTNTSPPVLKRHQREITRTTLQSDQEEIDYDDTISVEMKKEDFDIYDEDENQSPRSFQKKTRHYFIAAVERLWDYGMSSSPHVLRNRAQSGSVPQFKKVVFQEFTDGSFTQPLYRGELNEHLGLLGPYIRAEVEDNIMVTFRNQASRPYSFYSSLISYEEDQRQGAEPRKNFVKPNETKTYFWKVQHHMAPTKDEFDCKAWAYFSDVDLEKDVHSGLIGPLLVCHTNTLNPAHGRQVTVQEFALFFTIFDETKSWYFTENMERNCRAPCNIQMEDPTFKENYRFHAINGYIMDTLPGLVMAQDQRIRWYLLSMGSNENIHSIHFSGHVFTVRKKEEYKMALYNLYPGVFETVEMLPSKAGIWRVECLIGEHLHAGMSTLFLVYSNKCQTPLGMASGHIRDFQITASGQYGQWAPKLARLHYSGSINAWSTKEPFSWIKVDLLAPMIIHGIKTQGARQKFSSLYISQFIIMYSLDGKKWQTYRGNSTGTLMVFFGNVDSSGIKHNIFNPPIIARYIRLHPTHYSIRSTLRMELMGCDLNSCSMPLGMESKAISDAQITASSYFTNMFATWSPSKARLHLQGRSNAWRPQVNNPKEWLQVDFQKTMKVTGVTTQGVKSLLTSMYVKEFLISSSQDGHQWTLFFQNGKVKVFQGNQDSFTPVVNSLDPPLLTRYLRIHPQSWVHQIALRMEVLGCEAQDLY

SEQ ID NO: 6 - protein, 1498 aa, synthetic construct
ATRRYYLGAVELSWDYMQSDLGELPVDARFPPRVPKSFPFNTSVVYKKTLFVEFTDHLFNIAKPRPPWMGLLGPTIQAEVYDTVVITLKNMASHPVSLHAVGVSYWKASEGAEYDDQTSQREKEDDKVFPGGSHTYVWQVLKENGPMASDPLCLTYSYLSHVDLVKDLNSGLIGALLVCREGSLAKEKTQTLHKFILLFAVFDEGKSWHSETKNSLMQDRDAASARAWPKMHTVNGYVNRSLPGLIGCHRKSVYWHVIGMGTTPEVHSIFLEGHTFLVRNHRQASLEISPITFLTAQTLLMDLGQFLLFCHISSHQHDGMEAYVKVDSCPEEPQLRMKNNEEAEDYDDDLTDSEMDVVRFDDDNSPSFIQIRSVAKKHPKTWVHYIAAEEEDWDYAPLVLAPDDRSYKSQYLNNGPQRIGRKYKKVRFMAYTDETFKTREAIQHESGILGPLLYGEVGDTLLIIFKNQASRPYNIYPHGITDVRPLYSRRLPKGVKHLKDFPILPGEIFKYKWTVTVEDGPTKSDPRCLTRYYSSFVNMERDLASGLIGPLLICYKESVDQRGNQIMSDKRNVILFSVFDENRSWYLTENIQRFLPNPAGVQLEDPEFQASNIMHSINGYVFDSLQLSVCLHEVAYWYILSIGAQTDFLSVFFSGYTFKHKMVYEDTLTLFPFSGETVFMSMENPGLWILGCHNSDFRNRGMTALLKVSSCDKNTGDYYEDSYEDISAYLLSKNNAIEPRSFSQNSRHPSTRQKQFNATNVSNNSNTSNDSNVSNKTSNNSNATNKTNNTNDSTNRTNQTNTSQQNFVTQRSKREITRTTLQSDQEEIDYDDTISVEMKKEDFDIYDEDENQSPRSFQKKTRHYFIAAVERLWDYGMSSSPHVLRNRAQSGSVPQFKKVVFQEFTDGSFTQPLYRGELNEHLGLLGPYIRAEVEDNIMVTFRNQASRPYSFYSSLISYEEDQRQGAEPRKNFVKPNETKTYFWKVQHHMAPTKDEFDCKAWAYFSDVDLEKDVHSGLIGPLLVCHTNTLNPAHGRQVTVQEFALFFTIFDETKSWYFTENMERNCRAPCNIQMEDPTFKENYRFHAINGYIMDTLPGLVMAQDQRIRWYLLSMGSNENIHSIHFSGHVFTVRKKEEYKMALYNLYPGVFETVEMLPSKAGIWRVECLIGEHLHAGMSTLFLVYSNKCQTPLGMASGHIRDFQITASGQYGQWAPKLARLHYSGSINAWSTKEPFSWIKVDLLAPMIIHGIKTQGARQKFSSLYISQFIIMYSLDGKKWQTYRGNSTGTLMVFFGNVDSSGIKHNIFNPPIIARYIRLHPTHYSIRSTLRMELMGCDLNSCSMPLGMESKAISDAQITASSYFTNMFATWSPSKARLHLQGRSNAWRPQVNNPKEWLQVDFQKTMKVTGVTTQGVKSLLTSMYVKEFLISSSQDGHQWTLFFQNGKVKVFQGNQDSFTPVVNSLDPPLLTRYLRIHPQSWVHQIALRMEVLGCEAQDLY

SEQ ID NO: 7 - DNA, 4491 bp, synthetic construct
  source 1..4491: mol_type = other DNA
gccaccaggaggtactacctgggggctgtggagctgagctgggactacatgcagtctgacctgggggagctgcctgtggatgctaggttcccccctagagtgcccaagtccttccccttcaacacttctgtggtgtacaagaagaccctgtttgtggagttcactgaccacctgtttaacattgccaagcccaggcccccttggatgggcctgctggggcccaccatccaggctgaggtgtatgacactgtggtgatcaccctgaagaacatggccagccatcctgtgagcctgcatgctgtgggggtgagctactggaaggccagcgagggggctgagtatgatgaccagactagccagagggagaaggaggatgacaaggtgtttcctggaggcagccacacctatgtgtggcaggtgctgaaggagaatggccccatggcctctgaccccctgtgcctgacctacagctacctgagccatgtggatctggtgaaggacctgaactctggcctgattggggctctgctggtgtgtagagagggcagcctggctaaggagaagacccagaccctgcataagttcatcctgctgtttgctgtgtttgatgagggcaagagctggcactctgagaccaagaacagcctgatgcaggatagggatgctgcctctgccagggcttggcccaagatgcacactgtgaatggctatgtgaataggagcctgcctggcctgattggctgccacaggaagtctgtgtactggcatgtgattggaatgggcacaacccctgaggtccatagcatcttcctggagggccacactttcctggtgaggaaccacagacaggcctctctggagattagccccatcaccttcctgactgctcagactctgctgatggacctgggccagttcctgctgttttgccatattagctctcaccagcatgatggcatggaggcctatgtgaaggtggacagctgccctgaggagcctcagctgaggatgaagaacaatgaggaggctgaagactatgatgatgacctgactgattctgagatggatgtggtgaggtttgatgatgacaatagccccagcttcattcagatcagatctgtggccaaaaagcaccccaagacctgggtgcattacattgctgctgaagaggaggactgggactatgcccctctggtgctggcccctgatgataggagctataagagccagtacctgaacaatgggccccagaggattggcagaaagtacaagaaggtgaggttcatggcttacactgatgaaaccttcaaaaccagggaggccatccagcatgagtctggcatcctgggccctctgctgtatggagaggtgggagacaccctgctgatcatcttcaagaaccaggccagcaggccctacaacatctatcctcatggcatcactgatgtgagacctctgtacagcaggaggctgcctaagggggtgaaacacctgaaggactttcccatcctgcctggggagatcttcaagtataagtggactgtgactgtggaggatggccctaccaagtctgaccccaggtgtctgacaaggtattacagcagctttgtgaacatggagagggacctggcctctggcctgattggccctctgctgatctgctacaaggagtctgtggaccagaggggcaaccagatcatgtctgacaagaggaatgtgatcctgttctctgtgtttgatgagaataggagctggtatctgactgagaacatccagagattcctgcccaatcctgctggggtgcagctggaggaccctgagtttcaggccagcaatatcatgcacagcatcaatggctatgtgtttgacagcctgcagctgtctgtgtgcctgcatgaggtggcctactggtacatcctgagcattggagcccagactgattttctgtctgtgttcttttctggctataccttcaagcacaagatggtgtatgaggacaccctgaccctgttccccttctctggggagactgtgttcatgtctatggagaatcctgggctgtggattctgggctgccacaactctgatttcaggaacaggggcatgactgccctgctgaaggtgagcagctgtgacaagaacactggggactactatgaggatagctatgaggacatttctgcttatctgctgtctaagaataatgccattgagcccaggagcttcagccagaatagcagacaccctagcaccagacagaaacagtttaatgccactaatgtgagcaacaacagcaacaccagcaatgacagcaatgtgtctaacaagacatctaacaacagcaatgccacaaacaagaccaacaacacaaatgatagcacaaacaggaccaaccagaccaataccagcccccctgtgctgaagagacatcagagggagatcaccaggactaccctgcagtctgatcaggaggagattgactatgatgacacaatctctgtggagatgaagaaggaggattttgacatctatgatgaggatgagaaccagagccccagatcttttcagaagaagaccagacactacttcattgctgctgtggagaggctgtgggactatggcatgagcagcagccctcatgtgctgaggaacagggcccagtctggctctgtgccccagttcaagaaggtggtgttccaggagtttactgatggcagcttcacccagcccctgtacagaggggagctgaatgagcacctgggcctgctgggcccttatatcagggctgaggtggaggataacattatggtgactttcaggaaccaggcctctaggccctacagcttctatagcagcctgatctcttatgaggaggatcagaggcagggggctgagcccagaaagaactttgtgaagcctaatgagactaagacctacttctggaaggtccagcaccacatggcccccaccaaggatgagtttgattgcaaggcctgggcctatttctctgatgtggacctggagaaggatgtccattctggcctgattggccctctgctggtgtgccacactaacactctgaatcctgcccatggcaggcaggtgactgtccaggagtttgccctgttcttcactatctttgatgagaccaagagctggtactttactgagaacatggagagaaactgcagggctccttgcaatatccagatggaggaccccaccttcaaggagaactacaggtttcatgccatcaatgggtacatcatggacaccctgcctggcctggtgatggctcaggaccagagaatcagatggtatctgctgagcatgggcagcaatgagaatatccacagcatccacttctctggacatgtgttcactgtgaggaagaaggaggagtacaagatggctctgtataatctgtaccctggagtgtttgaaactgtggagatgctgccttctaaggctggcatctggagggtggagtgcctgattggggagcacctgcatgctggcatgagcaccctgttcctggtgtacagcaacaagtgtcagacccccctgggcatggcctctggacacatcagggacttccagatcacagcctctggccagtatggccagtgggcccccaagctggccaggctgcattattctggcagcatcaatgcctggtctaccaaggagccctttagctggatcaaggtggacctgctggcccccatgattatccatggcatcaagacccagggggccaggcagaagttctctagcctgtacatcagccagttcatcatcatgtactctctggatggcaagaagtggcagacctacaggggcaacagcactggcacactgatggtgttctttggcaatgtggacagctctggcatcaagcacaacatcttcaatccccccattatcgctaggtatattaggctgcatcccacccactacagcatcagatctaccctgagaatggagctgatgggctgtgacctgaactcttgcagcatgcccctgggcatggagtctaaggccatctctgatgcccagattactgccagcagctacttcaccaatatgtttgccacctggagcccttctaaggccaggctgcatctgcaggggaggagcaatgcctggaggcctcaggtgaacaaccctaaggagtggctgcaggtggatttccagaagaccatgaaggtgactggagtgaccacccagggagtcaagagcctgctgaccagcatgtatgtgaaggagtttctgatcagctctagccaggatggccaccagtggactctgttctttcagaatgggaaggtgaaggtgtttcagggcaatcaggactctttcacccctgtggtgaacagcctggacccccccctgctgaccagatacctgagaatccacccccagagctgggtgcaccagatcgccctgaggatggaggtgctgggctgtgaggctcaggatctgtactga

SEQ ID NO: 8 - DNA, 4497 bp, synthetic construct
  source 1..4497: mol_type = other DNA
gccaccaggaggtactacctgggggctgtggagctgagctgggactacatgcagtctgacctgggggagctgcctgtggatgctaggttcccccctagagtgcccaagtccttccccttcaacacttctgtggtgtacaagaagaccctgtttgtggagttcactgaccacctgtttaacattgccaagcccaggcccccttggatgggcctgctggggcccaccatccaggctgaggtgtatgacactgtggtgatcaccctgaagaacatggccagccatcctgtgagcctgcatgctgtgggggtgagctactggaaggccagcgagggggctgagtatgatgaccagactagccagagggagaaggaggatgacaaggtgtttcctggaggcagccacacctatgtgtggcaggtgctgaaggagaatggccccatggcctctgaccccctgtgcctgacctacagctacctgagccatgtggatctggtgaaggacctgaactctggcctgattggggctctgctggtgtgtagagagggcagcctggctaaggagaagacccagaccctgcataagttcatcctgctgtttgctgtgtttgatgagggcaagagctggcactctgagaccaagaacagcctgatgcaggatagggatgctgcctctgccagggcttggcccaagatgcacactgtgaatggctatgtgaataggagcctgcctggcctgattggctgccacaggaagtctgtgtactggcatgtgattggaatgggcacaacccctgaggtccatagcatcttcctggagggccacactttcctggtgaggaaccacagacaggcctctctggagattagccccatcaccttcctgactgctcagactctgctgatggacctgggccagttcctgctgttttgccatattagctctcaccagcatgatggcatggaggcctatgtgaaggtggacagctgccctgaggagcctcagctgaggatgaagaacaatgaggaggctgaagactatgatgatgacctgactgattctgagatggatgtggtgaggtttgatgatgacaatagccccagcttcattcagatcagatctgtggccaaaaagcaccccaagacctgggtgcattacattgctgctgaagaggaggactgggactatgcccctctggtgctggcccctgatgataggagctataagagccagtacctgaacaatgggccccagaggattggcagaaagtacaagaaggtgaggttcatggcttacactgatgaaaccttcaaaaccagggaggccatccagcatgagtctggcatcctgggccctctgctgtatggagaggtgggagacaccctgctgatcatcttcaagaaccaggccagcaggccctacaacatctatcctcatggcatcactgatgtgagacctctgtacagcaggaggctgcctaagggggtgaaacacctgaaggactttcccatcctgcctggggagatcttcaagtataagtggactgtgactgtggaggatggccctaccaagtctgaccccaggtgtctgacaaggtattacagcagctttgtgaacatggagagggacctggcctctggcctgattggccctctgctgatctgctacaaggagtctgtggaccagaggggcaaccagatcatgtctgacaagaggaatgtgatcctgttctctgtgtttgatgagaataggagctggtatctgactgagaacatccagagattcctgcccaatcctgctggggtgcagctggaggaccctgagtttcaggccagcaatatcatgcacagcatcaatggctatgtgtttgacagcctgcagctgtctgtgtgcctgcatgaggtggcctactggtacatcctgagcattggagcccagactgattttctgtctgtgttcttttctggctataccttcaagcacaagatggtgtatgaggacaccctgaccctgttccccttctctggggagactgtgttcatgtctatggagaatcctgggctgtggattctgggctgccacaactctgatttcaggaacaggggcatgactgccctgctgaaggtgagcagctgtgacaagaacactggggactactatgaggatagctatgaggacatttctgcttatctgctgtctaagaataatgccattgagcccaggagcttcagccagaattctagacaccctagcaccagacagaaacagtttaatgccactaatgtgtctaacaacagcaacaccagcaatgacagcaatgtgtctaacaagacatctaacaacagcaacgccacaaacaagaccaacaacacaaatgatagcacaaaccggaccaaccagaccaataccagccagcagaacttcgtgacccagagaagtaagagagagatcaccaggactaccctgcagtctgatcaggaggagattgactatgatgacacaatctctgtggagatgaagaaggaggattttgacatctatgatgaggatgagaaccagagccccagatcttttcagaagaagaccagacactacttcattgctgctgtggagaggctgtgggactatggcatgagcagcagccctcatgtgctgaggaacagggcccagtctggctctgtgccccagttcaagaaggtggtgttccaggagtttactgatggcagcttcacccagcccctgtacagaggggagctgaatgagcacctgggcctgctgggcccttatatcagggctgaggtggaggataacattatggtgactttcaggaaccaggcctctaggccctacagcttctatagcagcctgatctcttatgaggaggatcagaggcagggggctgagcccagaaagaactttgtgaagcctaatgagactaagacctacttctggaaggtccagcaccacatggcccccaccaaggatgagtttgattgcaaggcctgggcctatttctctgatgtggacctggagaaggatgtccattctggcctgattggccctctgctggtgtgccacactaacactctgaatcctgcccatggcaggcaggtgactgtccaggagtttgccctgttcttcactatctttgatgagaccaagagctggtactttactgagaacatggagagaaactgcagggctccttgcaatatccagatggaggaccccaccttcaaggagaactacaggtttcatgccatcaatgggtacatcatggacaccctgcctggcctggtgatggctcaggaccagagaatcagatggtatctgctgagcatgggcagcaatgagaatatccacagcatccacttctctggacatgtgttcactgtgaggaagaaggaggagtacaagatggctctgtataatctgtaccctggagtgtttgaaactgtggagatgctgccttctaaggctggcatctggagggtggagtgcctgattggggagcacctgcatgctggcatgagcaccctgttcctggtgtacagcaacaagtgtcagacccccctgggcatggcctctggacacatcagggacttccagatcacagcctctggccagtatggccagtgggcccccaagctggccaggctgcattattctggcagcatcaatgcctggtctaccaaggagccctttagctggatcaaggtggacctgctggcccccatgattatccatggcatcaagacccagggggccaggcagaagttctctagcctgtacatcagccagttcatcatcatgtactctctggatggcaagaagtggcagacctacaggggcaacagcactggcacactgatggtgttctttggcaatgtggacagctctggcatcaagcacaacatcttcaatccccccattatcgctaggtatattaggctgcatcccacccactacagcatcagatctaccctgagaatggagctgatgggctgtgacctgaactcttgcagcatgcccctgggcatggagtctaaggccatctctgatgcccagattactgccagcagctacttcaccaatatgtttgccacctggagcccttctaaggccaggctgcatctgcaggggaggagcaatgcctggaggcctcaggtgaacaaccctaaggagtggctgcaggtggatttccagaagaccatgaaggtgactggagtgaccacccagggagtcaagagcctgctgaccagcatgtatgtgaaggagtttctgatcagctctagccaggatggccaccagtggactctgttctttcagaatgggaaggtgaaggtgtttcagggcaatcaggactctttcacccctgtggtgaacagcctggacccccccctgctgaccagatacctgagaatccacccccagagctgggtgcaccagatcgccctgaggatggaggtgctgggctgtgaggctcaggatctgtactga

SEQ ID NO: 9 - protein, 31 aa, synthetic construct
SFSQNATNVSNNSNTSNDSNVSPPVLKRHQR

SEQ ID NO: 10 - protein, 21 aa, synthetic construct
SFSQNSRHPSQNPPVLKRHQR

SEQ ID NO: 11 - protein, 2122 aa, synthetic construct
ATRRYYLGAVELSWDYMQSDLGELPVDARFPPRVPKSFPFNTSVVYKKTLFVEFTDHLFNIAKPRPPWMGLLGPTIQAEVYDTVVITLKNMASHPVSLHAVGVSYWKASEGAEYDDQTSQREKEDDKVFPGGSHTYVWQVLKENGPMASDPLCLTYSYLSHVDLVKDLNSGLIGALLVCREGSLAKEKTQTLHKFILLFAVFDEGKSWHSETKNSLMQDRDAASARAWPKMHTVNGYVNRSLPGLIGCHRKSVYWHVIGMGTTPEVHSIFLEGHTFLVRNHRQASLEISPITFLTAQTLLMDLGQFLLFCHISSHQHDGMEAYVKVDSCPEEPQLRMKNNEEAEDYDDDLTDSEMDVVRFDDDNSPSFIQIRSVAKKHPKTWVHYIAAEEEDWDYAPLVLAPDDRSYKSQYLNNGPQRIGRKYKKVRFMAYTDETFKTREAIQHESGILGPLLYGEVGDTLLIIFKNQASRPYNIYPHGITDVRPLYSRRLPKGVKHLKDFPILPGEIFKYKWTVTVEDGPTKSDPRCLTRYYSSFVNMERDLASGLIGPLLICYKESVDQRGNQIMSDKRNVILFSVFDENRSWYLTENIQRFLPNPAGVQLEDPEFQASNIMHSINGYVFDSLQLSVCLHEVAYWYILSIGAQTDFLSVFFSGYTFKHKMVYEDTLTLFPFSGETVFMSMENPGLWILGCHNSDFRNRGMTALLKVSSCDKNTGDYYEDSYEDISAYLLSKNNAIEPRSFSQNPPVLKRHQREITRTTLQSDQEEIDYDDTISVEMKKEDFDIYDEDENQSPRSFQKKTRHYFIAAVERLWDYGMSSSPHVLRNRAQSGSVPQFKKVVFQEFTDGSFTQPLYRGELNEHLGLLGPYIRAEVEDNIMVTFRNQASRPYSFYSSLISYEEDQRQGAEPRKNFVKPNETKTYFWKVQHHMAPTKDEFDCKAWAYFSDVDLEKDVHSGLIGPLLVCHTNTLNPAHGRQVTVQEFALFFTIFDETKSWYFTENMERNCRAPCNIQMEDPTFKENYRFHAINGYIMDTLPGLVMAQDQRIRWYLLSMGSNENIHSIHFSGHVFTVRKKEEYKMALYNLYPGVFETVEMLPSKAGIWRVECLIGEHLHAGMSTLFLVYSNKCQTPLGMASGHIRDFQITASGQYGQWAPKLARLHYSGSINAWSTKEPFSWIKVDLLAPMIIHGIKTQGARQKFSSLYISQFIIMYSLDGKKWQTYRGNSTGTLMVFFGNVDSSGIKHNIFNPPIIARYIRLHPTHYSIRSTLRMELMGCDLNSCSMPLGMESKAISDAQITASSYFTNMFATWSPSKARLHLQGRSNAWRPQVNNPKEWLQVDFQKTMKVTGVTTQGVKSLLTSMYVKEFLISSSQDGHQWTLFFQNGKVKVFQGNQDSFTPVVNSLDPPLLTRYLRIHPQSWVHQIALRMEVLGCEAQDLYEITRTTLQSDQEEIDYDDTISVEMKKEDFDIYDEDENQSPRSFQKKTRHYFIAAVERLWDYGMSSSPHVLRNRAQSGSVPQFKKVVFQEFTDGSFTQPLYRGELNEHLGLLGPYIRAEVEDNIMVTFRNQASRPYSFYSSLISYEEDQRQGAEPRKNFVKPNETKTYFWKVQHHMAPTKDEFDCKAWAYFSDVDLEKDVHSGLIGPLLVCHTNTLNPAHGRQVTVQEFALFFTIFDETKSWYFTENMERNCRAPCNIQMEDPTFKENYRFHAINGYIMDTLPGLVMAQDQRIRWYLLSMGSNENIHSIHFSGHVFTVRKKEEYKMALYNLYPGVFETVEMLPSKAGIWRVECLIGEHLHAGMSTLFLVYSNKCQTPLGMASGHIRDFQITASGQYGQWAPKLARLHYSGSINAWSTKEPFSWIKVDLLAPMIIHGIKTQGARQKFSSLYISQFIIMYSLDGKKWQTYRGNSTGTLMVFFGNVDSSGIKHNIFNPPIIARYIRLHPTHYSIRSTLRMELMGCDLNSCSMPLGMESKAISDAQITASSYFTNMFATWSPSKARLHLQGRSNAWRPQVNNPKEWLQVDFQKTMKVTGVTTQGVKSLLTSMYVKEFLISSSQDGHQWTLFFQNGKVKVFQGNQDSFTPVVNSLDPPLLTRYLRIHPQSWVHQIALRMEVLGCEAQDLY

SEQ ID NO: 12 - protein, 1455 aa, synthetic construct
ATRRYYLGAVELSWDYMQSDLGELPVDARFPPRVPKSFPFNTSVVYKKTLFVEFTDHLFNIAKPRPPWMGLLGPTIQAEVYDTVVITLKNMASHPVSLHAVGVSYWKASEGAEYDDQTSQREKEDDKVFPGGSHTYVWQVLKENGPMASDPLCLTYSYLSHVDLVKDLNSGLIGALLVCREGSLAKEKTQTLHKFILLFAVFDEGKSWHSETKNSLMQDRDAASARAWPKMHTVNGYVNRSLPGLIGCHRKSVYWHVIGMGTTPEVHSIFLEGHTFLVRNHRQASLEISPITFLTAQTLLMDLGQFLLFCHISSHQHDGMEAYVKVDSCPEEPQLRMKNNEEAEDYDDDLTDSEMDVVRFDDDNSPSFIQIRSVAKKHPKTWVHYIAAEEEDWDYAPLVLAPDDRSYKSQYLNNGPQRIGRKYKKVRFMAYTDETFKTREAIQHESGILGPLLYGEVGDTLLIIFKNQASRPYNIYPHGITDVRPLYSRRLPKGVKHLKDFPILPGEIFKYKWTVTVEDGPTKSDPRCLTRYYSSFVNMERDLASGLIGPLLICYKESVDQRGNQIMSDKRNVILFSVFDENRSWYLTENIQRFLPNPAGVQLEDPEFQASNIMHSINGYVFDSLQLSVCLHEVAYWYILSIGAQTDFLSVFFSGYTFKHKMVYEDTLTLFPFSGETVFMSMENPGLWILGCHNSDFRNRGMTALLKVSSCDKNTGDYYEDSYEDISAYLLSKNNAIEPRSFSQNATNVSNNSNTSNDSNVSPPVLKRHQREITRTTLQSDQEEIDYDDTISVEMKKEDFDIYDEDENQSPRSFQKKTRHYFIAAVERLWDYGMSSSPHVLRNRAQSGSVPQFKKVVFQEFTDGSFTQPLYRGELNEHLGLLGPYIRAEVEDNIMVTFRNQASRPYSFYSSLISYEEDQRQGAEPRKNFVKPNETKTYFWKVQHHMAPTKDEFDCKAWAYFSDVDLEKDVHSGLIGPLLVCHTNTLNPAHGRQVTVQEFALFFTIFDETKSWYFTENMERNCRAPCNIQMEDPTFKENYRFHAINGYIMDTLPGLVMAQDQRIRWYLLSMGSNENIHSIHFSGHVFTVRKKEEYKMALYNLYPGVFETVEMLPSKAGIWRVECLIGEHLHAGMSTLFLVYSNKCQTPLGMASGHIRDFQITASGQYGQWAPKLARLHYSGSINAWSTKEPFSWIKVDLLAPMIIHGIKTQGARQKFSSLYISQFIIMYSLDGKKWQTYRGNSTGTLMVFFGNVDSSGIKHNIFNPPIIARYIRLHPTHYSIRSTLRMELMGCDLNSCSMPLGMESKAISDAQITASSYFTNMFATWSPSKARLHLQGRSNAWRPQVNNPKEWLQVDFQKTMKVTGVTTQGVKSLLTSMYVKEFLISSSQDGHQWTLFFQNGKVKVFQGNQDSFTPVVNSLDPPLLTRYLRIHPQSWVHQIALRMEVLGCEAQDLY

SEQ ID NO: 13 - protein, 1445 aa, synthetic construct
ATRRYYLGAVELSWDYMQSDLGELPVDARFPPRVPKSFPFNTSVVYKKTLFVEFTDHLFNIAKPRPPWMGLLGPTIQAEVYDTVVITLKNMASHPVSLHAVGVSYWKASEGAEYDDQTSQREKEDDKVFPGGSHTYVWQVLKENGPMASDPLCLTYSYLSHVDLVKDLNSGLIGALLVCREGSLAKEKTQTLHKFILLFAVFDEGKSWHSETKNSLMQDRDAASARAWPKMHTVNGYVNRSLPGLIGCHRKSVYWHVIGMGTTPEVHSIFLEGHTFLVRNHRQASLEISPITFLTAQTLLMDLGQFLLFCHISSHQHDGMEAYVKVDSCPEEPQLRMKNNEEAEDYDDDLTDSEMDVVRFDDDNSPSFIQIRSVAKKHPKTWVHYIAAEEEDWDYAPLVLAPDDRSYKSQYLNNGPQRIGRKYKKVRFMAYTDETFKTREAIQHESGILGPLLYGEVGDTLLIIFKNQASRPYNIYPHGITDVRPLYSRRLPKGVKHLKDFPILPGEIFKYKWTVTVEDGPTKSDPRCLTRYYSSFVNMERDLASGLIGPLLICYKESVDQRGNQIMSDKRNVILFSVFDENRSWYLTENIQRFLPNPAGVQLEDPEFQASNIMHSINGYVFDSLQLSVCLHEVAYWYILSIGAQTDFLSVFFSGYTFKHKMVYEDTLTLFPFSGETVFMSMENPGLWILGCHNSDFRNRGMTALLKVSSCDKNTGDYYEDSYEDISAYLLSKNNAIEPRSFSQNSRHPSQNPPVLKRHQREITRTTLQSDQEEIDYDDTISVEMKKEDFDIYDEDENQSPRSFQKKTRHYFIAAVERLWDYGMSSSPHVLRNRAQSGSVPQFKKVVFQEFTDGSFTQPLYRGELNEHLGLLGPYIRAEVEDNIMVTFRNQASRPYSFYSSLISYEEDQRQGAEPRKNFVKPNETKTYFWKVQHHMAPTKDEFDCKAWAYFSDVDLEKDVHSGLIGPLLVCHTNTLNPAHGRQVTVQEFALFFTIFDETKSWYFTENMERNCRAPCNIQMEDPTFKENYRFHAINGYIMDTLPGLVMAQDQRIRWYLLSMGSNENIHSIHFSGHVFTVRKKEEYKMALYNLYPGVFETVEMLPSKAGIWRVECLIGEHLHAGMSTLFLVYSNKCQTPLGMASGHIRDFQITASGQYGQWAPKLARLHYSGSINAWSTKEPFSWIKVDLLAPMIIHGIKTQGARQKFSSLYISQFIIMYSLDGKKWQTYRGNSTGTLMVFFGNVDSSGIKHNIFNPPIIARYIRLHPTHYSIRSTLRMELMGCDLNSCSMPLGMESKAISDAQITASSYFTNMFATWSPSKARLHLQGRSNAWRPQVNNPKEWLQVDFQKTMKVTGVTTQGVKSLLTSMYVKEFLISSSQDGHQWTLFFQNGKVKVFQGNQDSFTPVVNSLDPPLLTRYLRIHPQSWVHQIALRMEVLGCEAQDLY

SEQ ID NO: 14 - protein, 1539 aa, synthetic construct
ATRRYYLGAVELSWDYMQSDLGELPVDARFPPRVPKSFPFNTSVVYKKTLFVEFTDHLFNIAKPRPPWMGLLGPTIQAEVYDTVVITLKNMASHPVSLHAVGVSYWKASEGAEYDDQTSQREKEDDKVFPGGSHTYVWQVLKENGPMASDPLCLTYSYLSHVDLVKDLNSGLIGALLVCREGSLAKEKTQTLHKFILLFAVFDEGKSWHSETKNSLMQDRDAASARAWPKMHTVNGYVNRSLPGLIGCHRKSVYWHVIGMGTTPEVHSIFLEGHTFLVRNHRQASLEISPITFLTAQTLLMDLGQFLLFCHISSHQHDGMEAYVKVDSCPEEPQLRMKNNEEAEDYDDDLTDSEMDVVRFDDDNSPSFIQIRSVAKKHPKTWVHYIAAEEEDWDYAPLVLAPDDRSYKSQYLNNGPQRIGRKYKKVRFMAYTDETFKTREAIQHESGILGPLLYGEVGDTLLIIFKNQASRPYNIYPHGITDVRPLYSRRLPKGVKHLKDFPILPGEIFKYKWTVTVEDGPTKSDPRCLTRYYSSFVNMERDLASGLIGPLLICYKESVDQRGNQIMSDKRNVILFSVFDENRSWYLTENIQRFLPNPAGVQLEDPEFQASNIMHSINGYVFDSLQLSVCLHEVAYWYILSIGAQTDFLSVFFSGYTFKHKMVYEDTLTLFPFSGETVFMSMENPGLWILGCHNSDFRNRGMTALLKVSSCDKNTGDYYEDSYEDISAYLLSKNNAIEPRSFSQNSRHPSTRQKQFNATNVSNNSNTSNDSNVSNKTSNNSNATNKTNNTNDSTNRTNQTNTSQQNFVTQRRKRGSGATNFSLLKQAGDVEENPGPMQIELSTCFFLCLLRFCFSEITRTTLQSDQEEIDYDDTISVEMKKEDFDIYDEDENQSPRSFQKKTRHYFIAAVERLWDYGMSSSPHVLRNRAQSGSVPQFKKVVFQEFTDGSFTQPLYRGELNEHLGLLGPYIRAEVEDNIMVTFRNQASRPYSFYSSLISYEEDQRQGAEPRKNFVKPNETKTYFWKVQHHMAPTKDEFDCKAWAYFSDVDLEKDVHSGLIGPLLVCHTNTLNPAHGRQVTVQEFALFFTIFDETKSWYFTENMERNCRAPCNIQMEDPTFKENYRFHAINGYIMDTLPGLVMAQDQRIRWYLLSMGSNENIHSIHFSGHVFTVRKKEEYKMALYNLYPGVFETVEMLPSKAGIWRVECLIGEHLHAGMSTLFLVYSNKCQTPLGMASGHIRDFQITASGQYGQWAPKLARLHYSGSINAWSTKEPFSWIKVDLLAPMIIHGIKTQGARQKFSSLYISQFIIMYSLDGKKWQTYRGNSTGTLMVFFGNVDSSGIKHNIFNPPIIARYIRLHPTHYSIRSTLRMELMGCDLNSCSMPLGMESKAISDAQITASSYFTNMFATWSPSKARLHLQGRSNAWRPQVNNPKEWLQVDFQKTMKVTGVTTQGVKSLLTSMYVKEFLISSSQDGHQWTLFFQNGKVKVFQGNQDSFTPVVNSLDPPLLTRYLRIHPQSWVHQIALRMEVLGCEAQDLY

SEQ ID NO: 15 - DNA, 4317 bp, synthetic construct
  source 1..4317: mol_type = other DNA
gccaccaggaggtactacctgggggctgtggagctgagctgggactacatgcagtctgacctgggggagctgcctgtggatgctaggttcccccctagagtgcccaagtccttccccttcaacacttctgtggtgtacaagaagaccctgtttgtggagttcactgaccacctgtttaacattgccaagcccaggcccccttggatgggcctgctggggcccaccatccaggctgaggtgtatgacactgtggtgatcaccctgaagaacatggccagccatcctgtgagcctgcatgctgtgggggtgagctactggaaggccagcgagggggctgagtatgatgaccagactagccagagggagaaggaggatgacaaggtgtttcctggaggcagccacacctatgtgtggcaggtgctgaaggagaatggccccatggcctctgaccccctgtgcctgacctacagctacctgagccatgtggatctggtgaaggacctgaactctggcctgattggggctctgctggtgtgtagagagggcagcctggctaaggagaagacccagaccctgcataagttcatcctgctgtttgctgtgtttgatgagggcaagagctggcactctgagaccaagaacagcctgatgcaggatagggatgctgcctctgccagggcttggcccaagatgcacactgtgaatggctatgtgaataggagcctgcctggcctgattggctgccacaggaagtctgtgtactggcatgtgattggaatgggcacaacccctgaggtccatagcatcttcctggagggccacactttcctggtgaggaaccacagacaggcctctctggagattagccccatcaccttcctgactgctcagactctgctgatggacctgggccagttcctgctgttttgccatattagctctcaccagcatgatggcatggaggcctatgtgaaggtggacagctgccctgaggagcctcagctgaggatgaagaacaatgaggaggctgaagactatgatgatgacctgactgattctgagatggatgtggtgaggtttgatgatgacaatagccccagcttcattcagatcagatctgtggccaaaaagcaccccaagacctgggtgcattacattgctgctgaagaggaggactgggactatgcccctctggtgctggcccctgatgataggagctataagagccagtacctgaacaatgggccccagaggattggcagaaagtacaagaaggtgaggttcatggcttacactgatgaaaccttcaaaaccagggaggccatccagcatgagtctggcatcctgggccctctgctgtatggagaggtgggagacaccctgctgatcatcttcaagaaccaggccagcaggccctacaacatctatcctcatggcatcactgatgtgagacctctgtacagcaggaggctgcctaagggggtgaaacacctgaaggactttcccatcctgcctggggagatcttcaagtataagtggactgtgactgtggaggatggccctaccaagtctgaccccaggtgtctgacaaggtattacagcagctttgtgaacatggagagggacctggcctctggcctgattggccctctgctgatctgctacaaggagtctgtggaccagaggggcaaccagatcatgtctgacaagaggaatgtgatcctgttctctgtgtttgatgagaataggagctggtatctgactgagaacatccagagattcctgcccaatcctgctggggtgcagctggaggaccctgagtttcaggccagcaatatcatgcacagcatcaatggctatgtgtttgacagcctgcagctgtctgtgtgcctgcatgaggtggcctactggtacatcctgagcattggagcccagactgattttctgtctgtgttcttttctggctataccttcaagcacaagatggtgtatgaggacaccctgaccctgttccccttctctggggagactgtgttcatgtctatggagaatcctgggctgtggattctgggctgccacaactctgatttcaggaacaggggcatgactgccctgctgaaggtgagcagctgtgacaagaacactggggactactatgaggatagctatgaggacatttctgcttatctgctgtctaagaataatgccattgagcccaggagcttcagccagaatccccctgtgctgaagagacatcagagggagatcaccaggactaccctgcagtctgatcaggaggagattgactatgatgacacaatctctgtggagatgaagaaggaggattttgacatctatgatgaggatgagaaccagagccccagatcttttcagaagaagaccagacactacttcattgctgctgtggagaggctgtgggactatggcatgagcagcagccctcatgtgctgaggaacagggcccagtctggctctgtgccccagttcaagaaggtggtgttccaggagtttactgatggcagcttcacccagcccctgtacagaggggagctgaatgagcacctgggcctgctgggcccttatatcagggctgaggtggaggataacattatggtgactttcaggaaccaggcctctaggccctacagcttctatagcagcctgatctcttatgaggaggatcagaggcagggggctgagcccagaaagaactttgtgaagcctaatgagactaagacctacttctggaaggtccagcaccacatggcccccaccaaggatgagtttgattgcaaggcctgggcctatttctctgatgtggacctggagaaggatgtccattctggcctgattggccctctgctggtgtgccacactaacactctgaatcctgcccatggcaggcaggtgactgtccaggagtttgccctgttcttcactatctttgatgagaccaagagctggtactttactgagaacatggagagaaactgcagggctccttgcaatatccagatggaggaccccaccttcaaggagaactacaggtttcatgccatcaatgggtacatcatggacaccctgcctggcctggtgatggctcaggaccagagaatcagatggtatctgctgagcatgggcagcaatgagaatatccacagcatccacttctctggacatgtgttcactgtgaggaagaaggaggagtacaagatggctctgtataatctgtaccctggagtgtttgaaactgtggagatgctgccttctaaggctggcatctggagggtggagtgcctgattggggagcacctgcatgctggcatgagcaccctgttcctggtgtacagcaacaagtgtcagacccccctgggcatggcctctggacacatcagggacttccagatcacagcctctggccagtatggccagtgggcccccaagctggccaggctgcattattctggcagcatcaatgcctggtctaccaaggagccctttagctggatcaaggtggacctgctggcccccatgattatccatggcatcaagacccagggggccaggcagaagttctctagcctgtacatcagccagttcatcatcatgtactctctggatggcaagaagtggcagacctacaggggcaacagcactggcacactgatggtgttctttggcaatgtggacagctctggcatcaagcacaacatcttcaatccccccattatcgctaggtatattaggctgcatcccacccactacagcatcagatctaccctgagaatggagctgatgggctgtgacctgaactcttgcagcatgcccctgggcatggagtctaaggccatctctgatgcccagattactgccagcagctacttcaccaatatgtttgccacctggagcccttctaaggccaggctgcatctgcaggggaggagcaatgcctggaggcctcaggtgaacaaccctaaggagtggctgcaggtggatttccagaagaccatgaaggtgactggagtgaccacccagggagtcaagagcctgctgaccagcatgtatgtgaaggagtttctgatcagctctagccaggatggccaccagtggactctgttctttcagaatgggaaggtgaaggtgtttcagggcaatcaggactctttcacccctgtggtgaacagcctggacccccccctgctgaccagatacctgagaatccacccccagagctgggtgcaccagatcgccctgaggatggaggtgctgggctgtgaggctcaggatctgtactga

SEQ ID NO: 16 - DNA, 4368 bp, synthetic construct
  source 1..4368: mol_type = other DNA
gccaccaggaggtactacctgggggctgtggagctgagctgggactacatgcagtctgacctgggggagctgcctgtggatgctaggttcccccctagagtgcccaagtccttccccttcaacacttctgtggtgtacaagaagaccctgtttgtggagttcactgaccacctgtttaacattgccaagcccaggcccccttggatgggcctgctggggcccaccatccaggctgaggtgtatgacactgtggtgatcaccctgaagaacatggccagccatcctgtgagcctgcatgctgtgggggtgagctactggaaggccagcgagggggctgagtatgatgaccagactagccagagggagaaggaggatgacaaggtgtttcctggaggcagccacacctatgtgtggcaggtgctgaaggagaatggccccatggcctctgaccccctgtgcctgacctacagctacctgagccatgtggatctggtgaaggacctgaactctggcctgattggggctctgctggtgtgtagagagggcagcctggctaaggagaagacccagaccctgcataagttcatcctgctgtttgctgtgtttgatgagggcaagagctggcactctgagaccaagaacagcctgatgcaggatagggatgctgcctctgccagggcttggcccaagatgcacactgtgaatggctatgtgaataggagcctgcctggcctgattggctgccacaggaagtctgtgtactggcatgtgattggaatgggcacaacccctgaggtccatagcatcttcctggagggccacactttcctggtgaggaaccacagacaggcctctctggagattagccccatcaccttcctgactgctcagactctgctgatggacctgggccagttcctgctgttttgccatattagctctcaccagcatgatggcatggaggcctatgtgaaggtggacagctgccctgaggagcctcagctgaggatgaagaacaatgaggaggctgaagactatgatgatgacctgactgattctgagatggatgtggtgaggtttgatgatgacaatagccccagcttcattcagatcagatctgtggccaaaaagcaccccaagacctgggtgcattacattgctgctgaagaggaggactgggactatgcccctctggtgctggcccctgatgataggagctataagagccagtacctgaacaatgggccccagaggattggcagaaagtacaagaaggtgaggttcatggcttacactgatgaaaccttcaaaaccagggaggccatccagcatgagtctggcatcctgggccctctgctgtatggagaggtgggagacaccctgctgatcatcttcaagaaccaggccagcaggccctacaacatctatcctcatggcatcactgatgtgagacctctgtacagcaggaggctgcctaagggggtgaaacacctgaaggactttcccatcctgcctggggagatcttcaagtataagtggactgtgactgtggaggatggccctaccaagtctgaccccaggtgtctgacaaggtattacagcagctttgtgaacatggagagggacctggcctctggcctgattggccctctgctgatctgctacaaggagtctgtggaccagaggggcaaccagatcatgtctgacaagaggaatgtgatcctgttctctgtgtttgatgagaataggagctggtatctgactgagaacatccagagattcctgcccaatcctgctggggtgcagctggaggaccctgagtttcaggccagcaatatcatgcacagcatcaatggctatgtgtttgacagcctgcagctgtctgtgtgcctgcatgaggtggcctactggtacatcctgagcattggagcccagactgattttctgtctgtgttcttttctggctataccttcaagcacaagatggtgtatgaggacaccctgaccctgttccccttctctggggagactgtgttcatgtctatggagaatcctgggctgtggattctgggctgccacaactctgatttcaggaacaggggcatgactgccctgctgaaggtgagcagctgtgacaagaacactggggactactatgaggatagctatgaggacatttctgcttatctgctgtctaagaataatgccattgagcccaggagcttcagccagaatgccactaatgtgtctaacaacagcaacaccagcaatgacagcaatgtgtctccccctgtgctgaagagacatcagagggagatcaccaggactaccctgcagtctgatcaggaggagattgactatgatgacacaatctctgtggagatgaagaaggaggattttgacatctatgatgaggatgagaaccagagccccagatcttttcagaagaagaccagacactacttcattgctgctgtggagaggctgtgggactatggcatgagcagcagccctcatgtgctgaggaacagggcccagtctggctctgtgccccagttcaagaaggtggtgttccaggagtttactgatggcagcttcacccagcccctgtacagaggggagctgaatgagcacctgggcctgctgggcccttatatcagggctgaggtggaggataacattatggtgactttcaggaaccaggcctctaggccctacagcttctatagcagcctgatctcttatgaggaggatcagaggcagggggctgagcccagaaagaactttgtgaagcctaatgagactaagacctacttctggaaggtccagcaccacatggcccccaccaaggatgagtttgattgcaaggcctgggcctatttctctgatgtggacctggagaaggatgtccattctggcctgattggccctctgctggtgtgccacactaacactctgaatcctgcccatggcaggcaggtgactgtccaggagtttgccctgttcttcactatctttgatgagaccaagagctggtactttactgagaacatggagagaaactgcagggctccttgcaatatccagatggaggaccccaccttcaaggagaactacaggtttcatgccatcaatgggtacatcatggacaccctgcctggcctggtgatggctcaggaccagagaatcagatggtatctgctgagcatgggcagcaatgagaatatccacagcatccacttctctggacatgtgttcactgtgaggaagaaggaggagtacaagatggctctgtataatctgtaccctggagtgtttgaaactgtggagatgctgccttctaaggctggcatctggagggtggagtgcctgattggggagcacctgcatgctggcatgagcaccctgttcctggtgtacagcaacaagtgtcagacccccctgggcatggcctctggacacatcagggacttccagatcacagcctctggccagtatggccagtgggcccccaagctggccaggctgcattattctggcagcatcaatgcctggtctaccaaggagccctttagctggatcaaggtggacctgctggcccccatgattatccatggcatcaagacccagggggccaggcagaagttctctagcctgtacatcagccagttcatcatcatgtactctctggatggcaagaagtggcagacctacaggggcaacagcactggcacactgatggtgttctttggcaatgtggacagctctggcatcaagcacaacatcttcaatccccccattatcgctaggtatattaggctgcatcccacccactacagcatcagatctaccctgagaatggagctgatgggctgtgacctgaactcttgcagcatgcccctgggcatggagtctaaggccatctctgatgcccagattactgccagcagctacttcaccaatatgtttgccacctggagcccttctaaggccaggctgcatctgcaggggaggagcaatgcctggaggcctcaggtgaacaaccctaaggagtggctgcaggtggatttccagaagaccatgaaggtgactggagtgaccacccagggagtcaagagcctgctgaccagcatgtatgtgaaggagtttctgatcagctctagccaggatggccaccagtggactctgttctttcagaatgggaaggtgaaggtgtttcagggcaatcaggactctttcacccctgtggtgaacagcctggacccccccctgctgaccagatacctgagaatccacccccagagctgggtgcaccagatcgccctgaggatggaggtgctgggctgtgaggctcaggatctgtactga

SEQ ID NO: 17 - DNA, 4338 bp, synthetic construct
  source 1..4338: mol_type = other DNA
gccaccaggaggtactacctgggggctgtggagctgagctgggactacatgcagtctgacctgggggagctgcctgtggatgctaggttcccccctagagtgcccaagtccttccccttcaacacttctgtggtgtacaagaagaccctgtttgtggagttcactgaccacctgtttaacattgccaagcccaggcccccttggatgggcctgctggggcccaccatccaggctgaggtgtatgacactgtggtgatcaccctgaagaacatggccagccatcctgtgagcctgcatgctgtgggggtgagctactggaaggccagcgagggggctgagtatgatgaccagactagccagagggagaaggaggatgacaaggtgtttcctggaggcagccacacctatgtgtggcaggtgctgaaggagaatggccccatggcctctgaccccctgtgcctgacctacagctacctgagccatgtggatctggtgaaggacctgaactctggcctgattggggctctgctggtgtgtagagagggcagcctggctaaggagaagacccagaccctgcataagttcatcctgctgtttgctgtgtttgatgagggcaagagctggcactctgagaccaagaacagcctgatgcaggatagggatgctgcctctgccagggcttggcccaagatgcacactgtgaatggctatgtgaataggagcctgcctggcctgattggctgccacaggaagtctgtgtactggcatgtgattggaatgggcacaacccctgaggtccatagcatcttcctggagggccacactttcctggtgaggaaccacagacaggcctctctggagattagccccatcaccttcctgactgctcagactctgctgatggacctgggccagttcctgctgttttgccatattagctctcaccagcatgatggcatggaggcctatgtgaaggtggacagctgccctgaggagcctcagctgaggatgaagaacaatgaggaggctgaagactatgatgatgacctgactgattctgagatggatgtggtgaggtttgatgatgacaatagccccagcttcattcagatcagatctgtggccaaaaagcaccccaagacctgggtgcattacattgctgctgaagaggaggactgggactatgcccctctggtgctggcccctgatgataggagctataagagccagtacctgaacaatgggccccagaggattggcagaaagtacaagaaggtgaggttcatggcttacactgatgaaaccttcaaaaccagggaggccatccagcatgagtctggcatcctgggccctctgctgtatggagaggtgggagacaccctgctgatcatcttcaagaaccaggccagcaggccctacaacatctatcctcatggcatcactgatgtgagacctctgtacagcaggaggctgcctaagggggtgaaacacctgaaggactttcccatcctgcctggggagatcttcaagtataagtggactgtgactgtggaggatggccctaccaagtctgaccccaggtgtctgacaaggtattacagcagctttgtgaacatggagagggacctggcctctggcctgattggccctctgctgatctgctacaaggagtctgtggaccagaggggcaaccagatcatgtctgacaagaggaatgtgatcctgttctctgtgtttgatgagaataggagctggtatctgactgagaacatccagagattcctgcccaatcctgctggggtgcagctggaggaccctgagtttcaggccagcaatatcatgcacagcatcaatggctatgtgtttgacagcctgcagctgtctgtgtgcctgcatgaggtggcctactggtacatcctgagcattggagcccagactgattttctgtctgtgttcttttctggctataccttcaagcacaagatggtgtatgaggacaccctgaccctgttccccttctctggggagactgtgttcatgtctatggagaatcctgggctgtggattctgggctgccacaactctgatttcaggaacaggggcatgactgccctgctgaaggtgagcagctgtgacaagaacactggggactactatgaggatagctatgaggacatttctgcttatctgctgtctaagaataatgccattgagcccaggagcttcagccagaattctagacaccctagccaaaacccccctgtgctgaagagacatcagagggagatcaccaggactaccctgcagtctgatcaggaggagattgactatgatgacacaatctctgtggagatgaagaaggaggattttgacatctatgatgaggatgagaaccagagccccagatcttttcagaagaagaccagacactacttcattgctgctgtggagaggctgtgggactatggcatgagcagcagccctcatgtgctgaggaacagggcccagtctggctctgtgccccagttcaagaaggtggtgttccaggagtttactgatggcagcttcacccagcccctgtacagaggggagctgaatgagcacctgggcctgctgggcccttatatcagggctgaggtggaggataacattatggtgactttcaggaaccaggcctctaggccctacagcttctatagcagcctgatctcttatgaggaggatcagaggcagggggctgagcccagaaagaactttgtgaagcctaatgagactaagacctacttctggaaggtccagcaccacatggcccccaccaaggatgagtttgattgcaaggcctgggcctatttctctgatgtggacctggagaaggatgtccattctggcctgattggccctctgctggtgtgccacactaacactctgaatcctgcccatggcaggcaggtgactgtccaggagtttgccctgttcttcactatctttgatgagaccaagagctggtactttactgagaacatggagagaaactgcagggctccttgcaatatccagatggaggaccccaccttcaaggagaactacaggtttcatgccatcaatgggtacatcatggacaccctgcctggcctggtgatggctcaggaccagagaatcagatggtatctgctgagcatgggcagcaatgagaatatccacagcatccacttctctggacatgtgttcactgtgaggaagaaggaggagtacaagatggctctgtataatctgtaccctggagtgtttgaaactgtggagatgctgccttctaaggctggcatctggagggtggagtgcctgattggggagcacctgcatgctggcatgagcaccctgttcctggtgtacagcaacaagtgtcagacccccctgggcatggcctctggacacatcagggacttccagatcacagcctctggccagtatggccagtgggcccccaagctggccaggctgcattattctggcagcatcaatgcctggtctaccaaggagccctttagctggatcaaggtggacctgctggcccccatgattatccatggcatcaagacccagggggccaggcagaagttctctagcctgtacatcagccagttcatcatcatgtactctctggatggcaagaagtggcagacctacaggggcaacagcactggcacactgatggtgttctttggcaatgtggacagctctggcatcaagcacaacatcttcaatccccccattatcgctaggtatattaggctgcatcccacccactacagcatcagatctaccctgagaatggagctgatgggctgtgacctgaactcttgcagcatgcccctgggcatggagtctaaggccatctctgatgcccagattactgccagcagctacttcaccaatatgtttgccacctggagcccttctaaggccaggctgcatctgcaggggaggagcaatgcctggaggcctcaggtgaacaaccctaaggagtggctgcaggtggatttccagaagaccatgaaggtgactggagtgaccacccagggagtcaagagcctgctgaccagcatgtatgtgaaggagtttctgatcagctctagccaggatggccaccagtggactctgttctttcagaatgggaaggtgaaggtgtttcagggcaatcaggactctttcacccctgtggtgaacagcctggacccccccctgctgaccagatacctgagaatccacccccagagctgggtgcaccagatcgccctgaggatggaggtgctgggctgtgaggctcaggatctgtactga

SEQ ID NO: 18 - DNA, 4620 bp, synthetic construct
  source 1..4620: mol_type = other DNA
gccaccaggaggtactacctgggggctgtggagctgagctgggactacatgcagtctgacctgggggagctgcctgtggatgctaggttcccccctagagtgcccaagtccttccccttcaacacttctgtggtgtacaagaagaccctgtttgtggagttcactgaccacctgtttaacattgccaagcccaggcccccttggatgggcctgctggggcccaccatccaggctgaggtgtatgacactgtggtgatcaccctgaagaacatggccagccatcctgtgagcctgcatgctgtgggggtgagctactggaaggccagcgagggggctgagtatgatgaccagactagccagagggagaaggaggatgacaaggtgtttcctggaggcagccacacctatgtgtggcaggtgctgaaggagaatggccccatggcctctgaccccctgtgcctgacctacagctacctgagccatgtggatctggtgaaggacctgaactctggcctgattggggctctgctggtgtgtagagagggcagcctggctaaggagaagacccagaccctgcataagttcatcctgctgtttgctgtgtttgatgagggcaagagctggcactctgagaccaagaacagcctgatgcaggatagggatgctgcctctgccagggcttggcccaagatgcacactgtgaatggctatgtgaataggagcctgcctggcctgattggctgccacaggaagtctgtgtactggcatgtgattggaatgggcacaacccctgaggtccatagcatcttcctggagggccacactttcctggtgaggaaccacagacaggcctctctggagattagccccatcaccttcctgactgctcagactctgctgatggacctgggccagttcctgctgttttgccatattagctctcaccagcatgatggcatggaggcctatgtgaaggtggacagctgccctgaggagcctcagctgaggatgaagaacaatgaggaggctgaagactatgatgatgacctgactgattctgagatggatgtggtgaggtttgatgatgacaatagccccagcttcattcagatcagatctgtggccaaaaagcaccccaagacctgggtgcattacattgctgctgaagaggaggactgggactatgcccctctggtgctggcccctgatgataggagctataagagccagtacctgaacaatgggccccagaggattggcagaaagtacaagaaggtgaggttcatggcttacactgatgaaaccttcaaaaccagggaggccatccagcatgagtctggcatcctgggccctctgctgtatggagaggtgggagacaccctgctgatcatcttcaagaaccaggccagcaggccctacaacatctatcctcatggcatcactgatgtgagacctctgtacagcaggaggctgcctaagggggtgaaacacctgaaggactttcccatcctgcctggggagatcttcaagtataagtggactgtgactgtggaggatggccctaccaagtctgaccccaggtgtctgacaaggtattacagcagctttgtgaacatggagagggacctggcctctggcctgattggccctctgctgatctgctacaaggagtctgtggaccagaggggcaaccagatcatgtctgacaagaggaatgtgatcctgttctctgtgtttgatgagaataggagctggtatctgactgagaacatccagagattcctgcccaatcctgctggggtgcagctggaggaccctgagtttcaggccagcaatatcatgcacagcatcaatggctatgtgtttgacagcctgcagctgtctgtgtgcctgcatgaggtggcctactggtacatcctgagcattggagcccagactgattttctgtctgtgttcttttctggctataccttcaagcacaagatggtgtatgaggacaccctgaccctgttccccttctctggggagactgtgttcatgtctatggagaatcctgggctgtggattctgggctgccacaactctgatttcaggaacaggggcatgactgccctgctgaaggtgagcagctgtgacaagaacactggggactactatgaggatagctatgaggacatttctgcttatctgctgtctaagaataatgccattgagcccaggagcttcagccagaatagcagacaccctagcaccagacagaaacagtttaatgccactaatgtgagcaacaacagcaacaccagcaatgacagcaatgtgtctaacaagacatctaacaacagcaatgccacaaacaagaccaacaacacaaatgatagcacaaacaggaccaaccagaccaataccagccagcagaacttcgtgacccagagacggaagagaggctctggcgccaccaactttagcctgctgaagcaggcaggcgacgtggaggagaatcctggaccaatgcagattgagctgagcacctgcttcttcctgtgtctgctgaggttctgcttctctgagatcaccaggactaccctgcagtctgatcaggaggagattgactatgatgacacaatctctgtggagatgaagaaggaggattttgacatctatgatgaggatgagaaccagagccccagatcttttcagaagaagaccagacactacttcattgctgctgtggagaggctgtgggactatggcatgagcagcagccctcatgtgctgaggaacagggcccagtctggctctgtgccccagttcaagaaggtggtgttccaggagtttactgatggcagcttcacccagcccctgtacagaggggagctgaatgagcacctgggcctgctgggcccttatatcagggctgaggtggaggataacattatggtgactttcaggaaccaggcctctaggccctacagcttctatagcagcctgatctcttatgaggaggatcagaggcagggggctgagcccagaaagaactttgtgaagcctaatgagactaagacctacttctggaaggtccagcaccacatggcccccaccaaggatgagtttgattgcaaggcctgggcctatttctctgatgtggacctggagaaggatgtccattctggcctgattggccctctgctggtgtgccacactaacactctgaatcctgcccatggcaggcaggtgactgtccaggagtttgccctgttcttcactatctttgatgagaccaagagctggtactttactgagaacatggagagaaactgcagggctccttgcaatatccagatggaggaccccaccttcaaggagaactacaggtttcatgccatcaatgggtacatcatggacaccctgcctggcctggtgatggctcaggaccagagaatcagatggtatctgctgagcatgggcagcaatgagaatatccacagcatccacttctctggacatgtgttcactgtgaggaagaaggaggagtacaagatggctctgtataatctgtaccctggagtgtttgaaactgtggagatgctgccttctaaggctggcatctggagggtggagtgcctgattggggagcacctgcatgctggcatgagcaccctgttcctggtgtacagcaacaagtgtcagacccccctgggcatggcctctggacacatcagggacttccagatcacagcctctggccagtatggccagtgggcccccaagctggccaggctgcattattctggcagcatcaatgcctggtctaccaaggagccctttagctggatcaaggtggacctgctggcccccatgattatccatggcatcaagacccagggggccaggcagaagttctctagcctgtacatcagccagttcatcatcatgtactctctggatggcaagaagtggcagacctacaggggcaacagcactggcacactgatggtgttctttggcaatgtggacagctctggcatcaagcacaacatcttcaatccccccattatcgctaggtatattaggctgcatcccacccactacagcatcagatctaccctgagaatggagctgatgggctgtgacctgaactcttgcagcatgcccctgggcatggagtctaaggccatctctgatgcccagattactgccagcagctacttcaccaatatgtttgccacctggagcccttctaaggccaggctgcatctgcaggggaggagcaatgcctggaggcctcaggtgaacaaccctaaggagtggctgcaggtggatttccagaagaccatgaaggtgactggagtgaccacccagggagtcaagagcctgctgaccagcatgtatgtgaaggagtttctgatcagctctagccaggatggccaccagtggactctgttctttcagaatgggaaggtgaaggtgtttcagggcaatcaggactctttcacccctgtggtgaacagcctggacccccccctgctgaccagatacctgagaatccacccccagagctgggtgcaccagatcgccctgaggatggaggtgctgggctgtgaggctcaggatctgtactga

SEQ ID NO: 19 - DNA, 5310 bp, synthetic construct
  source 1..5310: mol_type = other DNA
gccaccaggaggtactacctgggggctgtggagctgagctgggactacatgcagtctgacctgggggagctgcctgtggatgctaggttcccccctagagtgcccaagtccttccccttcaacacttctgtggtgtacaagaagaccctgtttgtggagttcactgaccacctgtttaacattgccaagcccaggcccccttggatgggcctgctggggcccaccatccaggctgaggtgtatgacactgtggtgatcaccctgaagaacatggccagccatcctgtgagcctgcatgctgtgggggtgagctactggaaggccagcgagggggctgagtatgatgaccagactagccagagggagaaggaggatgacaaggtgtttcctggaggcagccacacctatgtgtggcaggtgctgaaggagaatggccccatggcctctgaccccctgtgcctgacctacagctacctgagccatgtggatctggtgaaggacctgaactctggcctgattggggctctgctggtgtgtagagagggcagcctggctaaggagaagacccagaccctgcataagttcatcctgctgtttgctgtgtttgatgagggcaagagctggcactctgagaccaagaacagcctgatgcaggatagggatgctgcctctgccagggcttggcccaagatgcacactgtgaatggctatgtgaataggagcctgcctggcctgattggctgccacaggaagtctgtgtactggcatgtgattggaatgggcacaacccctgaggtccatagcatcttcctggagggccacactttcctggtgaggaaccacagacaggcctctctggagattagccccatcaccttcctgactgctcagactctgctgatggacctgggccagttcctgctgttttgccatattagctctcaccagcatgatggcatggaggcctatgtgaaggtggacagctgccctgaggagcctcagctgaggatgaagaacaatgaggaggctgaagactatgatgatgacctgactgattctgagatggatgtggtgaggtttgatgatgacaatagccccagcttcattcagatcagatctgtggccaaaaagcaccccaagacctgggtgcattacattgctgctgaagaggaggactgggactatgcccctctggtgctggcccctgatgataggagctataagagccagtacctgaacaatgggccccagaggattggcagaaagtacaagaaggtgaggttcatggcttacactgatgaaaccttcaaaaccagggaggccatccagcatgagtctggcatcctgggccctctgctgtatggagaggtgggagacaccctgctgatcatcttcaagaaccaggccagcaggccctacaacatctatcctcatggcatcactgatgtgagacctctgtacagcaggaggctgcctaagggggtgaaacacctgaaggactttcccatcctgcctggggagatcttcaagtataagtggactgtgactgtggaggatggccctaccaagtctgaccccaggtgtctgacaaggtattacagcagctttgtgaacatggagagggacctggcctctggcctgattggccctctgctgatctgctacaaggagtctgtggaccagaggggcaaccagatcatgtctgacaagaggaatgtgatcctgttctctgtgtttgatgagaataggagctggtatctgactgagaacatccagagattcctgcccaatcctgctggggtgcagctggaggaccctgagtttcaggccagcaatatcatgcacagcatcaatggctatgtgtttgacagcctgcagctgtctgtgtgcctgcatgaggtggcctactggtacatcctgagcattggagcccagactgattttctgtctgtgttcttttctggctataccttcaagcacaagatggtgtatgaggacaccctgaccctgttccccttctctggggagactgtgttcatgtctatggagaatcctgggctgtggattctgggctgccacaactctgatttcaggaacaggggcatgactgccctgctgaaggtgagcagctgtgacaagaacactggggactactatgaggatagctatgaggacatttctgcttatctgctgtctaagaataatgccattgagcccaggagcttcagccagaatagcagacaccctagcaccagacagaaacagtttaatgccactaatgtgagcaacaacagcaacaccagcaatgacagcaatgtgtctaacaagacatctaacaacagcaatgccacaaacaagaccaacaacacaaatgatagcacaaacaggaccaaccagaccaataccagcccccctgtgctgaagagacatcagagggagatcaccaggactaccctgcagtctgatcaggaggagattgactatgatgacacaatctctgtggagatgaagaaggaggattttgacatctatgatgaggatgagaaccagagccccagatcttttcagaagaagaccagacactacttcattgctgctgtggagaggctgtgggactatggcatgagcagcagccctcatgtgctgaggaacagggcccagtctggctctgtgccccagttcaagaaggtggtgttccaggagtttactgatggcagcttcacccagcccctgtacagaggggagctgaatgagcacctgggcctgctgggcccttatatcagggctgaggtggaggataacattatggtgactttcaggaaccaggcctctaggccctacagcttctatagcagcctgatctcttatgaggaggatcagaggcagggggctgagcccagaaagaactttgtgaagcctaatgagactaagacctacttctggaaggtccagcaccacatggcccccaccaaggatgagtttgattgcaaggcctgggcctatttctctgatgtggacctggagaaggatgtccattctggcctgattggccctctgctggtgtgccacactaacactctgaatcctgcccatggcaggcaggtgactgtccaggagtttgccctgttcttcactatctttgatgagaccaagagctggtactttactgagaacatggagagaaactgcagggctccttgcaatatccagatggaggaccccaccttcaaggagaactacaggtttcatgccatcaatgggtacatcatggacaccctgcctggcctggtgatggctcaggaccagagaatcagatggtatctgctgagcatgggcagcaatgagaatatccacagcatccacttctctggacatgtgttcactgtgaggaagaaggaggagtacaagatggctctgtataatctgtaccctggagtgtttgaaactgtggagatgctgccttctaaggctggcatctggagggtggagtgcctgattggggagcacctgcatgctggcatgagcaccctgttcctggtgtacagcaacaagtgtcagacccccctgggcatggcctctggacacatcagggacttccagatcacagcctctggccagtatggccagtgggcccccaagctggccaggctgcattattctggcagcatcaatgcctggtctaccaaggagccctttagctggatcaaggtggacctgctggcccccatgattatccatggcatcaagacccagggggccaggcagaagttctctagcctgtacatcagccagttcatcatcatgtactctctggatggcaagaagtggcagacctacaggggcaacagcactggcacactgatggtgttctttggcaatgtggacagctctggcatcaagcacaacatcttcaatccccccattatcgctaggtatattaggctgcatcccacccactacagcatcagatctaccctgagaatggagctgatgggctgtgacctgaactcttgcagcatgcccctgggcatggagtctaaggccatctctgatgcccagattactgccagcagctacttcaccaatatgtttgccacctggagcccttctaaggccaggctgcatctgcaggggaggagcaatgcctggaggcctcaggtgaacaaccctaaggagtggctgcaggtggatttccagaagaccatgaaggtgactggagtgaccacccagggagtcaagagcctgctgaccagcatgtatgtgaaggagtttctgatcagctctagccaggatggccaccagtggactctgttctttcagaatgggaaggtgaaggtgtttcagggcaatcaggactctttcacccctgtggtgaacagcctggacccccccctgctgaccagatacctgagaatccacccccagagctgggtgcaccagatcgccctgaggatggaggtgctgggctgtgaggctcaggatctgtacggaggcggaggctctggaggaggcggctccggcggaggaggctctagctcaagttccaaagctcctcctccaagtctgccatctccaagcaggctccccggaccatccgatacccctattctgccacaagccgagtctaagtatggcccaccttgtcctccatgtcctgcccctccagtggctggaggaccttctgtgtttctgtttcccccaaagccaaaagatacactgatgatttctcgcactcctgaggtgacttgcgtggtggtggctgtgagccaggaggatcccgaggtgcagttcaactggtacgtggacggcgtggaggtgcacaacgccaagaccaagcccagagaggagcaattcaactccacctacagagtggtgagcgtgctcaccgtggtgcaccaggattggctgaatggcaaggaatacaaatgtaaggtgagcaataagggactgccaagtagcattgaaaaaacaatttctaaagctaaaggacagccaagagaaccccaggtttatactcttcccccctcccaggaggagatgaccaagaaccaggtgagcctgacctgcctggtgaagggcttttacccctccgacatcgccgtggagtgggagagcaacggccagcccgagaacaactacaagaccaccccccccgtgctggacagcgacggcagcttctttctgtattctaaacttacagtcgataaaagcagatggcaggaaggaaatgtgtttagctgtagcgtgatgcatgaagccctgcacaatcattacacgcagaaatccctgagcctgagcttaggtaaatga

SEQ ID NO: 20 - protein, 1769 aa, synthetic construct
ATRRYYLGAVELSWDYMQSDLGELPVDARFPPRVPKSFPFNTSVVYKKTLFVEFTDHLFNIAKPRPPWMGLLGPTIQAEVYDTVVITLKNMASHPVSLHAVGVSYWKASEGAEYDDQTSQREKEDDKVFPGGSHTYVWQVLKENGPMASDPLCLTYSYLSHVDLVKDLNSGLIGALLVCREGSLAKEKTQTLHKFILLFAVFDEGKSWHSETKNSLMQDRDAASARAWPKMHTVNGYVNRSLPGLIGCHRKSVYWHVIGMGTTPEVHSIFLEGHTFLVRNHRQASLEISPITFLTAQTLLMDLGQFLLFCHISSHQHDGMEAYVKVDSCPEEPQLRMKNNEEAEDYDDDLTDSEMDVVRFDDDNSPSFIQIRSVAKKHPKTWVHYIAAEEEDWDYAPLVLAPDDRSYKSQYLNNGPQRIGRKYKKVRFMAYTDETFKTREAIQHESGILGPLLYGEVGDTLLIIFKNQASRPYNIYPHGITDVRPLYSRRLPKGVKHLKDFPILPGEIFKYKWTVTVEDGPTKSDPRCLTRYYSSFVNMERDLASGLIGPLLICYKESVDQRGNQIMSDKRNVILFSVFDENRSWYLTENIQRFLPNPAGVQLEDPEFQASNIMHSINGYVFDSLQLSVCLHEVAYWYILSIGAQTDFLSVFFSGYTFKHKMVYEDTLTLFPFSGETVFMSMENPGLWILGCHNSDFRNRGMTALLKVSSCDKNTGDYYEDSYEDISAYLLSKNNAIEPRSFSQNSRHPSTRQKQFNATNVSNNSNTSNDSNVSNKTSNNSNATNKTNNTNDSTNRTNQTNTSPPVLKRHQREITRTTLQSDQEEIDYDDTISVEMKKEDFDIYDEDENQSPRSFQKKTRHYFIAAVERLWDYGMSSSPHVLRNRAQSGSVPQFKKVVFQEFTDGSFTQPLYRGELNEHLGLLGPYIRAEVEDNIMVTFRNQASRPYSFYSSLISYEEDQRQGAEPRKNFVKPNETKTYFWKVQHHMAPTKDEFDCKAWAYFSDVDLEKDVHSGLIGPLLVCHTNTLNPAHGRQVTVQEFALFFTIFDETKSWYFTENMERNCRAPCNIQMEDPTFKENYRFHAINGYIMDTLPGLVMAQDQRIRWYLLSMGSNENIHSIHFSGHVFTVRKKEEYKMALYNLYPGVFETVEMLPSKAGIWRVECLIGEHLHAGMSTLFLVYSNKCQTPLGMASGHIRDFQITASGQYGQWAPKLARLHYSGSINAWSTKEPFSWIKVDLLAPMIIHGIKTQGARQKFSSLYISQFIIMYSLDGKKWQTYRGNSTGTLMVFFGNVDSSGIKHNIFNPPIIARYIRLHPTHYSIRSTLRMELMGCDLNSCSMPLGMESKAISDAQITASSYFTNMFATWSPSKARLHLQGRSNAWRPQVNNPKEWLQVDFQKTMKVTGVTTQGVKSLLTSMYVKEFLISSSQDGHQWTLFFQNGKVKVFQGNQDSFTPVVNSLDPPLLTRYLRIHPQSWVHQIALRMEVLGCEAQDLYGGGGSGGGGSGGGGSSSSSKAPPPSLPSPSRLPGPSDTPILPQAESKYGPPCPPCPAPPVAGGPSVFLFPPKPKDTLMISRTPEVTCVVVAVSQEDPEVQFNWYVDGVEVHNAKTKPREEQFNSTYRVVSVLTVVHQDWLNGKEYKCKVSNKGLPSSIEKTISKAKGQPREPQVYTLPPSQEEMTKNQVSLTCLVKGFYPSDIAVEWESNGQPENNYKTTPPVLDSDGSFFLYSKLTVDKSRWQEGNVFSCSVMHEALHNHYTQKSLSLSLGK

SEQ ID NO: 21 - protein, 1496 aa, synthetic construct
ATRRYYLGAVELSWDYMQSDLGELPVDARFPPRVPKSFPFNTSVVYKKTLFVEFTDHLFNIAKPRPPWMGLLGPTIQAEVYDTVVVTLKNMASHPVSLHAVGVSYWKSSEGAEYDDQTSQREKEDDKVFPGKSHTYVWQVLKENGPTASDPPCLTYSYLSHVDLVKDLNSGLIGALLVCREGSLAKEKTQTLHKFILLFAVFDEGKSWHSETKNSLMQDRDAASARAWPKMHTVNGYVNRSLPGLIGCHRKSVYWHVIGMGTTPEVHSIFLEGHTFLVRNHRQASLEISPITFLTAQTLLMDLGQFLLFCHISSHQHDGMEAYVKVDSCPEEPQLRMKNNEEAEDYDDDLTDSEMDVVRFDDDNSPSFIQIRSVAKKHPKTWVHYIAAEEEDWDYAPLVLAPDDRSYKSQYLNNGPQRIGRKYKKVRFMAYTDETFKTREAIQHESGILGPLLYGEVGDTLLIIFKNQASRPYNIYPHGITDVRPLYSRRLPKGVKHLKDFPILPGEIFKYKWTVTVEDGPTKSDPRCLTRYYSSFVNMERDLASGLIGPLLICYKESVDQRGNQIMSDKRNVILFSVFDENRSWYLTENIQRFLPNPAGVQLEDPEFQASNIMHSINGYVFDSLQLSVCLHEVAYWYILSIGAQTDFLSVFFSGYTFKHKMVYEDTLTLFPFSGETVFMSMENPGLWILGCHNSDFRNRGMTALLKVSSCDKNTGDYYEDSYEDISAYLLSKNNAIEPRSFSQNSRHPSTRQKQFNATNVSNNSNTSNDSNVSNKTSNNSNATNKTNNTNDSTNRTNQTNTSPPVLKRHQREITRTTLQSDQEEIDYDDTISVEMKKEDFDIYDEDENQSPRSFQKKTRHYFIAAVERLWDYGMSSSPHVLRNRAQSGSVPQFKKVVFQEFTDGSFTQPLYRGELNEHLGLLGPYIRAEVEDNIMVTFRNQASRPYSFYSSLISYEEDQRQGAEPRKNFVKPNETKTYFWKVQHHMAPTKDEFDCKAWAYFSDVDLEKDVHSGLIGPLLVCHTNTLNPAHGRQVTVQEFALFFTIFDETKSWYFTENMERNCRAPCNIQMEDPTFKENYRFHAINGYIMDTLPGLVMAQDQRIRWYLLSMGSNENIHSIHFSGHVFTVRKKEEYKMALYNLYPGVFETVEMLPSKAGIWRVECLIGEHLHAGMSTLFLVYSNKCQTPLGMASGHIRDFQITASGQYGQWAPKLARLHYSGSINAWSTKEPFSWIKVDLLAPMIIHGIKTQGARQKFSSLYISQFIIMYSLDGKKWQTYRGNSTGTLMVFFGNVDSSGIKHNIFNPPIIARYIRLHPTHYSIRSTLRMELMGCDLNSCSMPLGMESKAISDAQITASSYFTNMFATWSPSKARLHLQGRSNAWRPQVNNPKEWLQVDFQKTMKVTGVTTQGVKSLLTSMYVKEFLISSSQDGHQWTLFFQNGKVKVFQGNQDSFTPVVNSLDPPLLTRYLRIHPQSWVHQIALRMEVLGCEAQDLY

SEQ ID NO: 22 - DNA, 4491 bp, synthetic construct
  source 1..4491: mol_type = other DNA
gccaccaggaggtactacctgggggctgtggagctgagctgggactacatgcagtctgacctgggggagctgcctgtggatgctaggttcccccctagagtgcccaagtccttccccttcaacacttctgtggtgtacaagaagaccctgtttgtggagttcactgaccacctgtttaacattgccaagcccaggcccccttggatgggcctgctggggcccaccatccaggctgaggtgtatgacactgtggtggtgaccctgaagaacatggccagccatcctgtgagcctgcatgctgtgggggtgagctactggaagagcagcgagggggctgagtatgatgaccagactagccagagggagaaggaggatgacaaggtgtttcctggaaagagccacacctatgtgtggcaggtgctgaaggagaatggccccacagcctctgaccccccttgcctgacctacagctacctgagccatgtggatctggtgaaggacctgaactctggcctgattggggctctgctggtgtgtagagagggcagcctggctaaggagaagacccagaccctgcataagttcatcctgctgtttgctgtgtttgatgagggcaagagctggcactctgagaccaagaacagcctgatgcaggatagggatgctgcctctgccagggcttggcccaagatgcacactgtgaatggctatgtgaataggagcctgcctggcctgattggctgccacaggaagtctgtgtactggcatgtgattggaatgggcacaacccctgaggtccatagcatcttcctggagggccacactttcctggtgaggaaccacagacaggcctctctggagattagccccatcaccttcctgactgctcagactctgctgatggacctgggccagttcctgctgttttgccatattagctctcaccagcatgatggcatggaggcctatgtgaaggtggacagctgccctgaggagcctcagctgaggatgaagaacaatgaggaggctgaagactatgatgatgacctgactgattctgagatggatgtggtgaggtttgatgatgacaatagccccagcttcattcagatcagatctgtggccaaaaagcaccccaagacctgggtgcattacattgctgctgaagaggaggactgggactatgcccctctggtgctggcccctgatgataggagctataagagccagtacctgaacaatgggccccagaggattggcagaaagtacaagaaggtgaggttcatggcttacactgatgaaaccttcaaaaccagggaggccatccagcatgagtctggcatcctgggccctctgctgtatggagaggtgggagacaccctgctgatcatcttcaagaaccaggccagcaggccctacaacatctatcctcatggcatcactgatgtgagacctctgtacagcaggaggctgcctaagggggtgaaacacctgaaggactttcccatcctgcctggggagatcttcaagtataagtggactgtgactgtggaggatggccctaccaagtctgaccccaggtgtctgacaaggtattacagcagctttgtgaacatggagagggacctggcctctggcctgattggccctctgctgatctgctacaaggagtctgtggaccagaggggcaaccagatcatgtctgacaagaggaatgtgatcctgttctctgtgtttgatgagaataggagctggtatctgactgagaacatccagagattcctgcccaatcctgctggggtgcagctggaggaccctgagtttcaggccagcaatatcatgcacagcatcaatggctatgtgtttgacagcctgcagctgtctgtgtgcctgcatgaggtggcctactggtacatcctgagcattggagcccagactgattttctgtctgtgttcttttctggctataccttcaagcacaagatggtgtatgaggacaccctgaccctgttccccttctctggggagactgtgttcatgtctatggagaatcctgggctgtggattctgggctgccacaactctgatttcaggaacaggggcatgactgccctgctgaaggtgagcagctgtgacaagaacactggggactactatgaggatagctatgaggacatttctgcttatctgctgtctaagaataatgccattgagcccaggagcttcagccagaatagcagacaccctagcaccagacagaaacagtttaatgccactaatgtgagcaacaacagcaacaccagcaatgacagcaatgtgtctaacaagacatctaacaacagcaatgccacaaacaagaccaacaacacaaatgatagcacaaacaggaccaaccagaccaataccagcccccctgtgctgaagagacatcagagggagatcaccaggactaccctgcagtctgatcaggaggagattgactatgatgacacaatctctgtggagatgaagaaggaggattttgacatctatgatgaggatgagaaccagagccccagatcttttcagaagaagaccagacactacttcattgctgctgtggagaggctgtgggactatggcatgagcagcagccctcatgtgctgaggaacagggcccagtctggctctgtgccccagttcaagaaggtggtgttccaggagtttactgatggcagcttcacccagcccctgtacagaggggagctgaatgagcacctgggcctgctgggcccttatatcagggctgaggtggaggataacattatggtgactttcaggaaccaggcctctaggccctacagcttctatagcagcctgatctcttatgaggaggatcagaggcagggggctgagcccagaaagaactttgtgaagcctaatgagactaagacctacttctggaaggtccagcaccacatggcccccaccaaggatgagtttgattgcaaggcctgggcctatttctctgatgtggacctggagaaggatgtccattctggcctgattggccctctgctggtgtgccacactaacactctgaatcctgcccatggcaggcaggtgactgtccaggagtttgccctgttcttcactatctttgatgagaccaagagctggtactttactgagaacatggagagaaactgcagggctccttgcaatatccagatggaggaccccaccttcaaggagaactacaggtttcatgccatcaatgggtacatcatggacaccctgcctggcctggtgatggctcaggaccagagaatcagatggtatctgctgagcatgggcagcaatgagaatatccacagcatccacttctctggacatgtgttcactgtgaggaagaaggaggagtacaagatggctctgtataatctgtaccctggagtgtttgaaactgtggagatgctgccttctaaggctggcatctggagggtggagtgcctgattggggagcacctgcatgctggcatgagcaccctgttcctggtgtacagcaacaagtgtcagacccccctgggcatggcctctggacacatcagggacttccagatcacagcctctggccagtatggccagtgggcccccaagctggccaggctgcattattctggcagcatcaatgcctggtctaccaaggagccctttagctggatcaaggtggacctgctggcccccatgattatccatggcatcaagacccagggggccaggcagaagttctctagcctgtacatcagccagttcatcatcatgtactctctggatggcaagaagtggcagacctacaggggcaacagcactggcacactgatggtgttctttggcaatgtggacagctctggcatcaagcacaacatcttcaatccccccattatcgctaggtatattaggctgcatcccacccactacagcatcagatctaccctgagaatggagctgatgggctgtgacctgaactcttgcagcatgcccctgggcatggagtctaaggccatctctgatgcccagattactgccagcagctacttcaccaatatgtttgccacctggagcccttctaaggccaggctgcatctgcaggggaggagcaatgcctggaggcctcaggtgaacaaccctaaggagtggctgcaggtggatttccagaagaccatgaaggtgactggagtgaccacccagggagtcaagagcctgctgaccagcatgtatgtgaaggagtttctgatcagctctagccaggatggccaccagtggactctgttctttcagaatgggaaggtgaaggtgtttcagggcaatcaggactctttcacccctgtggtgaacagcctggacccccccctgctgaccagatacctgagaatccacccccagagctgggtgcaccagatcgccctgaggatggaggtgctgggctgtgaggctcaggatctgtactga

SEQ ID NO: 23 - protein, 1498 aa, synthetic construct
ATRRYYLGAVELSWDYMQSDLGELPVDARFPPRVPKSFPFNTSVVYKKTLFVEFTDHLFNIAKPRPPWMGLLGPTIQAEVYDTVVVTLKNMASHPVSLHAVGVSYWKSSEGAEYDDQTSQREKEDDKVFPGKSHTYVWQVLKENGPTASDPPCLTYSYLSHVDLVKDLNSGLIGALLVCREGSLAKEKTQTLHKFILLFAVFDEGKSWHSETKNSLMQDRDAASARAWPKMHTVNGYVNRSLPGLIGCHRKSVYWHVIGMGTTPEVHSIFLEGHTFLVRNHRQASLEISPITFLTAQTLLMDLGQFLLFCHISSHQHDGMEAYVKVDSCPEEPQLRMKNNEEAEDYDDDLTDSEMDVVRFDDDNSPSFIQIRSVAKKHPKTWVHYIAAEEEDWDYAPLVLAPDDRSYKSQYLNNGPQRIGRKYKKVRFMAYTDETFKTREAIQHESGILGPLLYGEVGDTLLIIFKNQASRPYNIYPHGITDVRPLYSRRLPKGVKHLKDFPILPGEIFKYKWTVTVEDGPTKSDPRCLTRYYSSFVNMERDLASGLIGPLLICYKESVDQRGNQIMSDKRNVILFSVFDENRSWYLTENIQRFLPNPAGVQLEDPEFQASNIMHSINGYVFDSLQLSVCLHEVAYWYILSIGAQTDFLSVFFSGYTFKHKMVYEDTLTLFPFSGETVFMSMENPGLWILGCHNSDFRNRGMTALLKVSSCDKNTGDYYEDSYEDISAYLLSKNNAIEPRSFSQNSRHPSTRQKQFNATNVSNNSNTSNDSNVSNKTSNNSNATNKTNNTNDSTNRTNQTNTSQQNFVTQRSKREITRTTLQSDQEEIDYDDTISVEMKKEDFDIYDEDENQSPRSFQKKTRHYFIAAVERLWDYGMSSSPHVLRNRAQSGSVPQFKKVVFQEFTDGSFTQPLYRGELNEHLGLLGPYIRAEVEDNIMVTFRNQASRPYSFYSSLISYEEDQRQGAEPRKNFVKPNETKTYFWKVQHHMAPTKDEFDCKAWAYFSDVDLEKDVHSGLIGPLLVCHTNTLNPAHGRQVTVQEFALFFTIFDETKSWYFTENMERNCRAPCNIQMEDPTFKENYRFHAINGYIMDTLPGLVMAQDQRIRWYLLSMGSNENIHSIHFSGHVFTVRKKEEYKMALYNLYPGVFETVEMLPSKAGIWRVECLIGEHLHAGMSTLFLVYSNKCQTPLGMASGHIRDFQITASGQYGQWAPKLARLHYSGSINAWSTKEPFSWIKVDLLAPMIIHGIKTQGARQKFSSLYISQFIIMYSLDGKKWQTYRGNSTGTLMVFFGNVDSSGIKHNIFNPPIIARYIRLHPTHYSIRSTLRMELMGCDLNSCSMPLGMESKAISDAQITASSYFTNMFATWSPSKARLHLQGRSNAWRPQVNNPKEWLQVDFQKTMKVTGVTTQGVKSLLTSMYVKEFLISSSQDGHQWTLFFQNGKVKVFQGNQDSFTPVVNSLDPPLLTRYLRIHPQSWVHQIALRMEVLGCEAQDLY

SEQ ID NO: 24 - DNA, 4497 bp, synthetic construct
  source 1..4497: mol_type = other DNA
gccaccaggaggtactacctgggggctgtggagctgagctgggactacatgcagtctgacctgggggagctgcctgtggatgctaggttcccccctagagtgcccaagtccttccccttcaacacttctgtggtgtacaagaagaccctgtttgtggagttcactgaccacctgtttaacattgccaagcccaggcccccttggatgggcctgctggggcccaccatccaggctgaggtgtatgacactgtggtggtgaccctgaagaacatggccagccatcctgtgagcctgcatgctgtgggggtgagctactggaagagcagcgagggggctgagtatgatgaccagactagccagagggagaaggaggatgacaaggtgtttcctggaaagagccacacctatgtgtggcaggtgctgaaggagaatggccccacagcctctgaccccccttgcctgacctacagctacctgagccatgtggatctggtgaaggacctgaactctggcctgattggggctctgctggtgtgtagagagggcagcctggctaaggagaagacccagaccctgcataagttcatcctgctgtttgctgtgtttgatgagggcaagagctggcactctgagaccaagaacagcctgatgcaggatagggatgctgcctctgccagggcttggcccaagatgcacactgtgaatggctatgtgaataggagcctgcctggcctgattggctgccacaggaagtctgtgtactggcatgtgattggaatgggcacaacccctgaggtccatagcatcttcctggagggccacactttcctggtgaggaaccacagacaggcctctctggagattagccccatcaccttcctgactgctcagactctgctgatggacctgggccagttcctgctgttttgccatattagctctcaccagcatgatggcatggaggcctatgtgaaggtggacagctgccctgaggagcctcagctgaggatgaagaacaatgaggaggctgaagactatgatgatgacctgactgattctgagatggatgtggtgaggtttgatgatgacaatagccccagcttcattcagatcagatctgtggccaaaaagcaccccaagacctgggtgcattacattgctgctgaagaggaggactgggactatgcccctctggtgctggcccctgatgataggagctataagagccagtacctgaacaatgggccccagaggattggcagaaagtacaagaaggtgaggttcatggcttacactgatgaaaccttcaaaaccagggaggccatccagcatgagtctggcatcctgggccctctgctgtatggagaggtgggagacaccctgctgatcatcttcaagaaccaggccagcaggccctacaacatctatcctcatggcatcactgatgtgagacctctgtacagcaggaggctgcctaagggggtgaaacacctgaaggactttcccatcctgcctggggagatcttcaagtataagtggactgtgactgtggaggatggccctaccaagtctgaccccaggtgtctgacaaggtattacagcagctttgtgaacatggagagggacctggcctctggcctgattggccctctgctgatctgctacaaggagtctgtggaccagaggggcaaccagatcatgtctgacaagaggaatgtgatcctgttctctgtgtttgatgagaataggagctggtatctgactgagaacatccagagattcctgcccaatcctgctggggtgcagctggaggaccctgagtttcaggccagcaatatcatgcacagcatcaatggctatgtgtttgacagcctgcagctgtctgtgtgcctgcatgaggtggcctactggtacatcctgagcattggagcccagactgattttctgtctgtgttcttttctggctataccttcaagcacaagatggtgtatgaggacaccctgaccctgttccccttctctggggagactgtgttcatgtctatggagaatcctgggctgtggattctgggctgccacaactctgatttcaggaacaggggcatgactgccctgctgaaggtgagcagctgtgacaagaacactggggactactatgaggatagctatgaggacatttctgcttatctgctgtctaagaataatgccattgagcccaggagcttcagccagaattctagacaccctagcaccagacagaaacagtttaatgccactaatgtgtctaacaacagcaacaccagcaatgacagcaatgtgtctaacaagacatctaacaacagcaacgccacaaacaagaccaacaacacaaatgatagcacaaaccggaccaaccagaccaataccagccagcagaacttcgtgacccagagaagtaagagagagatcaccaggactaccctgcagtctgatcaggaggagattgactatgatgacacaatctctgtggagatgaagaaggaggattttgacatctatgatgaggatgagaaccagagccccagatcttttcagaagaagaccagacactacttcattgctgctgtggagaggctgtgggactatggcatgagcagcagccctcatgtgctgaggaacagggcccagtctggctctgtgccccagttcaagaaggtggtgttccaggagtttactgatggcagcttcacccagcccctgtacagaggggagctgaatgagcacctgggcctgctgggcccttatatcagggctgaggtggaggataacattatggtgactttcaggaaccaggcctctaggccctacagcttctatagcagcctgatctcttatgaggaggatcagaggcagggggctgagcccagaaagaactttgtgaagcctaatgagactaagacctacttctggaaggtccagcaccacatggcccccaccaaggatgagtttgattgcaaggcctgggcctatttctctgatgtggacctggagaaggatgtccattctggcctgattggccctctgctggtgtgccacactaacactctgaatcctgcccatggcaggcaggtgactgtccaggagtttgccctgttcttcactatctttgatgagaccaagagctggtactttactgagaacatggagagaaactgcagggctccttgcaatatccagatggaggaccccaccttcaaggagaactacaggtttcatgccatcaatgggtacatcatggacaccctgcctggcctggtgatggctcaggaccagagaatcagatggtatctgctgagcatgggcagcaatgagaatatccacagcatccacttctctggacatgtgttcactgtgaggaagaaggaggagtacaagatggctctgtataatctgtaccctggagtgtttgaaactgtggagatgctgccttctaaggctggcatctggagggtggagtgcctgattggggagcacctgcatgctggcatgagcaccctgttcctggtgtacagcaacaagtgtcagacccccctgggcatggcctctggacacatcagggacttccagatcacagcctctggccagtatggccagtgggcccccaagctggccaggctgcattattctggcagcatcaatgcctggtctaccaaggagccctttagctggatcaaggtggacctgctggcccccatgattatccatggcatcaagacccagggggccaggcagaagttctctagcctgtacatcagccagttcatcatcatgtactctctggatggcaagaagtggcagacctacaggggcaacagcactggcacactgatggtgttctttggcaatgtggacagctctggcatcaagcacaacatcttcaatccccccattatcgctaggtatattaggctgcatcccacccactacagcatcagatctaccctgagaatggagctgatgggctgtgacctgaactcttgcagcatgcccctgggcatggagtctaaggccatctctgatgcccagattactgccagcagctacttcaccaatatgtttgccacctggagcccttctaaggccaggctgcatctgcaggggaggagcaatgcctggaggcctcaggtgaacaaccctaaggagtggctgcaggtggatttccagaagaccatgaaggtgactggagtgaccacccagggagtcaagagcctgctgaccagcatgtatgtgaaggagtttctgatcagctctagccaggatggccaccagtggactctgttctttcagaatgggaaggtgaaggtgtttcagggcaatcaggactctttcacccctgtggtgaacagcctggacccccccctgctgaccagatacctgagaatccacccccagagctgggtgcaccagatcgccctgaggatggaggtgctgggctgtgaggctcaggatctgtactga

SEQ ID NO: 25 - DNA, 5928 bp, synthetic construct
  source 1..5928: mol_type = other DNA
ccccaactggggtaacctttgggctccccgggcgcgactagtgaattcgtcaatattggccattagccatattattcattggttatatagcataaatcaatattggctattggccattgcatacgttgtatctatatcataatatgtacatttatattggctcatgtccaatatgaccgccatgttggtgtggaaagtccccaggctccccagcaggcagaagtatgcaaagcatgcatctcaattagtcagcaaccaggcattgattattgactagttattaatagtaatcaattacggggtcattagttcatagcccatatatggagttccgcgttacataacttacggtaaatggcccgcctggctgaccgcccaacgacccccgcccattgacgtcaataatgacgtatgttcccatagtaacgccaatagggactttccattgacgtcaatgggtggagtatttacggtaaactgcccacttggcagtacatcaagtgtatcatatgccaagtccgccccctattgacgtcaatgacggtaaatggcccgcctggcattatgcccagtacatgaccttacgggactttcctacttggcagtacatctacgtattagtcatcgctattaccatggtgatgcggttttggcagtacaccaatgggcgtggatagcggtttgactcacggggatttccaagtctccaccccattgacgtcaatgggagtttgttttggcaccaaaatcaacgggactttccaaaatgtcgtaataaccccgccccgttgacgcaaatgggcggtaggcgtgtacggtgggaggtctatataagcagaggtcgtttagtgaaccgtcagatcactagtagctttattgcggtagtttatcacagttaaattgctaacgcagtcagtgctcgactgatcacaggtaagtatcaaggttacaagacaggtttaaggaggccaatagaaactgggcttgtcgagacagagaagattcttgcgtttctgataggcacctattggtcttactgacatccactttgcctttctctccacaggggtaccgaagccgctagcgctaccggtgccaccatgcagattgaactgagcacctgcttcttcctgtgtctgctgagattctgcttctctgccaccaggaggtactacctgggggctgtggagctgagctgggactacatgcagtctgacctgggggagctgcctgtggatgctaggttcccccctagagtgcccaagtccttccccttcaacacttctgtggtgtacaagaagaccctgtttgtggagttcactgaccacctgtttaacattgccaagcccaggcccccttggatgggcctgctggggcccaccatccaggctgaggtgtatgacactgtggtgatcaccctgaagaacatggccagccatcctgtgagcctgcatgctgtgggggtgagctactggaaggccagcgagggggctgagtatgatgaccagactagccagagggagaaggaggatgacaaggtgtttcctggaggcagccacacctatgtgtggcaggtgctgaaggagaatggccccatggcctctgaccccctgtgcctgacctacagctacctgagccatgtggatctggtgaaggacctgaactctggcctgattggggctctgctggtgtgtagagagggcagcctggctaaggagaagacccagaccctgcataagttcatcctgctgtttgctgtgtttgatgagggcaagagctggcactctgagaccaagaacagcctgatgcaggatagggatgctgcctctgccagggcttggcccaagatgcacactgtgaatggctatgtgaataggagcctgcctggcctgattggctgccacaggaagtctgtgtactggcatgtgattggaatgggcacaacccctgaggtccatagcatcttcctggagggccacactttcctggtgaggaaccacagacaggcctctctggagattagccccatcaccttcctgactgctcagactctgctgatggacctgggccagttcctgctgttttgccatattagctctcaccagcatgatggcatggaggcctatgtgaaggtggacagctgccctgaggagcctcagctgaggatgaagaacaatgaggaggctgaagactatgatgatgacctgactgattctgagatggatgtggtgaggtttgatgatgacaatagccccagcttcattcagatcagatctgtggccaaaaagcaccccaagacctgggtgcattacattgctgctgaagaggaggactgggactatgcccctctggtgctggcccctgatgataggagctataagagccagtacctgaacaatgggccccagaggattggcagaaagtacaagaaggtgaggttcatggcttacactgatgaaaccttcaaaaccagggaggccatccagcatgagtctggcatcctgggccctctgctgtatggagaggtgggagacaccctgctgatcatcttcaagaaccaggccagcaggccctacaacatctatcctcatggcatcactgatgtgagacctctgtacagcaggaggctgcctaagggggtgaaacacctgaaggactttcccatcctgcctggggagatcttcaagtataagtggactgtgactgtggaggatggccctaccaagtctgaccccaggtgtctgacaaggtattacagcagctttgtgaacatggagagggacctggcctctggcctgattggccctctgctgatctgctacaaggagtctgtggaccagaggggcaaccagatcatgtctgacaagaggaatgtgatcctgttctctgtgtttgatgagaataggagctggtatctgactgagaacatccagagattcctgcccaatcctgctggggtgcagctggaggaccctgagtttcaggccagcaatatcatgcacagcatcaatggctatgtgtttgacagcctgcagctgtctgtgtgcctgcatgaggtggcctactggtacatcctgagcattggagcccagactgattttctgtctgtgttcttttctggctataccttcaagcacaagatggtgtatgaggacaccctgaccctgttccccttctctggggagactgtgttcatgtctatggagaatcctgggctgtggattctgggctgccacaactctgatttcaggaacaggggcatgactgccctgctgaaggtgagcagctgtgacaagaacactggggactactatgaggatagctatgaggacatttctgcttatctgctgtctaagaataatgccattgagcccaggagcttcagccagaatagcagacaccctagcaccagacagaaacagtttaatgccactaatgtgagcaacaacagcaacaccagcaatgacagcaatgtgtctaacaagacatctaacaacagcaatgccacaaacaagaccaacaacacaaatgatagcacaaacaggaccaaccagaccaataccagcccccctgtgctgaagagacatcagagggagatcaccaggactaccctgcagtctgatcaggaggagattgactatgatgacacaatctctgtggagatgaagaaggaggattttgacatctatgatgaggatgagaaccagagccccagatcttttcagaagaagaccagacactacttcattgctgctgtggagaggctgtgggactatggcatgagcagcagccctcatgtgctgaggaacagggcccagtctggctctgtgccccagttcaagaaggtggtgttccaggagtttactgatggcagcttcacccagcccctgtacagaggggagctgaatgagcacctgggcctgctgggcccttatatcagggctgaggtggaggataacattatggtgactttcaggaaccaggcctctaggccctacagcttctatagcagcctgatctcttatgaggaggatcagaggcagggggctgagcccagaaagaactttgtgaagcctaatgagactaagacctacttctggaaggtccagcaccacatggcccccaccaaggatgagtttgattgcaaggcctgggcctatttctctgatgtggacctggagaaggatgtccattctggcctgattggccctctgctggtgtgccacactaacactctgaatcctgcccatggcaggcaggtgactgtccaggagtttgccctgttcttcactatctttgatgagaccaagagctggtactttactgagaacatggagagaaactgcagggctccttgcaatatccagatggaggaccccaccttcaaggagaactacaggtttcatgccatcaatgggtacatcatggacaccctgcctggcctggtgatggctcaggaccagagaatcagatggtatctgctgagcatgggcagcaatgagaatatccacagcatccacttctctggacatgtgttcactgtgaggaagaaggaggagtacaagatggctctgtataatctgtaccctggagtgtttgaaactgtggagatgctgccttctaaggctggcatctggagggtggagtgcctgattggggagcacctgcatgctggcatgagcaccctgttcctggtgtacagcaacaagtgtcagacccccctgggcatggcctctggacacatcagggacttccagatcacagcctctggccagtatggccagtgggcccccaagctggccaggctgcattattctggcagcatcaatgcctggtctaccaaggagccctttagctggatcaaggtggacctgctggcccccatgattatccatggcatcaagacccagggggccaggcagaagttctctagcctgtacatcagccagttcatcatcatgtactctctggatggcaagaagtggcagacctacaggggcaacagcactggcacactgatggtgttctttggcaatgtggacagctctggcatcaagcacaacatcttcaatccccccattatcgctaggtatattaggctgcatcccacccactacagcatcagatctaccctgagaatggagctgatgggctgtgacctgaactcttgcagcatgcccctgggcatggagtctaaggccatctctgatgcccagattactgccagcagctacttcaccaatatgtttgccacctggagcccttctaaggccaggctgcatctgcaggggaggagcaatgcctggaggcctcaggtgaacaaccctaaggagtggctgcaggtggatttccagaagaccatgaaggtgactggagtgaccacccagggagtcaagagcctgctgaccagcatgtatgtgaaggagtttctgatcagctctagccaggatggccaccagtggactctgttctttcagaatgggaaggtgaaggtgtttcagggcaatcaggactctttcacccctgtggtgaacagcctggacccccccctgctgaccagatacctgagaatccacccccagagctgggtgcaccagatcgccctgaggatggaggtgctgggctgtgaggctcaggatctgtactgagatatctctagagtcgacagtactggtgatcagcctcgactgtgccttctagttgccagccatctgttgtttgcccctcccccgtgccttccttgaccctggaaggtgccactcccactgtcctttcctaataaaatgaggaaattgcatcgcattgtctgagtaggtgtcattctattctggggggtggggtggggcaggacagcaagggggaggattgggaagacaatagcaggcatgctggggatgcggtgggctctatggaaccagctggggcccg

SEQ ID NO: 26 - DNA, 5934 bp, synthetic construct
  source 1..5934: mol_type = other DNA
ccccaactggggtaacctttgggctccccgggcgcgactagtgaattcgtcaatattggccattagccatattattcattggttatatagcataaatcaatattggctattggccattgcatacgttgtatctatatcataatatgtacatttatattggctcatgtccaatatgaccgccatgttggtgtggaaagtccccaggctccccagcaggcagaagtatgcaaagcatgcatctcaattagtcagcaaccaggcattgattattgactagttattaatagtaatcaattacggggtcattagttcatagcccatatatggagttccgcgttacataacttacggtaaatggcccgcctggctgaccgcccaacgacccccgcccattgacgtcaataatgacgtatgttcccatagtaacgccaatagggactttccattgacgtcaatgggtggagtatttacggtaaactgcccacttggcagtacatcaagtgtatcatatgccaagtccgccccctattgacgtcaatgacggtaaatggcccgcctggcattatgcccagtacatgaccttacgggactttcctacttggcagtacatctacgtattagtcatcgctattaccatggtgatgcggttttggcagtacaccaatgggcgtggatagcggtttgactcacggggatttccaagtctccaccccattgacgtcaatgggagtttgttttggcaccaaaatcaacgggactttccaaaatgtcgtaataaccccgccccgttgacgcaaatgggcggtaggcgtgtacggtgggaggtctatataagcagaggtcgtttagtgaaccgtcagatcactagtagctttattgcggtagtttatcacagttaaattgctaacgcagtcagtgctcgactgatcacaggtaagtatcaaggttacaagacaggtttaaggaggccaatagaaactgggcttgtcgagacagagaagattcttgcgtttctgataggcacctattggtcttactgacatccactttgcctttctctccacaggggtaccgaagccgctagcgctaccggtgccaccatgcagattgaactgagcacctgcttcttcctgtgtctgctgagattctgcttctctgccaccaggaggtactacctgggggctgtggagctgagctgggactacatgcagtctgacctgggggagctgcctgtggatgctaggttcccccctagagtgcccaagtccttccccttcaacacttctgtggtgtacaagaagaccctgtttgtggagttcactgaccacctgtttaacattgccaagcccaggcccccttggatgggcctgctggggcccaccatccaggctgaggtgtatgacactgtggtgatcaccctgaagaacatggccagccatcctgtgagcctgcatgctgtgggggtgagctactggaaggccagcgagggggctgagtatgatgaccagactagccagagggagaaggaggatgacaaggtgtttcctggaggcagccacacctatgtgtggcaggtgctgaaggagaatggccccatggcctctgaccccctgtgcctgacctacagctacctgagccatgtggatctggtgaaggacctgaactctggcctgattggggctctgctggtgtgtagagagggcagcctggctaaggagaagacccagaccctgcataagttcatcctgctgtttgctgtgtttgatgagggcaagagctggcactctgagaccaagaacagcctgatgcaggatagggatgctgcctctgccagggcttggcccaagatgcacactgtgaatggctatgtgaataggagcctgcctggcctgattggctgccacaggaagtctgtgtactggcatgtgattggaatgggcacaacccctgaggtccatagcatcttcctggagggccacactttcctggtgaggaaccacagacaggcctctctggagattagccccatcaccttcctgactgctcagactctgctgatggacctgggccagttcctgctgttttgccatattagctctcaccagcatgatggcatggaggcctatgtgaaggtggacagctgccctgaggagcctcagctgaggatgaagaacaatgaggaggctgaagactatgatgatgacctgactgattctgagatggatgtggtgaggtttgatgatgacaatagccccagcttcattcagatcagatctgtggccaaaaagcaccccaagacctgggtgcattacattgctgctgaagaggaggactgggactatgcccctctggtgctggcccctgatgataggagctataagagccagtacctgaacaatgggccccagaggattggcagaaagtacaagaaggtgaggttcatggcttacactgatgaaaccttcaaaaccagggaggccatccagcatgagtctggcatcctgggccctctgctgtatggagaggtgggagacaccctgctgatcatcttcaagaaccaggccagcaggccctacaacatctatcctcatggcatcactgatgtgagacctctgtacagcaggaggctgcctaagggggtgaaacacctgaaggactttcccatcctgcctggggagatcttcaagtataagtggactgtgactgtggaggatggccctaccaagtctgaccccaggtgtctgacaaggtattacagcagctttgtgaacatggagagggacctggcctctggcctgattggccctctgctgatctgctacaaggagtctgtggaccagaggggcaaccagatcatgtctgacaagaggaatgtgatcctgttctctgtgtttgatgagaataggagctggtatctgactgagaacatccagagattcctgcccaatcctgctggggtgcagctggaggaccctgagtttcaggccagcaatatcatgcacagcatcaatggctatgtgtttgacagcctgcagctgtctgtgtgcctgcatgaggtggcctactggtacatcctgagcattggagcccagactgattttctgtctgtgttcttttctggctataccttcaagcacaagatggtgtatgaggacaccctgaccctgttccccttctctggggagactgtgttcatgtctatggagaatcctgggctgtggattctgggctgccacaactctgatttcaggaacaggggcatgactgccctgctgaaggtgagcagctgtgacaagaacactggggactactatgaggatagctatgaggacatttctgcttatctgctgtctaagaataatgccattgagcccaggagcttcagccagaattctagacaccctagcaccagacagaaacagtttaatgccactaatgtgtctaacaacagcaacaccagcaatgacagcaatgtgtctaacaagacatctaacaacagcaacgccacaaacaagaccaacaacacaaatgatagcacaaaccggaccaaccagaccaataccagccagcagaacttcgtgacccagagaagtaagagagagatcaccaggactaccctgcagtctgatcaggaggagattgactatgatgacacaatctctgtggagatgaagaaggaggattttgacatctatgatgaggatgagaaccagagccccagatcttttcagaagaagaccagacactacttcattgctgctgtggagaggctgtgggactatggcatgagcagcagccctcatgtgctgaggaacagggcccagtctggctctgtgccccagttcaagaaggtggtgttccaggagtttactgatggcagcttcacccagcccctgtacagaggggagctgaatgagcacctgggcctgctgggcccttatatcagggctgaggtggaggataacattatggtgactttcaggaaccaggcctctaggccctacagcttctatagcagcctgatctcttatgaggaggatcagaggcagggggctgagcccagaaagaactttgtgaagcctaatgagactaagacctacttctggaaggtccagcaccacatggcccccaccaaggatgagtttgattgcaaggcctgggcctatttctctgatgtggacctggagaaggatgtccattctggcctgattggccctctgctggtgtgccacactaacactctgaatcctgcccatggcaggcaggtgactgtccaggagtttgccctgttcttcactatctttgatgagaccaagagctggtactttactgagaacatggagagaaactgcagggctccttgcaatatccagatggaggaccccaccttcaaggagaactacaggtttcatgccatcaatgggtacatcatggacaccctgcctggcctggtgatggctcaggaccagagaatcagatggtatctgctgagcatgggcagcaatgagaatatccacagcatccacttctctggacatgtgttcactgtgaggaagaaggaggagtacaagatggctctgtataatctgtaccctggagtgtttgaaactgtggagatgctgccttctaaggctggcatctggagggtggagtgcctgattggggagcacctgcatgctggcatgagcaccctgttcctggtgtacagcaacaagtgtcagacccccctgggcatggcctctggacacatcagggacttccagatcacagcctctggccagtatggccagtgggcccccaagctggccaggctgcattattctggcagcatcaatgcctggtctaccaaggagccctttagctggatcaaggtggacctgctggcccccatgattatccatggcatcaagacccagggggccaggcagaagttctctagcctgtacatcagccagttcatcatcatgtactctctggatggcaagaagtggcagacctacaggggcaacagcactggcacactgatggtgttctttggcaatgtggacagctctggcatcaagcacaacatcttcaatccccccattatcgctaggtatattaggctgcatcccacccactacagcatcagatctaccctgagaatggagctgatgggctgtgacctgaactcttgcagcatgcccctgggcatggagtctaaggccatctctgatgcccagattactgccagcagctacttcaccaatatgtttgccacctggagcccttctaaggccaggctgcatctgcaggggaggagcaatgcctggaggcctcaggtgaacaaccctaaggagtggctgcaggtggatttccagaagaccatgaaggtgactggagtgaccacccagggagtcaagagcctgctgaccagcatgtatgtgaaggagtttctgatcagctctagccaggatggccaccagtggactctgttctttcagaatgggaaggtgaaggtgtttcagggcaatcaggactctttcacccctgtggtgaacagcctggacccccccctgctgaccagatacctgagaatccacccccagagctgggtgcaccagatcgccctgaggatggaggtgctgggctgtgaggctcaggatctgtactgagatatctctagagtcgacagtactggtgatcagcctcgactgtgccttctagttgccagccatctgttgtttgcccctcccccgtgccttccttgaccctggaaggtgccactcccactgtcctttcctaataaaatgaggaaattgcatcgcattgtctgagtaggtgtcattctattctggggggtggggtggggcaggacagcaagggggaggattgggaagacaatagcaggcatgctggggatgcggtgggctctatggaaccagctggggcccg

SEQ ID NO: 27 - DNA, 5928 bp, synthetic construct
  source 1..5928: mol_type = other DNA
ccccaactggggtaacctttgggctccccgggcgcgactagtgaattcgtcaatattggccattagccatattattcattggttatatagcataaatcaatattggctattggccattgcatacgttgtatctatatcataatatgtacatttatattggctcatgtccaatatgaccgccatgttggtgtggaaagtccccaggctccccagcaggcagaagtatgcaaagcatgcatctcaattagtcagcaaccaggcattgattattgactagttattaatagtaatcaattacggggtcattagttcatagcccatatatggagttccgcgttacataacttacggtaaatggcccgcctggctgaccgcccaacgacccccgcccattgacgtcaataatgacgtatgttcccatagtaacgccaatagggactttccattgacgtcaatgggtggagtatttacggtaaactgcccacttggcagtacatcaagtgtatcatatgccaagtccgccccctattgacgtcaatgacggtaaatggcccgcctggcattatgcccagtacatgaccttacgggactttcctacttggcagtacatctacgtattagtcatcgctattaccatggtgatgcggttttggcagtacaccaatgggcgtggatagcggtttgactcacggggatttccaagtctccaccccattgacgtcaatgggagtttgttttggcaccaaaatcaacgggactttccaaaatgtcgtaataaccccgccccgttgacgcaaatgggcggtaggcgtgtacggtgggaggtctatataagcagaggtcgtttagtgaaccgtcagatcactagtagctttattgcggtagtttatcacagttaaattgctaacgcagtcagtgctcgactgatcacaggtaagtatcaaggttacaagacaggtttaaggaggccaatagaaactgggcttgtcgagacagagaagattcttgcgtttctgataggcacctattggtcttactgacatccactttgcctttctctccacaggggtaccgaagccgctagcgctaccggtgccaccatgcagattgaactgagcacctgcttcttcctgtgtctgctgagattctgcttctctgccaccaggaggtactacctgggggctgtggagctgagctgggactacatgcagtctgacctgggggagctgcctgtggatgctaggttcccccctagagtgcccaagtccttccccttcaacacttctgtggtgtacaagaagaccctgtttgtggagttcactgaccacctgtttaacattgccaagcccaggcccccttggatgggcctgctggggcccaccatccaggctgaggtgtatgacactgtggtggtgaccctgaagaacatggccagccatcctgtgagcctgcatgctgtgggggtgagctactggaagagcagcgagggggctgagtatgatgaccagactagccagagggagaaggaggatgacaaggtgtttcctggaaagagccacacctatgtgtggcaggtgctgaaggagaatggccccacagcctctgaccccccttgcctgacctacagctacctgagccatgtggatctggtgaaggacctgaactctggcctgattggggctctgctggtgtgtagagagggcagcctggctaaggagaagacccagaccctgcataagttcatcctgctgtttgctgtgtttgatgagggcaagagctggcactctgagaccaagaacagcctgatgcaggatagggatgctgcctctgccagggcttggcccaagatgcacactgtgaatggctatgtgaataggagcctgcctggcctgattggctgccacaggaagtctgtgtactggcatgtgattggaatgggcacaacccctgaggtccatagcatcttcctggagggccacactttcctggtgaggaaccacagacaggcctctctggagattagccccatcaccttcctgactgctcagactctgctgatggacctgggccagttcctgctgttttgccatattagctctcaccagcatgatggcatggaggcctatgtgaaggtggacagctgccctgaggagcctcagctgaggatgaagaacaatgaggaggctgaagactatgatgatgacctgactgattctgagatggatgtggtgaggtttgatgatgacaatagccccagcttcattcagatcagatctgtggccaaaaagcaccccaagacctgggtgcattacattgctgctgaagaggaggactgggactatgcccctctggtgctggcccctgatgataggagctataagagccagtacctgaacaatgggccccagaggattggcagaaagtacaagaaggtgaggttcatggcttacactgatgaaaccttcaaaaccagggaggccatccagcatgagtctggcatcctgggccctctgctgtatggagaggtgggagacaccctgctgatcatcttcaagaaccaggccagcaggccctacaacatctatcctcatggcatcactgatgtgagacctctgtacagcaggaggctgcctaagggggtgaaacacctgaaggactttcccatcctgcctggggagatcttcaagtataagtggactgtgactgtggaggatggccctaccaagtctgaccccaggtgtctgacaaggtattacagcagctttgtgaacatggagagggacctggcctctggcctgattggccctctgctgatctgctacaaggagtctgtggaccagaggggcaaccagatcatgtctgacaagaggaatgtgatcctgttctctgtgtttgatgagaataggagctggtatctgactgagaacatccagagattcctgcccaatcctgctggggtgcagctggaggaccctgagtttcaggccagcaatatcatgcacagcatcaatggctatgtgtttgacagcctgcagctgtctgtgtgcctgcatgaggtggcctactggtacatcctgagcattggagcccagactgattttctgtctgtgttcttttctggctataccttcaagcacaagatggtgtatgaggacaccctgaccctgttccccttctctggggagactgtgttcatgtctatggagaatcctgggctgtggattctgggctgccacaactctgatttcaggaacaggggcatgactgccctgctgaaggtgagcagctgtgacaagaacactggggactactatgaggatagctatgaggacatttctgcttatctgctgtctaagaataatgccattgagcccaggagcttcagccagaatagcagacaccctagcaccagacagaaacagtttaatgccactaatgtgagcaacaacagcaacaccagcaatgacagcaatgtgtctaacaagacatctaacaacagcaatgccacaaacaagaccaacaacacaaatgatagcacaaacaggaccaaccagaccaataccagcccccctgtgctgaagagacatcagagggagatcaccaggactaccctgcagtctgatcaggaggagattgactatgatgacacaatctctgtggagatgaagaaggaggattttgacatctatgatgaggatgagaaccagagccccagatcttttcagaagaagaccagacactacttcattgctgctgtggagaggctgtgggactatggcatgagcagcagccctcatgtgctgaggaacagggcccagtctggctctgtgccccagttcaagaaggtggtgttccaggagtttactgatggcagcttcacccagcccctgtacagaggggagctgaatgagcacctgggcctgctgggcccttatatcagggctgaggtggaggataacattatggtgactttcaggaaccaggcctctaggccctacagcttctatagcagcctgatctcttatgaggaggatcagaggcagggggctgagcccagaaagaactttgtgaagcctaatgagactaagacctacttctggaaggtccagcaccacatggcccccaccaaggatgagtttgattgcaaggcctgggcctatttctctgatgtggacctggagaaggatgtccattctggcctgattggccctctgctggtgtgccacactaacactctgaatcctgcccatggcaggcaggtgactgtccaggagtttgccctgttcttcactatctttgatgagaccaagagctggtactttactgagaacatggagagaaactgcagggctccttgcaatatccagatggaggaccccaccttcaaggagaactacaggtttcatgccatcaatgggtacatcatggacaccctgcctggcctggtgatggctcaggaccagagaatcagatggtatctgctgagcatgggcagcaatgagaatatccacagcatccacttctctggacatgtgttcactgtgaggaagaaggaggagtacaagatggctctgtataatctgtaccctggagtgtttgaaactgtggagatgctgccttctaaggctggcatctggagggtggagtgcctgattggggagcacctgcatgctggcatgagcaccctgttcctggtgtacagcaacaagtgtcagacccccctgggcatggcctctggacacatcagggacttccagatcacagcctctggccagtatggccagtgggcccccaagctggccaggctgcattattctggcagcatcaatgcctggtctaccaaggagccctttagctggatcaaggtggacctgctggcccccatgattatccatggcatcaagacccagggggccaggcagaagttctctagcctgtacatcagccagttcatcatcatgtactctctggatggcaagaagtggcagacctacaggggcaacagcactggcacactgatggtgttctttggcaatgtggacagctctggcatcaagcacaacatcttcaatccccccattatcgctaggtatattaggctgcatcccacccactacagcatcagatctaccctgagaatggagctgatgggctgtgacctgaactcttgcagcatgcccctgggcatggagtctaaggccatctctgatgcccagattactgccagcagctacttcaccaatatgtttgccacctggagcccttctaaggccaggctgcatctgcaggggaggagcaatgcctggaggcctcaggtgaacaaccctaaggagtggctgcaggtggatttccagaagaccatgaaggtgactggagtgaccacccagggagtcaagagcctgctgaccagcatgtatgtgaaggagtttctgatcagctctagccaggatggccaccagtggactctgttctttcagaatgggaaggtgaaggtgtttcagggcaatcaggactctttcacccctgtggtgaacagcctggacccccccctgctgaccagatacctgagaatccacccccagagctgggtgcaccagatcgccctgaggatggaggtgctgggctgtgaggctcaggatctgtactgagatatctctagagtcgacagtactggtgatcagcctcgactgtgccttctagttgccagccatctgttgtttgcccctcccccgtgccttccttgaccctggaaggtgccactcccactgtcctttcctaataaaatgaggaaattgcatcgcattgtctgagtaggtgtcattctattctggggggtggggtggggcaggacagcaagggggaggattgggaagacaatagcaggcatgctggggatgcggtgggctctatggaaccagctggggcccg

SEQ ID NO: 28 - DNA, 5934 bp, synthetic construct
  source 1..5934: mol_type = other DNA
ccccaactggggtaacctttgggctccccgggcgcgactagtgaattcgtcaatattggccattagccatattattcattggttatatagcataaatcaatattggctattggccattgcatacgttgtatctatatcataatatgtacatttatattggctcatgtccaatatgaccgccatgttggtgtggaaagtccccaggctccccagcaggcagaagtatgcaaagcatgcatctcaattagtcagcaaccaggcattgattattgactagttattaatagtaatcaattacggggtcattagttcatagcccatatatggagttccgcgttacataacttacggtaaatggcccgcctggctgaccgcccaacgacccccgcccattgacgtcaataatgacgtatgttcccatagtaacgccaatagggactttccattgacgtcaatgggtggagtatttacggtaaactgcccacttggcagtacatcaagtgtatcatatgccaagtccgccccctattgacgtcaatgacggtaaatggcccgcctggcattatgcccagtacatgaccttacgggactttcctacttggcagtacatctacgtattagtcatcgctattaccatggtgatgcggttttggcagtacaccaatgggcgtggatagcggtttgactcacggggatttccaagtctccaccccattgacgtcaatgggagtttgttttggcaccaaaatcaacgggactttccaaaatgtcgtaataaccccgccccgttgacgcaaatgggcggtaggcgtgtacggtgggaggtctatataagcagaggtcgtttagtgaaccgtcagatcactagtagctttattgcggtagtttatcacagttaaattgctaacgcagtcagtgctcgactgatcacaggtaagtatcaaggttacaagacaggtttaaggaggccaatagaaactgggcttgtcgagacagagaagattcttgcgtttctgataggcacctattggtcttactgacatccactttgcctttctctccacaggggtaccgaagccgctagcgctaccggtgccaccatgcagattgaactgagcacctgcttcttcctgtgtctgctgagattctgcttctctgccaccaggaggtactacctgggggctgtggagctgagctgggactacatgcagtctgacctgggggagctgcctgtggatgctaggttcccccctagagtgcccaagtccttccccttcaacacttctgtggtgtacaagaagaccctgtttgtggagttcactgaccacctgtttaacattgccaagcccaggcccccttggatgggcctgctggggcccaccatccaggctgaggtgtatgacactgtggtggtgaccctgaagaacatggccagccatcctgtgagcctgcatgctgtgggggtgagctactggaagagcagcgagggggctgagtatgatgaccagactagccagagggagaaggaggatgacaaggtgtttcctggaaagagccacacctatgtgtggcaggtgctgaaggagaatggccccacagcctctgaccccccttgcctgacctacagctacctgagccatgtggatctggtgaaggacctgaactctggcctgattggggctctgctggtgtgtagagagggcagcctggctaaggagaagacccagaccctgcataagttcatcctgctgtttgctgtgtttgatgagggcaagagctggcactctgagaccaagaacagcctgatgcaggatagggatgctgcctctgccagggcttggcccaagatgcacactgtgaatggctatgtgaataggagcctgcctggcctgattggctgccacaggaagtctgtgtactggcatgtgattggaatgggcacaacccctgaggtccatagcatcttcctggagggccacactttcctggtgaggaaccacagacaggcctctctggagattagccccatcaccttcctgactgctcagactctgctgatggacctgggccagttcctgctgttttgccatattagctctcaccagcatgatggcatggaggcctatgtgaaggtggacagctgccctgaggagcctcagctgaggatgaagaacaatgaggaggctgaagactatgatgatgacctgactgattctgagatggatgtggtgaggtttgatgatgacaatagccccagcttcattcagatcagatctgtggccaaaaagcaccccaagacctgggtgcattacattgctgctgaagaggaggactgggactatgcccctctggtgctggcccctgatgataggagctataagagccagtacctgaacaatgggccccagaggattggcagaaagtacaagaaggtgaggttcatggcttacactgatgaaaccttcaaaaccagggaggccatccagcatgagtctggcatcctgggccctctgctgtatggagaggtgggagacaccctgctgatcatcttcaagaaccaggccagcaggccctacaacatctatcctcatggcatcactgatgtgagacctctgtacagcaggaggctgcctaagggggtgaaacacctgaaggactttcccatcctgcctggggagatcttcaagtataagtggactgtgactgtggaggatggccctaccaagtctgaccccaggtgtctgacaaggtattacagcagctttgtgaacatggagagggacctggcctctggcctgattggccctctgctgatctgctacaaggagtctgtggaccagaggggcaaccagatcatgtctgacaagaggaatgtgatcctgttctctgtgtttgatgagaataggagctggtatctgactgagaacatccagagattcctgcccaatcctgctggggtgcagctggaggaccctgagtttcaggccagcaatatcatgcacagcatcaatggctatgtgtttgacagcctgcagctgtctgtgtgcctgcatgaggtggcctactggtacatcctgagcattggagcccagactgattttctgtctgtgttcttttctggctataccttcaagcacaagatggtgtatgaggacaccctgaccctgttccccttctctggggagactgtgttcatgtctatggagaatcctgggctgtggattctgggctgccacaactctgatttcaggaacaggggcatgactgccctgctgaaggtgagcagctgtgacaagaacactggggactactatgaggatagctatgaggacatttctgcttatctgctgtctaagaataatgccattgagcccaggagcttcagccagaattctagacaccctagcaccagacagaaacagtttaatgccactaatgtgtctaacaacagcaacaccagcaatgacagcaatgtgtctaacaagacatctaacaacagcaacgccacaaacaagaccaacaacacaaatgatagcacaaaccggaccaaccagaccaataccagccagcagaacttcgtgacccagagaagtaagagagagatcaccaggactaccctgcagtctgatcaggaggagattgactatgatgacacaatctctgtggagatgaagaaggaggattttgacatctatgatgaggatgagaaccagagccccagatcttttcagaagaagaccagacactacttcattgctgctgtggagaggctgtgggactatggcatgagcagcagccctcatgtgctgaggaacagggcccagtctggctctgtgccccagttcaagaaggtggtgttccaggagtttactgatggcagcttcacccagcccctgtacagaggggagctgaatgagcacctgggcctgctgggcccttatatcagggctgaggtggaggataacattatggtgactttcaggaaccaggcctctaggccctacagcttctatagcagcctgatctcttatgaggaggatcagaggcagggggctgagcccagaaagaactttgtgaagcctaatgagactaagacctacttctggaaggtccagcaccacatggcccccaccaaggatgagtttgattgcaaggcctgggcctatttctctgatgtggacctggagaaggatgtccattctggcctgattggccctctgctggtgtgccacactaacactctgaatcctgcccatggcaggcaggtgactgtccaggagtttgccctgttcttcactatctttgatgagaccaagagctggtactttactgagaacatggagagaaactgcagggctccttgcaatatccagatggaggaccccaccttcaaggagaactacaggtttcatgccatcaatgggtacatcatggacaccctgcctggcctggtgatggctcaggaccagagaatcagatggtatctgctgagcatgggcagcaatgagaatatccacagcatccacttctctggacatgtgttcactgtgaggaagaaggaggagtacaagatggctctgtataatctgtaccctggagtgtttgaaactgtggagatgctgccttctaaggctggcatctggagggtggagtgcctgattggggagcacctgcatgctggcatgagcaccctgttcctggtgtacagcaacaagtgtcagacccccctgggcatggcctctggacacatcagggacttccagatcacagcctctggccagtatggccagtgggcccccaagctggccaggctgcattattctggcagcatcaatgcctggtctaccaaggagccctttagctggatcaaggtggacctgctggcccccatgattatccatggcatcaagacccagggggccaggcagaagttctctagcctgtacatcagccagttcatcatcatgtactctctggatggcaagaagtggcagacctacaggggcaacagcactggcacactgatggtgttctttggcaatgtggacagctctggcatcaagcacaacatcttcaatccccccattatcgctaggtatattaggctgcatcccacccactacagcatcagatctaccctgagaatggagctgatgggctgtgacctgaactcttgcagcatgcccctgggcatggagtctaaggccatctctgatgcccagattactgccagcagctacttcaccaatatgtttgccacctggagcccttctaaggccaggctgcatctgcaggggaggagcaatgcctggaggcctcaggtgaacaaccctaaggagtggctgcaggtggatttccagaagaccatgaaggtgactggagtgaccacccagggagtcaagagcctgctgaccagcatgtatgtgaaggagtttctgatcagctctagccaggatggccaccagtggactctgttctttcagaatgggaaggtgaaggtgtttcagggcaatcaggactctttcacccctgtggtgaacagcctggacccccccctgctgaccagatacctgagaatccacccccagagctgggtgcaccagatcgccctgaggatggaggtgctgggctgtgaggctcaggatctgtactgagatatctctagagtcgacagtactggtgatcagcctcgactgtgccttctagttgccagccatctgttgtttgcccctcccccgtgccttccttgaccctggaaggtgccactcccactgtcctttcctaataaaatgaggaaattgcatcgcattgtctgagtaggtgtcattctattctggggggtggggtggggcaggacagcaagggggaggattgggaagacaatagcaggcatgctggggatgcggtgggctctatggaaccagctggggcccg

SEQ ID NO: 29 - DNA, 204 bp, synthetic construct
  source 1..204: mol_type = other DNA
gtgatgcggttttggcagtacaccaatgggcgtggatagcggtttgactcacggggatttccaagtctccaccccattgacgtcaatgggagtttgttttggcaccaaaatcaacgggactttccaaaatgtcgtaataaccccgccccgttgacgcaaatgggcggtaggcgtgtacggtgggaggtctatataagcagaggt

SEQ ID NO: 30 - DNA, 380 bp, synthetic construct
  source 1..380: mol_type = other DNA
ggcattgattattgactagttattaatagtaatcaattacggggtcattagttcatagcccatatatggagttccgcgttacataacttacggtaaatggcccgcctggctgaccgcccaacgacccccgcccattgacgtcaataatgacgtatgttcccatagtaacgccaatagggactttccattgacgtcaatgggtggagtatttacggtaaactgcccacttggcagtacatcaagtgtatcatatgccaagtccgccccctattgacgtcaatgacggtaaatggcccgcctggcattatgcccagtacatgaccttacgggactttcctacttggcagtacatctacgtattagtcatcgctattaccatg

SEQ ID NO: 31 - DNA, 88 bp, synthetic construct
  source 1..88: mol_type = other DNA
ggtaccgaagccgctagcgctaccggtcaagcttggatccgctagctccggagagctcagatctgatatctctagagtcgacagtact

SEQ ID NO: 32 - DNA, 225 bp, synthetic construct
  source 1..225: mol_type = other DNA
ctgtgccttctagttgccagccatctgttgtttgcccctcccccgtgccttccttgaccctggaaggtgccactcccactgtcctttcctaataaaatgaggaaattgcatcgcattgtctgagtaggtgtcattctattctggggggtggggtggggcaggacagcaagggggaggattgggaagacaatagcaggcatgctggggatgcggtgggctctatgg

SEQ ID NO: 33 - DNA, 57 bp, synthetic construct
  source 1..57: mol_type = other DNA
atgcagattgaactgagcacctgcttcttcctgtgtctgctgagattctgcttctct

SEQ ID NO: 34 - DNA, 57 bp, synthetic construct
  source 1..57: mol_type = other DNA
atgcaaatagagctctccacctgcttctttctgtgccttttgcgattctgctttagt

SEQ ID NO: 35 - DNA, 4317 bp, synthetic construct
  source 1..4317: mol_type = other DNA
gccaccagaagatactacctgggtgcagtggaactgtcatgggactatatgcaaagtgatctcggtgagctgcctgtggacgcaagatttcctcctagagtgccaaaatcttttccattcaacacctcagtcgtgtacaaaaagactctgtttgtagaattcacggatcaccttttcaacatcgctaagccaaggccaccctggatgggtctgctaggtcctaccatccaggctgaggtttatgatacagtggtcattacacttaagaacatggcttcccatcctgtcagtcttcatgctgttggtgtatcctactggaaagcttctgagggagctgaatatgatgatcagaccagtcaaagggagaaagaagatgataaagtcttccctggtggaagccatacatatgtctggcaggtcctgaaagagaatggtccaatggcctctgacccactgtgccttacctactcatatctttctcatgtggacctggtaaaagacttgaattcaggcctcattggagccctactagtatgtagagaagggagtctggccaaggaaaagacacagaccttgcacaaatttatactactttttgctgtatttgatgaagggaaaagttggcactcagaaacaaagaactccttgatgcaggatagggatgctgcatctgctcgggcctggcctaaaatgcacacagtcaatggttatgtaaacaggtctctgccaggtctgattggatgccacaggaaatcagtctattggcatgtgattggaatgggcaccactcctgaagtgcactcaatattcctcgaaggtcacacatttcttgtgaggaaccatcgccaggcgtccttggaaatctcgccaataactttccttactgctcaaacactcttgatggaccttggacagtttctactgttttgtcatatctcttcccaccaacatgatggcatggaagcttatgtcaaagtagacagctgtccagaggaaccccaactacgaatgaaaaataatgaagaagcggaagactatgatgatgatcttactgattctgaaatggatgtggtcaggtttgatgatgacaactctccttcctttatccaaattcgctcagttgccaagaagcatcctaaaacttgggtacattacattgctgctgaagaggaggactgggactatgctcccttagtcctcgcccccgatgacagaagttataaaagtcaatatttgaacaatggccctcagcggattggtaggaagtacaaaaaagtccgatttatggcatacacagatgaaacctttaagactcgtgaagctattcagcatgaatcaggaatcttgggacctttactttatggggaagttggagacacactgttgattatatttaagaatcaagcaagcagaccatataacatctaccctcacggaatcactgatgtccgtcctttgtattcaaggagattaccaaaaggtgtaaaacatttgaaggattttccaattctgccaggagaaatattcaaatataaatggacagtgactgtagaagatgggccaactaaatcagatcctcggtgcctgacccgctattactctagtttcgttaatatggagagagatctagcttcaggactcattggccctctcctcatctgctacaaagaatctgtagatcaaagaggaaaccagataatgtcagacaagaggaatgtcatcctgttttctgtatttgatgagaaccgaagctggtacctcacagagaatatacaacgctttctccccaatccagctggagtgcagcttgaggatccagagttccaagcctccaacatcatgcacagcatcaatggctatgtttttgatagtttgcagttgtcagtttgtttgcatgaggtggcatactggtacattctaagcattggagcacagactgacttcctttctgtcttcttctctggatataccttcaaacacaaaatggtctatgaagacacactcaccctattcccattctcaggagaaactgtcttcatgtcgatggaaaacccaggtctatggattctggggtgccacaactcagactttcggaacagaggcatgaccgccttactgaaggtttctagttgtgacaagaacactggtgattattacgaggacagttatgaagatatttcagcatacttgctgagtaaaaacaatgccattgaaccaagaagcttctctcaaaacccaccagtcttgaaacgccatcaacgggaaataactcgtactactcttcagtcagatcaagaggaaattgactatgatgataccatatcagttgaaatgaagaaggaagattttgacatttatgatgaggatgaaaatcagagcccccgcagctttcaaaagaaaacacgacactattttattgctgcagtggagaggctctgggattatgggatgagtagctccccacatgttctaagaaacagggctcagagtggcagtgtccctcagttcaagaaagttgttttccaggaatttactgatggctcctttactcagcccttataccgtggagaactaaatgaacatttgggactcctggggccatatataagagcagaagttgaagataatatcatggtaactttcagaaatcaggcctctcgtccctattccttctattctagccttatttcttatgaggaagatcagaggcaaggagcagaacctagaaaaaactttgtcaagcctaatgaaaccaaaacttacttttggaaagtgcaacatcatatggcacccactaaagatgagtttgactgcaaagcctgggcttatttctctgatgttgacctggaaaaagatgtgcactcaggcctgattggaccccttctggtctgccacactaacacactgaaccctgctcatgggagacaagtgacagtacaggaatttgctctgtttttcaccatctttgatgagaccaaaagctggtacttcactgaaaatatggaaagaaactgcagggctccctgcaatatccagatggaagatcccacttttaaagagaattatcgcttccatgcaatcaatggctacataatggatacactacctggcttagtaatggctcaggatcaaaggattcgatggtatctgctcagcatgggcagcaatgaaaacatccattctattcatttcagtggacatgtgttcactgtacgaaaaaaagaggagtataaaatggcactgtacaatctctatccaggtgtttttgagacagtggaaatgttaccatccaaagctggaatttggcgggtggaatgccttattggcgagcatctacatgctgggatgagcacactttttctggtgtacagcaataagtgtcagactcccctgggaatggcttctggacacattagagattttcagattacagcttcaggacaatatggacagtgggccccaaagctggccagacttcattattccggatcaatcaatgcctggagcaccaaggagcccttttcttggatcaaggtggatctgttggcaccaatgattattcacggcatcaagacccagggtgcccgtcagaagttctccagcctctacatctctcagtttatcatcatgtatagtcttgatgggaagaagtggcagacttatcgaggaaattccactggaaccttaatggtcttctttggcaatgtggattcatctgggataaaacacaatatttttaaccctccaattattgctcgatacatccgtttgcacccaactcattatagcattcgcagcactcttcgcatggagttgatgggctgtgatttaaatagttgcagcatgccattgggaatggagagtaaagcaatatcagatgcacagattactgcttcatcctactttaccaatatgtttgccacctggtctccttcaaaagctcgacttcacctccaagggaggagtaatgcctggagacctcaggtgaataatccaaaagagtggctgcaagtggacttccagaagacaatgaaagtcacaggagtaactactcagggagtaaaatctctgcttaccagcatgtatgtgaaggagttcctcatctccagcagtcaagatggccatcagtggactctcttttttcagaatggcaaagtaaaggtttttcagggaaatcaagactccttcacacctgtggtgaactctctagacccaccgttactgactcgctaccttcgaattcacccccagagttgggtgcaccagattgccctgaggatggaggttctgggctgcgaggcacaggacctctactga

SEQ ID NO: 36 - DNA, 4368 bp, synthetic construct
  source 1..4368: mol_type = other DNA
gccaccagaagatactacctgggtgcagtggaactgtcatgggactatatgcaaagtgatctcggtgagctgcctgtggacgcaagatttcctcctagagtgccaaaatcttttccattcaacacctcagtcgtgtacaaaaagactctgtttgtagaattcacggatcaccttttcaacatcgctaagccaaggccaccctggatgggtctgctaggtcctaccatccaggctgaggtttatgatacagtggtcattacacttaagaacatggcttcccatcctgtcagtcttcatgctgttggtgtatcctactggaaagcttctgagggagctgaatatgatgatcagaccagtcaaagggagaaagaagatgataaagtcttccctggtggaagccatacatatgtctggcaggtcctgaaagagaatggtccaatggcctctgacccactgtgccttacctactcatatctttctcatgtggacctggtaaaagacttgaattcaggcctcattggagccctactagtatgtagagaagggagtctggccaaggaaaagacacagaccttgcacaaatttatactactttttgctgtatttgatgaagggaaaagttggcactcagaaacaaagaactccttgatgcaggatagggatgctgcatctgctcgggcctggcctaaaatgcacacagtcaatggttatgtaaacaggtctctgccaggtctgattggatgccacaggaaatcagtctattggcatgtgattggaatgggcaccactcctgaagtgcactcaatattcctcgaaggtcacacatttcttgtgaggaaccatcgccaggcgtccttggaaatctcgccaataactttccttactgctcaaacactcttgatggaccttggacagtttctactgttttgtcatatctcttcccaccaacatgatggcatggaagcttatgtcaaagtagacagctgtccagaggaaccccaactacgaatgaaaaataatgaagaagcggaagactatgatgatgatcttactgattctgaaatggatgtggtcaggtttgatgatgacaactctccttcctttatccaaattcgctcagttgccaagaagcatcctaaaacttgggtacattacattgctgctgaagaggaggactgggactatgctcccttagtcctcgcccccgatgacagaagttataaaagtcaatatttgaacaatggccctcagcggattggtaggaagtacaaaaaagtccgatttatggcatacacagatgaaacctttaagactcgtgaagctattcagcatgaatcaggaatcttgggacctttactttatggggaagttggagacacactgttgattatatttaagaatcaagcaagcagaccatataacatctaccctcacggaatcactgatgtccgtcctttgtattcaaggagattaccaaaaggtgtaaaacatttgaaggattttccaattctgccaggagaaatattcaaatataaatggacagtgactgtagaagatgggccaactaaatcagatcctcggtgcctgacccgctattactctagtttcgttaatatggagagagatctagcttcaggactcattggccctctcctcatctgctacaaagaatctgtagatcaaagaggaaaccagataatgtcagacaagaggaatgtcatcctgttttctgtatttgatgagaaccgaagctggtacctcacagagaatatacaacgctttctccccaatccagctggagtgcagcttgaggatccagagttccaagcctccaacatcatgcacagcatcaatggctatgtttttgatagtttgcagttgtcagtttgtttgcatgaggtggcatactggtacattctaagcattggagcacagactgacttcctttctgtcttcttctctggatataccttcaaacacaaaatggtctatgaagacacactcaccctattcccattctcaggagaaactgtcttcatgtcgatggaaaacccaggtctatggattctggggtgccacaactcagactttcggaacagaggcatgaccgccttactgaaggtttctagttgtgacaagaacactggtgattattacgaggacagttatgaagatatttcagcatacttgctgagtaaaaacaatgccattgaaccaagaagcttcagccagaatgccactaatgtgtctaacaacagcaacaccagcaatgacagcaatgtgtctccccctgtgctgaagagacatcagagggaaataactcgtactactcttcagtcagatcaagaggaaattgactatgatgataccatatcagttgaaatgaagaaggaagattttgacatttatgatgaggatgaaaatcagagcccccgcagctttcaaaagaaaacacgacactattttattgctgcagtggagaggctctgggattatgggatgagtagctccccacatgttctaagaaacagggctcagagtggcagtgtccctcagttcaagaaagttgttttccaggaatttactgatggctcctttactcagcccttataccgtggagaactaaatgaacatttgggactcctggggccatatataagagcagaagttgaagataatatcatggtaactttcagaaatcaggcctctcgtccctattccttctattctagccttatttcttatgaggaagatcagaggcaaggagcagaacctagaaaaaactttgtcaagcctaatgaaaccaaaacttacttttggaaagtgcaacatcatatggcacccactaaagatgagtttgactgcaaagcctgggcttatttctctgatgttgacctggaaaaagatgtgcactcaggcctgattggaccccttctggtctgccacactaacacactgaaccctgctcatgggagacaagtgacagtacaggaatttgctctgtttttcaccatctttgatgagaccaaaagctggtacttcactgaaaatatggaaagaaactgcagggctccctgcaatatccagatggaagatcccacttttaaagagaattatcgcttccatgcaatcaatggctacataatggatacactacctggcttagtaatggctcaggatcaaaggattcgatggtatctgctcagcatgggcagcaatgaaaacatccattctattcatttcagtggacatgtgttcactgtacgaaaaaaagaggagtataaaatggcactgtacaatctctatccaggtgtttttgagacagtggaaatgttaccatccaaagctggaatttggcgggtggaatgccttattggcgagcatctacatgctgggatgagcacactttttctggtgtacagcaataagtgtcagactcccctgggaatggcttctggacacattagagattttcagattacagcttcaggacaatatggacagtgggccccaaagctggccagacttcattattccggatcaatcaatgcctggagcaccaaggagcccttttcttggatcaaggtggatctgttggcaccaatgattattcacggcatcaagacccagggtgcccgtcagaagttctccagcctctacatctctcagtttatcatcatgtatagtcttgatgggaagaagtggcagacttatcgaggaaattccactggaaccttaatggtcttctttggcaatgtggattcatctgggataaaacacaatatttttaaccctccaattattgctcgatacatccgtttgcacccaactcattatagcattcgcagcactcttcgcatggagttgatgggctgtgatttaaatagttgcagcatgccattgggaatggagagtaaagcaatatcagatgcacagattactgcttcatcctactttaccaatatgtttgccacctggtctccttcaaaagctcgacttcacctccaagggaggagtaatgcctggagacctcaggtgaataatccaaaagagtggctgcaagtggacttccagaagacaatgaaagtcacaggagtaactactcagggagtaaaatctctgcttaccagcatgtatgtgaaggagttcctcatctccagcagtcaagatggccatcagtggactctcttttttcagaatggcaaagtaaaggtttttcagggaaatcaagactccttcacacctgtggtgaactctctagacccaccgttactgactcgctaccttcgaattcacccccagagttgggtgcaccagattgccctgaggatggaggttctgggctgcgaggcacaggacctctactga

SEQ ID NO: 37 - DNA, 4338 bp, synthetic construct
  source 1..4338: mol_type = other DNA
gccaccagaagatactacctgggtgcagtggaactgtcatgggactatatgcaaagtgatctcggtgagctgcctgtggacgcaagatttcctcctagagtgccaaaatcttttccattcaacacctcagtcgtgtacaaaaagactctgtttgtagaattcacggatcaccttttcaacatcgctaagccaaggccaccctggatgggtctgctaggtcctaccatccaggctgaggtttatgatacagtggtcattacacttaagaacatggcttcccatcctgtcagtcttcatgctgttggtgtatcctactggaaagcttctgagggagctgaatatgatgatcagaccagtcaaagggagaaagaagatgataaagtcttccctggtggaagccatacatatgtctggcaggtcctgaaagagaatggtccaatggcctctgacccactgtgccttacctactcatatctttctcatgtggacctggtaaaagacttgaattcaggcctcattggagccctactagtatgtagagaagggagtctggccaaggaaaagacacagaccttgcacaaatttatactactttttgctgtatttgatgaagggaaaagttggcactcagaaacaaagaactccttgatgcaggatagggatgctgcatctgctcgggcctggcctaaaatgcacacagtcaatggttatgtaaacaggtctctgccaggtctgattggatgccacaggaaatcagtctattggcatgtgattggaatgggcaccactcctgaagtgcactcaatattcctcgaaggtcacacatttcttgtgaggaaccatcgccaggcgtccttggaaatctcgccaataactttccttactgctcaaacactcttgatggaccttggacagtttctactgttttgtcatatctcttcccaccaacatgatggcatggaagcttatgtcaaagtagacagctgtccagaggaaccccaactacgaatgaaaaataatgaagaagcggaagactatgatgatgatcttactgattctgaaatggatgtggtcaggtttgatgatgacaactctccttcctttatccaaattcgctcagttgccaagaagcatcctaaaacttgggtacattacattgctgctgaagaggaggactgggactatgctcccttagtcctcgcccccgatgacagaagttataaaagtcaatatttgaacaatggccctcagcggattggtaggaagtacaaaaaagtccgatttatggcatacacagatgaaacctttaagactcgtgaagctattcagcatgaatcaggaatcttgggacctttactttatggggaagttggagacacactgttgattatatttaagaatcaagcaagcagaccatataacatctaccctcacggaatcactgatgtccgtcctttgtattcaaggagattaccaaaaggtgtaaaacatttgaaggattttccaattctgccaggagaaatattcaaatataaatggacagtgactgtagaagatgggccaactaaatcagatcctcggtgcctgacccgctattactctagtttcgttaatatggagagagatctagcttcaggactcattggccctctcctcatctgctacaaagaatctgtagatcaaagaggaaaccagataatgtcagacaagaggaatgtcatcctgttttctgtatttgatgagaaccgaagctggtacctcacagagaatatacaacgctttctccccaatccagctggagtgcagcttgaggatccagagttccaagcctccaacatcatgcacagcatcaatggctatgtttttgatagtttgcagttgtcagtttgtttgcatgaggtggcatactggtacattctaagcattggagcacagactgacttcctttctgtcttcttctctggatataccttcaaacacaaaatggtctatgaagacacactcaccctattcccattctcaggagaaactgtcttcatgtcgatggaaaacccaggtctatggattctggggtgccacaactcagactttcggaacagaggcatgaccgccttactgaaggtttctagttgtgacaagaacactggtgattattacgaggacagttatgaagatatttcagcatacttgctgagtaaaaacaatgccattgaaccaagaagcttcagccagaattctagacaccctagccaaaacccccctgtgctgaagagacatcagagggaaataactcgtactactcttcagtcagatcaagaggaaattgactatgatgataccatatcagttgaaatgaagaaggaagattttgacatttatgatgaggatgaaaatcagagcccccgcagctttcaaaagaaaacacgacactattttattgctgcagtggagaggctctgggattatgggatgagtagctccccacatgttctaagaaacagggctcagagtggcagtgtccctcagttcaagaaagttgttttccaggaatttactgatggctcctttactcagcccttataccgtggagaactaaatgaacatttgggactcctggggccatatataagagcagaagttgaagataatatcatggtaactttcagaaatcaggcctctcgtccctattccttctattctagccttatttcttatgaggaagatcagaggcaaggagcagaacctagaaaaaactttgtcaagcctaatgaaaccaaaacttacttttggaaagtgcaacatcatatggcacccactaaagatgagtttgactgcaaagcctgggcttatttctctgatgttgacctggaaaaagatgtgcactcaggcctgattggaccccttctggtctgccacactaacacactgaaccctgctcatgggagacaagtgacagtacaggaatttgctctgtttttcaccatctttgatgagaccaaaagctggtacttcactgaaaatatggaaagaaactgcagggctccctgcaatatccagatggaagatcccacttttaaagagaattatcgcttccatgcaatcaatggctacataatggatacactacctggcttagtaatggctcaggatcaaaggattcgatggtatctgctcagcatgggcagcaatgaaaacatccattctattcatttcagtggacatgtgttcactgtacgaaaaaaagaggagtataaaatggcactgtacaatctctatccaggtgtttttgagacagtggaaatgttaccatccaaagctggaatttggcgggtggaatgccttattggcgagcatctacatgctgggatgagcacactttttctggtgtacagcaataagtgtcagactcccctgggaatggcttctggacacattagagattttcagattacagcttcaggacaatatggacagtgggccccaaagctggccagacttcattattccggatcaatcaatgcctggagcaccaaggagcccttttcttggatcaaggtggatctgttggcaccaatgattattcacggcatcaagacccagggtgcccgtcagaagttctccagcctctacatctctcagtttatcatcatgtatagtcttgatgggaagaagtggcagacttatcgaggaaattccactggaaccttaatggtcttctttggcaatgtggattcatctgggataaaacacaatatttttaaccctccaattattgctcgatacatccgtttgcacccaactcattatagcattcgcagcactcttcgcatggagttgatgggctgtgatttaaatagttgcagcatgccattgggaatggagagtaaagcaatatcagatgcacagattactgcttcatcctactttaccaatatgtttgccacctggtctccttcaaaagctcgacttcacctccaagggaggagtaatgcctggagacctcaggtgaataatccaaaagagtggctgcaagtggacttccagaagacaatgaaagtcacaggagtaactactcagggagtaaaatctctgcttaccagcatgtatgtgaaggagttcctcatctccagcagtcaagatggccatcagtggactctcttttttcagaatggcaaagtaaaggtttttcagggaaatcaagactccttcacacctgtggtgaactctctagacccaccgttactgactcgctaccttcgaattcacccccagagttgggtgcaccagattgccctgaggatggaggttctgggctgcgaggcacaggacctctactga

SEQ ID NO: 38 - DNA, 4491 bp, synthetic construct
  source 1..4491: mol_type = other DNA
gccaccagaagatactacctgggtgcagtggaactgtcatgggactatatgcaaagtgatctcggtgagctgcctgtggacgcaagatttcctcctagagtgccaaaatcttttccattcaacacctcagtcgtgtacaaaaagactctgtttgtagaattcacggatcaccttttcaacatcgctaagccaaggccaccctggatgggtctgctaggtcctaccatccaggctgaggtttatgatacagtggtcattacacttaagaacatggcttcccatcctgtcagtcttcatgctgttggtgtatcctactggaaagcttctgagggagctgaatatgatgatcagaccagtcaaagggagaaagaagatgataaagtcttccctggtggaagccatacatatgtctggcaggtcctgaaagagaatggtccaatggcctctgacccactgtgccttacctactcatatctttctcatgtggacctggtaaaagacttgaattcaggcctcattggagccctactagtatgtagagaagggagtctggccaaggaaaagacacagaccttgcacaaatttatactactttttgctgtatttgatgaagggaaaagttggcactcagaaacaaagaactccttgatgcaggatagggatgctgcatctgctcgggcctggcctaaaatgcacacagtcaatggttatgtaaacaggtctctgccaggtctgattggatgccacaggaaatcagtctattggcatgtgattggaatgggcaccactcctgaagtgcactcaatattcctcgaaggtcacacatttcttgtgaggaaccatcgccaggcgtccttggaaatctcgccaataactttccttactgctcaaacactcttgatggaccttggacagtttctactgttttgtcatatctcttcccaccaacatgatggcatggaagcttatgtcaaagtagacagctgtccagaggaaccccaactacgaatgaaaaataatgaagaagcggaagactatgatgatgatcttactgattctgaaatggatgtggtcaggtttgatgatgacaactctccttcctttatccaaattcgctcagttgccaagaagcatcctaaaacttgggtacattacattgctgctgaagaggaggactgggactatgctcccttagtcctcgcccccgatgacagaagttataaaagtcaatatttgaacaatggccctcagcggattggtaggaagtacaaaaaagtccgatttatggcatacacagatgaaacctttaagactcgtgaagctattcagcatgaatcaggaatcttgggacctttactttatggggaagttggagacacactgttgattatatttaagaatcaagcaagcagaccatataacatctaccctcacggaatcactgatgtccgtcctttgtattcaaggagattaccaaaaggtgtaaaacatttgaaggattttccaattctgccaggagaaatattcaaatataaatggacagtgactgtagaagatgggccaactaaatcagatcctcggtgcctgacccgctattactctagtttcgttaatatggagagagatctagcttcaggactcattggccctctcctcatctgctacaaagaatctgtagatcaaagaggaaaccagataatgtcagacaagaggaatgtcatcctgttttctgtatttgatgagaaccgaagctggtacctcacagagaatatacaacgctttctccccaatccagctggagtgcagcttgaggatccagagttccaagcctccaacatcatgcacagcatcaatggctatgtttttgatagtttgcagttgtcagtttgtttgcatgaggtggcatactggtacattctaagcattggagcacagactgacttcctttctgtcttcttctctggatataccttcaaacacaaaatggtctatgaagacacactcaccctattcccattctcaggagaaactgtcttcatgtcgatggaaaacccaggtctatggattctggggtgccacaactcagactttcggaacagaggcatgaccgccttactgaaggtttctagttgtgacaagaacactggtgattattacgaggacagttatgaagatatttcagcatacttgctgagtaaaaacaatgccattgaaccaagaagcttcagccagaatagcagacaccctagcaccagacagaaacagtttaatgccactaatgtgagcaacaacagcaacaccagcaatgacagcaatgtgtctaacaagacatctaacaacagcaatgccacaaacaagaccaacaacacaaatgatagcacaaacaggaccaaccagaccaataccagcccccctgtgctgaagagacatcagagggaaataactcgtactactcttcagtcagatcaagaggaaattgactatgatgataccatatcagttgaaatgaagaaggaagattttgacatttatgatgaggatgaaaatcagagcccccgcagctttcaaaagaaaacacgacactattttattgctgcagtggagaggctctgggattatgggatgagtagctccccacatgttctaagaaacagggctcagagtggcagtgtccctcagttcaagaaagttgttttccaggaatttactgatggctcctttactcagcccttataccgtggagaactaaatgaacatttgggactcctggggccatatataagagcagaagttgaagataatatcatggtaactttcagaaatcaggcctctcgtccctattccttctattctagccttatttcttatgaggaagatcagaggcaaggagcagaacctagaaaaaactttgtcaagcctaatgaaaccaaaacttacttttggaaagtgcaacatcatatggcacccactaaagatgagtttgactgcaaagcctgggcttatttctctgatgttgacctggaaaaagatgtgcactcaggcctgattggaccccttctggtctgccacactaacacactgaaccctgctcatgggagacaagtgacagtacaggaatttgctctgtttttcaccatctttgatgagaccaaaagctggtacttcactgaaaatatggaaagaaactgcagggctccctgcaatatccagatggaagatcccacttttaaagagaattatcgcttccatgcaatcaatggctacataatggatacactacctggcttagtaatggctcaggatcaaaggattcgatggtatctgctcagcatgggcagcaatgaaaacatccattctattcatttcagtggacatgtgttcactgtacgaaaaaaagaggagtataaaatggcactgtacaatctctatccaggtgtttttgagacagtggaaatgttaccatccaaagctggaatttggcgggtggaatgccttattggcgagcatctacatgctgggatgagcacactttttctggtgtacagcaataagtgtcagactcccctgggaatggcttctggacacattagagattttcagattacagcttcaggacaatatggacagtgggccccaaagctggccagacttcattattccggatcaatcaatgcctggagcaccaaggagcccttttcttggatcaaggtggatctgttggcaccaatgattattcacggcatcaagacccagggtgcccgtcagaagttctccagcctctacatctctcagtttatcatcatgtatagtcttgatgggaagaagtggcagacttatcgaggaaattccactggaaccttaatggtcttctttggcaatgtggattcatctgggataaaacacaatatttttaaccctccaattattgctcgatacatccgtttgcacccaactcattatagcattcgcagcactcttcgcatggagttgatgggctgtgatttaaatagttgcagcatgccattgggaatggagagtaaagcaatatcagatgcacagattactgcttcatcctactttaccaatatgtttgccacctggtctccttcaaaagctcgacttcacctccaagggaggagtaatgcctggagacctcaggtgaataatccaaaagagtggctgcaagtggacttccagaagacaatgaaagtcacaggagtaactactcagggagtaaaatctctgcttaccagcatgtatgtgaaggagttcctcatctccagcagtcaagatggccatcagtggactctcttttttcagaatggcaaagtaaaggtttttcagggaaatcaagactccttcacacctgtggtgaactctctagacccaccgttactgactcgctaccttcgaattcacccccagagttgggtgcaccagattgccctgaggatggaggttctgggctgcgaggcacaggacctctactga

SEQ ID NO: 39 - DNA, 4497 bp, synthetic construct
  source 1..4497: mol_type = other DNA
gccaccagaagatactacctgggtgcagtggaactgtcatgggactatatgcaaagtgatctcggtgagctgcctgtggacgcaagatttcctcctagagtgccaaaatcttttccattcaacacctcagtcgtgtacaaaaagactctgtttgtagaattcacggatcaccttttcaacatcgctaagccaaggccaccctggatgggtctgctaggtcctaccatccaggctgaggtttatgatacagtggtcattacacttaagaacatggcttcccatcctgtcagtcttcatgctgttggtgtatcctactggaaagcttctgagggagctgaatatgatgatcagaccagtcaaagggagaaagaagatgataaagtcttccctggtggaagccatacatatgtctggcaggtcctgaaagagaatggtccaatggcctctgacccactgtgccttacctactcatatctttctcatgtggacctggtaaaagacttgaattcaggcctcattggagccctactagtatgtagagaagggagtctggccaaggaaaagacacagaccttgcacaaatttatactactttttgctgtatttgatgaagggaaaagttggcactcagaaacaaagaactccttgatgcaggatagggatgctgcatctgctcgggcctggcctaaaatgcacacagtcaatggttatgtaaacaggtctctgccaggtctgattggatgccacaggaaatcagtctattggcatgtgattggaatgggcaccactcctgaagtgcactcaatattcctcgaaggtcacacatttcttgtgaggaaccatcgccaggcgtccttggaaatctcgccaataactttccttactgctcaaacactcttgatggaccttggacagtttctactgttttgtcatatctcttcccaccaacatgatggcatggaagcttatgtcaaagtagacagctgtccagaggaaccccaactacgaatgaaaaataatgaagaagcggaagactatgatgatgatcttactgattctgaaatggatgtggtcaggtttgatgatgacaactctccttcctttatccaaattcgctcagttgccaagaagcatcctaaaacttgggtacattacattgctgctgaagaggaggactgggactatgctcccttagtcctcgcccccgatgacagaagttataaaagtcaatatttgaacaatggccctcagcggattggtaggaagtacaaaaaagtccgatttatggcatacacagatgaaacctttaagactcgtgaagctattcagcatgaatcaggaatcttgggacctttactttatggggaagttggagacacactgttgattatatttaagaatcaagcaagcagaccatataacatctaccctcacggaatcactgatgtccgtcctttgtattcaaggagattaccaaaaggtgtaaaacatttgaaggattttccaattctgccaggagaaatattcaaatataaatggacagtgactgtagaagatgggccaactaaatcagatcctcggtgcctgacccgctattactctagtttcgttaatatggagagagatctagcttcaggactcattggccctctcctcatctgctacaaagaatctgtagatcaaagaggaaaccagataatgtcagacaagaggaatgtcatcctgttttctgtatttgatgagaaccgaagctggtacctcacagagaatatacaacgctttctccccaatccagctggagtgcagcttgaggatccagagttccaagcctccaacatcatgcacagcatcaatggctatgtttttgatagtttgcagttgtcagtttgtttgcatgaggtggcatactggtacattctaagcattggagcacagactgacttcctttctgtcttcttctctggatataccttcaaacacaaaatggtctatgaagacacactcaccctattcccattctcaggagaaactgtcttcatgtcgatggaaaacccaggtctatggattctggggtgccacaactcagactttcggaacagaggcatgaccgccttactgaaggtttctagttgtgacaagaacactggtgattattacgaggacagttatgaagatatttcagcatacttgctgagtaaaaacaatgccattgaaccaagaagcttcagccagaattctagacaccctagcaccagacagaaacagtttaatgccactaatgtgtctaacaacagcaacaccagcaatgacagcaatgtgtctaacaagacatctaacaacagcaacgccacaaacaagaccaacaacacaaatgatagcacaaaccggaccaaccagaccaataccagccagcagaacttcgtgacccagagaagtaagagagaaataactcgtactactcttcagtcagatcaagaggaaattgactatgatgataccatatcagttgaaatgaagaaggaagattttgacatttatgatgaggatgaaaatcagagcccccgcagctttcaaaagaaaacacgacactattttattgctgcagtggagaggctctgggattatgggatgagtagctccccacatgttctaagaaacagggctcagagtggcagtgtccctcagttcaagaaagttgttttccaggaatttactgatggctcctttactcagcccttataccgtggagaactaaatgaacatttgggactcctggggccatatataagagcagaagttgaagataatatcatggtaactttcagaaatcaggcctctcgtccctattccttctattctagccttatttcttatgaggaagatcagaggcaaggagcagaacctagaaaaaactttgtcaagcctaatgaaaccaaaacttacttttggaaagtgcaacatcatatggcacccactaaagatgagtttgactgcaaagcctgggcttatttctctgatgttgacctggaaaaagatgtgcactcaggcctgattggaccccttctggtctgccacactaacacactgaaccctgctcatgggagacaagtgacagtacaggaatttgctctgtttttcaccatctttgatgagaccaaaagctggtacttcactgaaaatatggaaagaaactgcagggctccctgcaatatccagatggaagatcccacttttaaagagaattatcgcttccatgcaatcaatggctacataatggatacactacctggcttagtaatggctcaggatcaaaggattcgatggtatctgctcagcatgggcagcaatgaaaacatccattctattcatttcagtggacatgtgttcactgtacgaaaaaaagaggagtataaaatggcactgtacaatctctatccaggtgtttttgagacagtggaaatgttaccatccaaagctggaatttggcgggtggaatgccttattggcgagcatctacatgctgggatgagcacactttttctggtgtacagcaataagtgtcagactcccctgggaatggcttctggacacattagagattttcagattacagcttcaggacaatatggacagtgggccccaaagctggccagacttcattattccggatcaatcaatgcctggagcaccaaggagcccttttcttggatcaaggtggatctgttggcaccaatgattattcacggcatcaagacccagggtgcccgtcagaagttctccagcctctacatctctcagtttatcatcatgtatagtcttgatgggaagaagtggcagacttatcgaggaaattccactggaaccttaatggtcttctttggcaatgtggattcatctgggataaaacacaatatttttaaccctccaattattgctcgatacatccgtttgcacccaactcattatagcattcgcagcactcttcgcatggagttgatgggctgtgatttaaatagttgcagcatgccattgggaatggagagtaaagcaatatcagatgcacagattactgcttcatcctactttaccaatatgtttgccacctggtctccttcaaaagctcgacttcacctccaagggaggagtaatgcctggagacctcaggtgaataatccaaaagagtggctgcaagtggacttccagaagacaatgaaagtcacaggagtaactactcagggagtaaaatctctgcttaccagcatgtatgtgaaggagttcctcatctccagcagtcaagatggccatcagtggactctcttttttcagaatggcaaagtaaaggtttttcagggaaatcaagactccttcacacctgtggtgaactctctagacccaccgttactgactcgctaccttcgaattcacccccagagttgggtgcaccagattgccctgaggatggaggttctgggctgcgaggcacaggacctctactga

SEQ ID NO: 40 - protein, 2122 aa, synthetic construct; identical to SEQ ID NO: 11

SEQ ID NO: 41 - protein, 1455 aa, synthetic construct; identical to SEQ ID NO: 12

SEQ ID NO: 42 - protein, 1445 aa, synthetic construct; identical to SEQ ID NO: 13

SEQ ID NO: 43 - protein, 1496 aa, synthetic construct; identical to SEQ ID NO: 5

SEQ ID NO: 44 - protein, 1498 aa, synthetic construct; identical to SEQ ID NO: 6

SEQ ID NO: 45 - DNA, 4317 bp, synthetic construct
  source 1..4317: mol_type = other DNA
gccaccaggagatactacctgggggctgtggagctgagctgggactacatgcagtctgacctgggggagctgcctgtggatgccaggttcccccccagagtgcccaagagcttccccttcaacacctctgtggtgtacaagaagaccctgtttgtggagttcactgaccacctgttcaacattgccaagcccaggcccccctggatgggcctgctgggccccaccatccaggctgaggtgtatgacactgtggtgatcaccctgaagaacatggccagccaccctgtgagcctgcatgctgtgggggtgagctactggaaggcctctgagggggctgagtatgatgaccagaccagccagagggagaaggaggatgacaaggtgttccctgggggcagccacacctatgtgtggcaggtgctgaaggagaatggccccatggcctctgaccccctgtgcctgacctacagctacctgagccatgtggacctggtgaaggacctgaactctggcctgattggggccctgctggtgtgcagggagggcagcctggccaaggagaagacccagaccctgcacaagttcatcctgctgtttgctgtgtttgatgagggcaagagctggcactctgaaaccaagaacagcctgatgcaggacagggatgctgcctctgccagggcctggcccaagatgcacactgtgaatggctatgtgaacaggagcctgcctggcctgattggctgccacaggaagtctgtgtactggcatgtgattggcatgggcaccacccctgaggtgcacagcatcttcctggagggccacaccttcctggtcaggaaccacaggcaggccagcctggagatcagccccatcaccttcctgactgcccagaccctgctgatggacctgggccagttcctgctgttctgccacatcagcagccaccagcatgatggcatggaggcctatgtgaaggtggacagctgccctgaggagccccagctgaggatgaagaacaatgaggaggctgaggactatgatgatgacctgactgactctgagatggatgtggtgaggtttgatgatgacaacagccccagcttcatccagatcaggtctgtggccaagaagcaccccaagacctgggtgcactacattgctgctgaggaggaggactgggactatgcccccctggtgctggcccctgatgacaggagctacaagagccagtacctgaacaatggcccccagaggattggcaggaagtacaagaaggtcaggttcatggcctacactgatgaaaccttcaagaccagggaggccatccagcatgagtctggcatcctgggccccctgctgtatggggaggtgggggacaccctgctgatcatcttcaagaaccaggccagcaggccctacaacatctacccccatggcatcactgatgtgaggcccctgtacagcaggaggctgcccaagggggtgaagcacctgaaggacttccccatcctgcctggggagatcttcaagtacaagtggactgtgactgtggaggatggccccaccaagtctgaccccaggtgcctgaccagatactacagcagctttgtgaacatggagagggacctggcctctggcctgattggccccctgctgatctgctacaaggagtctgtggaccagaggggcaaccagatcatgtctgacaagaggaatgtgatcctgttctctgtgtttgatgagaacaggagctggtacctgactgagaacatccagaggttcctgcccaaccctgctggggtgcagctggaggaccctgagttccaggccagcaacatcatgcacagcatcaatggctatgtgtttgacagcctgcagctgtctgtgtgcctgcatgaggtggcctactggtacatcctgagcattggggcccagactgacttcctgtctgtgttcttctctggctacaccttcaagcacaagatggtgtatgaggacaccctgaccctgttccccttctctggggagactgtgttcatgagcatggagaaccctggcctgtggattctgggctgccacaactctgacttcaggaacaggggcatgactgccctgctgaaagtctccagctgtgacaagaacactggggactactatgaggacagctatgaggacatctctgcctacctgctgagcaagaacaatgccattgagcccaggagcttcagccagaatcccccagtgctgaagaggcaccagagggagatcaccaggaccaccctgcagtctgaccaggaggagattgactatgatgacaccatctctgtggagatgaagaaggaggactttgacatctacgacgaggacgagaaccagagccccaggagcttccagaagaagaccaggcactacttcattgctgctgtggagaggctgtgggactatggcatgagcagcagcccccatgtgctgaggaacagggcccagtctggctctgtgccccagttcaagaaggtggtgttccaggagttcactgatggcagcttcacccagcccctgtacagaggggagctgaatgagcacctgggcctgctgggcccctacatcagggctgaggtggaggacaacatcatggtgaccttcaggaaccaggccagcaggccctacagcttctacagcagcctgatcagctatgaggaggaccagaggcagggggctgagcccaggaagaactttgtgaagcccaatgaaaccaagacctacttctggaaggtgcagcaccacatggcccccaccaaggatgagtttgactgcaaggcctgggcctacttctctgatgtggacctggagaaggatgtgcactctggcctgattggccccctgctggtgtgccacaccaacaccctgaaccctgcccatggcaggcaggtgactgtgcaggagtttgccctgttcttcaccatctttgatgaaaccaagagctggtacttcactgagaacatggagaggaactgcagggccccctgcaacatccagatggaggaccccaccttcaaggagaactacaggttccatgccatcaatggctacatcatggacaccctgcctggcctggtgatggcccaggaccagaggatcaggtggtacctgctgagcatgggcagcaatgagaacatccacagcatccacttctctggccatgtgttcactgtgaggaagaaggaggagtacaagatggccctgtacaacctgtaccctggggtgtttgagactgtggagatgctgcccagcaaggctggcatctggagggtggagtgcctgattggggagcacctgcatgctggcatgagcaccctgttcctggtgtacagcaacaagtgccagacccccctgggcatggcctctggccacatcagggacttccagatcactgcctctggccagtatggccagtgggcccccaagctggccaggctgcactactctggcagcatcaatgcctggagcaccaaggagcccttcagctggatcaaggtggacctgctggcccccatgatcatccatggcatcaagacccagggggccaggcagaagttcagcagcctgtacatcagccagttcatcatcatgtacagcctggatggcaagaagtggcagacctacaggggcaacagcactggcaccctgatggtgttctttggcaatgtggacagctctggcatcaagcacaacatcttcaacccccccatcattgccagatacatcaggctgcaccccacccactacagcatcaggagcaccctgaggatggagctgatgggctgtgacctgaacagctgcagcatgcccctgggcatggagagcaaggccatctctgatgcccagatcactgccagcagctacttcaccaacatgtttgccacctggagccccagcaaggccaggctgcacctgcagggcaggagcaatgcctggaggccccaggtcaacaaccccaaggagtggctgcaggtggacttccagaagaccatgaaggtgactggggtgaccacccagggggtgaagagcctgctgaccagcatgtatgtgaaggagttcctgatcagcagcagccaggatggccaccagtggaccctgttcttccagaatggcaaggtgaaggtgttccagggcaaccaggacagcttcacccctgtggtgaacagcctggacccccccctgctgaccagatacctgaggattcacccccagagctgggtgcaccagattgccctgaggatggaggtgctgggctgtgaggcccaggacctgtactga

SEQ ID NO: 46 - DNA, 5928 bp, synthetic construct
  source 1..5928: mol_type = other DNA
ccccaactggggtaacctttgggctccccgggcgcgactagtgaattcgtcaatattggccattagccatattattcattggttatatagcataaatcaatattggctattggccattgcatacgttgtatctatatcataatatgtacatttatattggctcatgtccaatatgaccgccatgttggtgtggaaagtccccaggctccccagcaggcagaagtatgcaaagcatgcatctcaattagtcagcaaccaggcattgattattgactagttattaatagtaatcaattacggggtcattagttcatagcccatatatggagttccgcgttacataacttacggtaaatggcccgcctggctgaccgcccaacgacccccgcccattgacgtcaataatgacgtatgttcccatagtaacgccaatagggactttccattgacgtcaatgggtggagtatttacggtaaactgcccacttggcagtacatcaagtgtatcatatgccaagtccgccccctattgacgtcaatgacggtaaatggcccgcctggcattatgcccagtacatgaccttacgggactttcctacttggcagtacatctacgtattagtcatcgctattaccatggtgatgcggttttggcagtacaccaatgggcgtggatagcggtttgactcacggggatttccaagtctccaccccattgacgtcaatgggagtttgttttggcaccaaaatcaacgggactttccaaaatgtcgtaataaccccgccccgttgacgcaaatgggcggtaggcgtgtacggtgggaggtctatataagcagaggtcgtttagtgaaccgtcagatcactagtagctttattgcggtagtttatcacagttaaattgctaacgcagtcagtgctcgactgatcacaggtaagtatcaaggttacaagacaggtttaaggaggccaatagaaactgggcttgtcgagacagagaagattcttgcgtttctgataggcacctattggtcttactgacatccactttgcctttctctccacaggggtaccgaagccgctagcgctaccggtgccaccatgcaaatagagctctccacctgcttctttctgtgccttttgcgattctgctttagtgccaccagaagatactacctgggtgcagtggaactgtcatgggactatatgcaaagtgatctcggtgagctgcctgtggacgcaagatttcctcctagagtgccaaaatcttttccattcaacacctcagtcgtgtacaaaaagactctgtttgtagaattcacggatcaccttttcaacatcgctaagccaaggccaccctggatgggtctgctaggtcctaccatccaggctgaggtttatgatacagtggtcattacacttaagaacatggcttcccatcctgtcagtcttcatgctgttggtgtatcctactggaaagcttctgagggagctgaatatgatgatcagaccagtcaaagggagaaagaagatgataaagtcttccctggtggaagccatacatatgtctggcaggtcctgaaagagaatggtccaatggcctctgacccactgtgccttacctactcatatctttctcatgtggacctggtaaaagacttgaattcaggcctcattggagccctactagtatgtagagaagggagtctggccaaggaaaagacacagaccttgcacaaatttatactactttttgctgtatttgatgaagggaaaagttggcactcagaaacaaagaactccttgatgcaggatagggatgctgcatctgctcgggcctggcctaaaatgcacacagtcaatggttatgtaaacaggtctctgccaggtctgattggatgccacaggaaatcagtctattggcatgtgattggaatgggcaccactcctgaagtgcactcaatattcctcgaaggtcacacatttcttgtgaggaaccatcgccaggcgtccttggaaatctcgccaataactttccttactgctcaaacactcttgatggaccttggacagtttctactgttttgtcatatctcttcccaccaacatgatggcatggaagcttatgtcaaagtagacagctgtccagaggaaccccaactacgaatgaaaaataatgaagaagcggaagactatgatgatgatcttactgattctgaaatggatgtggtcaggtttgatgatgacaactctccttcctttatccaaattcgctcagttgccaagaagcatcctaaaacttgggtacattacattgctgctgaagaggaggactgggactatgctcccttagtcctcgcccccgatgacagaagttataaaagtcaatatttgaacaatggccctcagcggattggtaggaagtacaaaaaagtccgatttatggcatacacagatgaaacctttaagactcgtgaagctattcagcatgaatcaggaatcttgggacctttactttatggggaagttggagacacactgttgattatatttaagaatcaagcaagcagaccatataacatctaccctcacggaatcactgatgtccgtcctttgtattcaaggagattaccaaaaggtgtaaaacatttgaaggattttccaattctgccaggagaaatattcaaatataaatggacagtgactgtagaagatgggccaactaaatcagatcctcggtgcctgacccgctattactctagtttcgttaatatggagagagatctagcttcaggactcattggccctctcctcatctgctacaaagaatctgtagatcaaagaggaaaccagataatgtcagacaagaggaatgtcatcctgttttctgtatttgatgagaaccgaagctggtacctcacagagaatatacaacgctttctccccaatccagctggagtgcagcttgaggatccagagttccaagcctccaacatcatgcacagcatcaatggctatgtttttgatagtttgcagttgtcagtttgtttgcatgaggtggcatactggtacattctaagcattggagcacagactgacttcctttctgtcttcttctctggatataccttcaaacacaaaatggtctatgaagacacactcaccctattcccattctcaggagaaactgtcttcatgtcgatggaaaacccaggtctatggattctggggtgccacaactcagactttcggaacagaggcatgaccgccttactgaaggtttctagttgtgacaagaacactggtgattattacgaggacagttatgaagatatttcagcatacttgctgagtaaaaacaatgccattgaaccaagaagcttcagccagaatagcagacaccctagcaccagacagaaacagtttaatgccactaatgtgagcaacaacagcaacaccagcaatgacagcaatgtgtctaacaagacatctaacaacagcaatgccacaaacaagaccaacaacacaaatgatagcacaaacaggaccaaccagaccaataccagcccccctgtgctgaagagacatcagagggaaataactcgtactactcttcagtcagatcaagaggaaattgactatgatgataccatatcagttgaaatgaagaaggaagattttgacatttatgatgaggatgaaaatcagagcccccgcagctttcaaaagaaaacacgacactattttattgctgcagtggagaggctctgggattatgggatgagtagctccccacatgttctaagaaacagggctcagagtggcagtgtccctcagttcaagaaagttgttttccaggaatttactgatggctcctttactcagcccttataccgtggagaactaaatgaacatttgggactcctggggccatatataagagcagaagttgaagataatatcatggtaactttcagaaatcaggcctctcgtccctattccttctattctagccttatttcttatgaggaagatcagaggcaaggagcagaacctagaaaaaactttgtcaagcctaatgaaaccaaaacttacttttggaaagtgcaacatcatatggcacccactaaagatgagtttgactgcaaagcctgggcttatttctctgatgttgacctggaaaaagatgtgcactcaggcctgattggaccccttctggtctgccacactaacacactgaaccctgctcatgggagacaagtgacagtacaggaatttgctctgtttttcaccatctttgatgagaccaaaagctggtacttcactgaaaatatggaaagaaactgcagggctccctgcaatatccagatggaagatcccacttttaaagagaattatcgcttccatgcaatcaatggctacataatggatacactacctggcttagtaatggctcaggatcaaaggattcgatggtatctgctcagcatgggcagcaatgaaaacatccattctattcatttcagtggacatgtgttcactgtacgaaaaaaagaggagtataaaatggcactgtacaatctctatccaggtgtttttgagacagtggaaatgttaccatccaaagctggaatttggcgggtggaatgccttattggcgagcatctacatgctgggatgagcacactttttctggtgtacagcaataagtgtcagactcccctgggaatggcttctggacacattagagattttcagattacagcttcaggacaatatggacagtgggccccaaagctggccagacttcattattccggatcaatcaatgcctggagcaccaaggagcccttttcttggatcaaggtggatctgttggcaccaatgattattcacggcatcaagacccagggtgcccgtcagaagttctccagcctctacatctctcagtttatcatcatgtatagtcttgatgggaagaagtggcagacttatcgaggaaattccactggaaccttaatggtcttctttggcaatgtggattcatctgggataaaacacaatatttttaaccctccaattattgctcgatacatccgtttgcacccaactcattatagcattcgcagcactcttcgcatggagttgatgggctgtgatttaaatagttgcagcatgccattgggaatggagagtaaagcaatatcagatgcacagattactgcttcatcctactttaccaatatgtttgccacctggtctccttcaaaagctcgacttcacctccaagggaggagtaatgcctggagacctcaggtgaataatccaaaagagtggctgcaagtggacttccagaagacaatgaaagtcacaggagtaactactcagggagtaaaatctctgcttaccagcatgtatgtgaaggagttcctcatctccagcagtcaagatggccatcagtggactctcttttttcagaatggcaaagtaaaggtttttcagggaaatcaagactccttcacacctgtggtgaactctctagacccaccgttactgactcgctaccttcgaattcacccccagagttgggtgcaccagattgccctgaggatggaggttctgggctgcgaggcacaggacctctactgagatatctctagagtcgacagtactggtgatcagcctcgactgtgccttctagttgccagccatctgttgtttgcccctcccccgtgccttccttgaccctggaaggtgccactcccactgtcctttcctaataaaatgaggaaattgcatcgcattgtctgagtaggtgtcattctattctggggggtggggtggggcaggacagcaagggggaggattgggaagacaatagcaggcatgctggggatgcggtgggctctatggaaccagctggggcccg

SEQ ID NO: 47 - DNA, 5934 bp, synthetic construct
  source 1..5934: mol_type = other DNA
ccccaactggggtaacctttgggctccccgggcgcgactagtgaattcgtcaatattggccattagccatattattcattggttatatagcataaatcaatattggctattggccattgcatacgttgtatctatatcataatatgtacatttatattggctcatgtccaatatgaccgccatgttggtgtggaaagtccccaggctccccagcaggcagaagtatgcaaagcatgcatctcaattagtcagcaaccaggcattgattattgactagttattaatagtaatcaattacggggtcattagttcatagcccatatatggagttccgcgttacataacttacggtaaatggcccgcctggctgaccgcccaacgacccccgcccattgacgtcaataatgacgtatgttcccatagtaacgccaatagggactttccattgacgtcaatgggtggagtatttacggtaaactgcccacttggcagtacatcaagtgtatcatatgccaagtccgccccctattgacgtcaatgacggtaaatggcccgcctggcattatgcccagtacatgaccttacgggactttcctacttggcagtacatctacgtattagtcatcgctattaccatggtgatgcggttttggcagtacaccaatgggcgtggatagcggtttgactcacggggatttccaagtctccaccccattgacgtcaatgggagtttgttttggcaccaaaatcaacgggactttccaaaatgtcgtaataaccccgccccgttgacgcaaatgggcggtaggcgtgtacggtgggaggtctatataagcagaggtcgtttagtgaaccgtcagatcactagtagctttattgcggtagtttatcacagttaaattgctaacgcagtcagtgctcgactgatcacaggtaagtatcaaggttacaagacaggtttaaggaggccaatagaaactgggcttgtcgagacagagaagattcttgcgtttctgataggcacctattggtcttactgacatccactttgcctttctctccacaggggtaccgaagccgctagcgctaccggtgccaccatgcaaatagagctctccacctgcttctttctgtgccttttgcgattctgctttagtgccaccagaagatactacctgggtgcagtggaactgtcatgggactatatgcaaagtgatctcggtgagctgcctgtggacgcaagatttcctcctagagtgccaaaatcttttccattcaacacctcagtcgtgtacaaaaagactctgtttgtagaattcacggatcaccttttcaacatcgctaagccaaggccaccctggatgggtctgctaggtcctaccatccaggctgaggtttatgatacagtggtcattacacttaagaacatggcttcccatcctgtcagtcttcatgctgttggtgtatcctactggaaagcttctgagggagctgaatatgatgatcagaccagtcaaagggagaaagaagatgataaagtcttccctggtggaagccatacatatgtctggcaggtcctgaaagagaatggtccaatggcctctgacccactgtgccttacctactcatatctttctcatgtggacctggtaaaagacttgaattcaggcctcattggagccctactagtatgtagagaagggagtctggccaaggaaaagacacagaccttgcacaaatttatactactttttgctgtatttgatgaagggaaaagttggcactcagaaacaaagaactccttgatgcaggatagggatgctgcatctgctcgggcctggcctaaaatgcacacagtcaatggttatgtaaacaggtctctgccaggtctgattggatgccacaggaaatcagtctattggcatgtgattggaatgggcaccactcctgaagtgcactcaatattcctcgaaggtcacacatttcttgtgaggaaccatcgccaggcgtccttggaaatctcgccaataactttccttactgctcaaacactcttgatggaccttggacagtttctactgttttgtcatatctcttcccaccaacatgatggcatggaagcttatgtcaaagtagacagctgtccagaggaaccccaactacgaatgaaaaataatgaagaagcggaagactatgatgatgatcttactgattctgaaatggatgtggtcaggtttgatgatgacaactctccttcctttatccaaattcgctcagttgccaagaagcatcctaaaacttgggtacattacattgctgctgaagaggaggactgggactatgctcccttagtcctcgcccccgatgacagaagttataaaagtcaatatttgaacaatggccctcagcggattggtaggaagtacaaaaaagtccgatttatggcatacacagatgaaacctttaagactcgtgaagctattcagcatgaatcaggaatcttgggacctttactttatggggaagttggagacacactgttgattatatttaagaatcaagcaagcagaccatataacatctaccctcacggaatcactgatgtccgtcctttgtattcaaggagattaccaaaaggtgtaaaacatttgaaggattttccaattctgccaggagaaatattcaaatataaatggacagtgactgtagaagatgggccaactaaatcagatcctcggtgcctgacccgctattactctagtttcgttaatatggagagagatctagcttcaggactcattggccctctcctcatctgctacaaagaatctgtagatcaaagaggaaaccagataatgtcagacaagaggaatgtcatcctgttttctgtatttgatgagaaccgaagctggtacctcacagagaatatacaacgctttctccccaatccagctggagtgcagcttgaggatccagagttccaagcctccaacatcatgcacagcatcaatggctatgtttttgatagtttgcagttgtcagtttgtttgcatgaggtggcatactggtacattctaagcattggagcacagactgacttcctttctgtcttcttctctggatataccttcaaacacaaaatggtctatgaagacacactcaccctattcccattctcaggagaaactgtcttcatgtcgatggaaaacccaggtctatggattctggggtgccacaactcagactttcggaacagaggcatgaccgccttactgaaggtttctagttgtgacaagaacactggtgattattacgaggacagttatgaagatatttcagcatacttgctgagtaaaaacaatgccattgaaccaagaagcttcagccagaattctagacaccctagcaccagacagaaacagtttaatgccactaatgtgtctaacaacagcaacaccagcaatgacagcaatgtgtctaacaagacatctaacaacagcaacgccacaaacaagaccaacaacacaaatgatagcacaaaccggaccaaccagaccaataccagccagcagaacttcgtgacccagagaagtaagagagaaataactcgtactactcttcagtcagatcaagaggaaattgactatgatgataccatatcagttgaaatgaagaaggaagattttgacatttatgatgaggatgaaaatcagagcccccgcagctttcaaaagaaaacacgacactattttattgctgcagtggagaggctctgggattatgggatgagtagctccccacatgttctaagaaacagggctcagagtggcagtgtccctcagttcaagaaagttgttttccaggaatttactgatggctcctttactcagcccttataccgtggagaactaaatgaacatttgggactcctggggccatatataagagcagaagttgaagataatatcatggtaactttcagaaatcaggcctctcgtccctattccttctattctagccttatttcttatgaggaagatcagaggcaaggagcagaacctagaaaaaactttgtcaagcctaatgaaaccaaaacttacttttggaaagtgcaacatcatatggcacccactaaagatgagtttgactgcaaagcctgggcttatttctctgatgttgacctggaaaaagatgtgcactcaggcctgattggaccccttctggtctgccacactaacacactgaaccctgctcatgggagacaagtgacagtacaggaatttgctctgtttttcaccatctttgatgagaccaaaagctggtacttcactgaaaatatggaaagaaactgcagggctccctgcaatatccagatggaagatcccacttttaaagagaattatcgcttccatgcaatcaatggctacataatggatacactacctggcttagtaatggctcaggatcaaaggattcgatggtatctgctcagcatgggcagcaatgaaaacatccattctattcatttcagtggacatgtgttcactgtacgaaaaaaagaggagtataaaatggcactgtacaatctctatccaggtgtttttgagacagtggaaatgttaccatccaaagctggaatttggcgggtggaatgccttattggcgagcatctacatgctgggatgagcacactttttctggtgtacagcaataagtgtcagactcccctgggaatggcttctggacacattagagattttcagattacagcttcaggacaatatggacagtgggccccaaagctggccagacttcattattccggatcaatcaatgcctggagcaccaaggagcccttttcttggatcaaggtggatctgttggcaccaatgattattcacggcatcaagacccagggtgcccgtcagaagttctccagcctctacatctctcagtttatcatcatgtatagtcttgatgggaagaagtggcagacttatcgaggaaattccactggaaccttaatggtcttctttggcaatgtggattcatctgggataaaacacaatatttttaaccctccaattattgctcgatacatccgtttgcacccaactcattatagcattcgcagcactcttcgcatggagttgatgggctgtgatttaaatagttgcagcatgccattgggaatggagagtaaagcaatatcagatgcacagattactgcttcatcctactttaccaatatgtttgccacctggtctccttcaaaagctcgacttcacctccaagggaggagtaatgcctggagacctcaggtgaataatccaaaagagtggctgcaagtggacttccagaagacaatgaaagtcacaggagtaactactcagggagtaaaatctctgcttaccagcatgtatgtgaaggagttcctcatctccagcagtcaagatggccatcagtggactctcttttttcagaatggcaaagtaaaggtttttcagggaaatcaagactccttcacacctgtggtgaactctctagacccaccgttactgactcgctaccttcgaattcacccccagagttgggtgcaccagattgccctgaggatggaggttctgggctgcgaggcacaggacctctactgagatatctctagagtcgacagtactggtgatcagcctcgactgtgccttctagttgccagccatctgttgtttgcccctcccccgtgccttccttgaccctggaaggtgccactcccactgtcctttcctaataaaatgaggaaattgcatcgcattgtctgagtaggtgtcattctattctggggggtggggtggggcaggacagcaagggggaggattgggaagacaatagcaggcatgctggggatgcggtgggctctatggaaccagctggggcccg

SEQ ID NO: 48 - DNA, 5754 bp, synthetic construct
  source 1..5754: mol_type = other DNA
ccccaactggggtaacctttgggctccccgggcgcgactagtgaattcgtcaatattggccattagccatattattcattggttatatagcataaatcaatattggctattggccattgcatacgttgtatctatatcataatatgtacatttatattggctcatgtccaatatgaccgccatgttggtgtggaaagtccccaggctccccagcaggcagaagtatgcaaagcatgcatctcaattagtcagcaaccaggcattgattattgactagttattaatagtaatcaattacggggtcattagttcatagcccatatatggagttccgcgttacataacttacggtaaatggcccgcctggctgaccgcccaacgacccccgcccattgacgtcaataatgacgtatgttcccatagtaacgccaatagggactttccattgacgtcaatgggtggagtatttacggtaaactgcccacttggcagtacatcaagtgtatcatatgccaagtccgccccctattgacgtcaatgacggtaaatggcccgcctggcattatgcccagtacatgaccttacgggactttcctacttggcagtacatctacgtattagtcatcgctattaccatggtgatgcggttttggcagtacaccaatgggcgtggatagcggtttgactcacggggatttccaagtctccaccccattgacgtcaatgggagtttgttttggcaccaaaatcaacgggactttccaaaatgtcgtaataaccccgccccgttgacgcaaatgggcggtaggcgtgtacggtgggaggtctatataagcagaggtcgtttagtgaaccgtcagatcactagtagctttattgcggtagtttatcacagttaaattgctaacgcagtcagtgctcgactgatcacaggtaagtatcaaggttacaagacaggtttaaggaggccaatagaaactgggcttgtcgagacagagaagattcttgcgtttctgataggcacctattggtcttactgacatccactttgcctttctctccacaggggtaccgaagccgctagcgctaccggtgccaccatgcagattgagctgagcacctgcttcttcctgtgcctgctgaggttctgcttctctgccaccaggagatactacctgggggctgtggagctgagctgggactacatgcagtctgacctgggggagctgcctgtggatgccaggttcccccccagagtgcccaagagcttccccttcaacacctctgtggtgtacaagaagaccctgtttgtggagttcactgaccacctgttcaacattgccaagcccaggcccccctggatgggcctgctgggccccaccatccaggctgaggtgtatgacactgtggtgatcaccctgaagaacatggccagccaccctgtgagcctgcatgctgtgggggtgagctactggaaggcctctgagggggctgagtatgatgaccagaccagccagagggagaaggaggatgacaaggtgttccctgggggcagccacacctatgtgtggcaggtgctgaaggagaatggccccatggcctctgaccccctgtgcctgacctacagctacctgagccatgtggacctggtgaaggacctgaactctggcctgattggggccctgctggtgtgcagggagggcagcctggccaaggagaagacccagaccctgcacaagttcatcctgctgtttgctgtgtttgatgagggcaagagctggcactctgaaaccaagaacagcctgatgcaggacagggatgctgcctctgccagggcctggcccaagatgcacactgtgaatggctatgtgaacaggagcctgcctggcctgattggctgccacaggaagtctgtgtactggcatgtgattggcatgggcaccacccctgaggtgcacagcatcttcctggagggccacaccttcctggtcaggaaccacaggcaggccagcctggagatcagccccatcaccttcctgactgcccagaccctgctgatggacctgggccagttcctgctgttctgccacatcagcagccaccagcatgatggcatggaggcctatgtgaaggtggacagctgccctgaggagccccagctgaggatgaagaacaatgaggaggctgaggactatgatgatgacctgactgactctgagatggatgtggtgaggtttgatgatgacaacagccccagcttcatccagatcaggtctgtggccaagaagcaccccaagacctgggtgcactacattgctgctgaggaggaggactgggactatgcccccctggtgctggcccctgatgacaggagctacaagagccagtacctgaacaatggcccccagaggattggcaggaagtacaagaaggtcaggttcatggcctacactgatgaaaccttcaagaccagggaggccatccagcatgagtctggcatcctgggccccctgctgtatggggaggtgggggacaccctgctgatcatcttcaagaaccaggccagcaggccctacaacatctacccccatggcatcactgatgtgaggcccctgtacagcaggaggctgcccaagggggtgaagcacctgaaggacttccccatcctgcctggggagatcttcaagtacaagtggactgtgactgtggaggatggccccaccaagtctgaccccaggtgcctgaccagatactacagcagctttgtgaacatggagagggacctggcctctggcctgattggccccctgctgatctgctacaaggagtctgtggaccagaggggcaaccagatcatgtctgacaagaggaatgtgatcctgttctctgtgtttgatgagaacaggagctggtacctgactgagaacatccagaggttcctgcccaaccctgctggggtgcagctggaggaccctgagttccaggccagcaacatcatgcacagcatcaatggctatgtgtttgacagcctgcagctgtctgtgtgcctgcatgaggtggcctactggtacatcctgagcattggggcccagactgacttcctgtctgtgttcttctctggctacaccttcaagcacaagatggtgtatgaggacaccctgaccctgttccccttctctggggagactgtgttcatgagcatggagaaccctggcctgtggattctgggctgccacaactctgacttcaggaacaggggcatgactgccctgctgaaagtctccagctgtgacaagaacactggggactactatgaggacagctatgaggacatctctgcctacctgctgagcaagaacaatgccattgagcccaggagcttcagccagaatcccccagtgctgaagaggcaccagagggagatcaccaggaccaccctgcagtctgaccaggaggagattgactatgatgacaccatctctgtggagatgaagaaggaggactttgacatctacgacgaggacgagaaccagagccccaggagcttccagaagaagaccaggcactacttcattgctgctgtggagaggctgtgggactatggcatgagcagcagcccccatgtgctgaggaacagggcccagtctggctctgtgccccagttcaagaaggtggtgttccaggagttcactgatggcagcttcacccagcccctgtacagaggggagctgaatgagcacctgggcctgctgggcccctacatcagggctgaggtggaggacaacatcatggtgaccttcaggaaccaggccagcaggccctacagcttctacagcagcctgatcagctatgaggaggaccagaggcagggggctgagcccaggaagaactttgtgaagcccaatgaaaccaagacctacttctggaaggtgcagcaccacatggcccccaccaaggatgagtttgactgcaaggcctgggcctacttctctgatgtggacctggagaaggatgtgcactctggcctgattggccccctgctggtgtgccacaccaacaccctgaaccctgcccatggcaggcaggtgactgtgcaggagtttgccctgttcttcaccatctttgatgaaaccaagagctggtacttcactgagaacatggagaggaactgcagggccccctgcaacatccagatggaggaccccaccttcaaggagaactacaggttccatgccatcaatggctacatcatggacaccctgcctggcctggtgatggcccaggaccagaggatcaggtggtacctgctgagcatgggcagcaatgagaacatccacagcatccacttctctggccatgtgttcactgtgaggaagaaggaggagtacaagatggccctgtacaacctgtaccctggggtgtttgagactgtggagatgctgcccagcaaggctggcatctggagggtggagtgcctgattggggagcacctgcatgctggcatgagcaccctgttcctggtgtacagcaacaagtgccagacccccctgggcatggcctctggccacatcagggacttccagatcactgcctctggccagtatggccagtgggcccccaagctggccaggctgcactactctggcagcatcaatgcctggagcaccaaggagcccttcagctggatcaaggtggacctgctggcccccatgatcatccatggcatcaagacccagggggccaggcagaagttcagcagcctgtacatcagccagttcatcatcatgtacagcctggatggcaagaagtggcagacctacaggggcaacagcactggcaccctgatggtgttctttggcaatgtggacagctctggcatcaagcacaacatcttcaacccccccatcattgccagatacatcaggctgcaccccacccactacagcatcaggagcaccctgaggatggagctgatgggctgtgacctgaacagctgcagcatgcccctgggcatggagagcaaggccatctctgatgcccagatcactgccagcagctacttcaccaacatgtttgccacctggagccccagcaaggccaggctgcacctgcagggcaggagcaatgcctggaggccccaggtcaacaaccccaaggagtggctgcaggtggacttccagaagaccatgaaggtgactggggtgaccacccagggggtgaagagcctgctgaccagcatgtatgtgaaggagttcctgatcagcagcagccaggatggccaccagtggaccctgttcttccagaatggcaaggtgaaggtgttccagggcaaccaggacagcttcacccctgtggtgaacagcctggacccccccctgctgaccagatacctgaggattcacccccagagctgggtgcaccagattgccctgaggatggaggtgctgggctgtgaggcccaggacctgtactgagatatctctagagtcgacagtactggtgatcagcctcgactgtgccttctagttgccagccatctgttgtttgcccctcccccgtgccttccttgaccctggaaggtgccactcccactgtcctttcctaataaaatgaggaaattgcatcgcattgtctgagtaggtgtcattctattctggggggtggggtggggcaggacagcaagggggaggattgggaagacaatagcaggcatgctggggatgcggtgggctctatggaaccagctggggcccg

SEQ ID NO: 49 - DNA, 5754 bp, synthetic construct
  source 1..5754: mol_type = other DNA
ccccaactggggtaacctttgggctccccgggcgcgactagtgaattcgtcaatattggccattagccatattattcattggttatatagcataaatcaatattggctattggccattgcatacgttgtatctatatcataatatgtacatttatattggctcatgtccaatatgaccgccatgttggtgtggaaagtccccaggctccccagcaggcagaagtatgcaaagcatgcatctcaattagtcagcaaccaggcattgattattgactagttattaatagtaatcaattacggggtcattagttcatagcccatatatggagttccgcgttacataacttacggtaaatggcccgcctggctgaccgcccaacgacccccgcccattgacgtcaataatgacgtatgttcccatagtaacgccaatagggactttccattgacgtcaatgggtggagtatttacggtaaactgcccacttggcagtacatcaagtgtatcatatgccaagtccgccccctattgacgtcaatgacggtaaatggcccgcctggcattatgcccagtacatgaccttacgggactttcctacttggcagtacatctacgtattagtcatcgctattaccatggtgatgcggttttggcagtacaccaatgggcgtggatagcggtttgactcacggggatttccaagtctccaccccattgacgtcaatgggagtttgttttggcaccaaaatcaacgggactttccaaaatgtcgtaataaccccgccccgttgacgcaaatgggcggtaggcgtgtacggtgggaggtctatataagcagaggtcgtttagtgaaccgtcagatcactagtagctttattgcggtagtttatcacagttaaattgctaacgcagtcagtgctcgactgatcacaggtaagtatcaaggttacaagacaggtttaaggaggccaatagaaactgggcttgtcgagacagagaagattcttgcgtttctgataggcacctattggtcttactgacatccactttgcctttctctccacaggggtaccgaagccgctagcgctaccggtgccaccatgcagattgaactgagcacctgcttcttcctgtgtctgctgagattctgcttctctgccaccaggaggtactacctgggggctgtggagctgagctgggactacatgcagtctgacctgggggagctgcctgtggatgctaggttcccccctagagtgcccaagtccttccccttcaacacttctgtggtgtacaagaagaccctgtttgtggagttcactgaccacctgtttaacattgccaagcccaggcccccttggatgggcctgctggggcccaccatccaggctgaggtgtatgacactgtggtgatcaccctgaagaacatggccagccatcctgtgagcctgcatgctgtgggggtgagctactggaaggccagcgagggggctgagtatgatgaccagactagccagagggagaaggaggatgacaaggtgtttcctggaggcagccacacctatgtgtggcaggtgctgaaggagaatggccccatggcctctgaccccctgtgcctgacctacagctacctgagccatgtggatctggtgaaggacctgaactctggcctgattggggctctgctggtgtgtagagagggcagcctggctaaggagaagacccagaccctgcataagttcatcctgctgtttgctgtgtttgatgagggcaagagctggcactctgagaccaagaacagcctgatgcaggatagggatgctgcctctgccagggcttggcccaagatgcacactgtgaatggctatgtgaataggagcctgcctggcctgattggctgccacaggaagtctgtgtactggcatgtgattggaatgggcacaacccctgaggtccatagcatcttcctggagggccacactttcctggtgaggaaccacagacaggcctctctggagattagccccatcaccttcctgactgctcagactctgctgatggacctgggccagttcctgctgttttgccatattagctctcaccagcatgatggcatggaggcctatgtgaaggtggacagctgccctgaggagcctcagctgaggatgaagaacaatgaggaggctgaagactatgatgatgacctgactgattctgagatggatgtggtgaggtttgatgatgacaatagccccagcttcattcagatcagatctgtggccaaaaagcaccccaagacctgggtgcattacattgctgctgaagaggaggactgggactatgcccctctggtgctggcccctgatgataggagctataagagccagtacctgaacaatgggccccagaggattggcagaaagtacaagaaggtgaggttcatggcttacactgatgaaaccttcaaaaccagggaggccatccagcatgagtctggcatcctgggccctctgctgtatggagaggtgggagacaccctgctgatcatcttcaagaaccaggccagcaggccctacaacatctatcctcatggcatcactgatgtgagacctctgtacagcaggaggctgcctaagggggtgaaacacctgaaggactttcccatcctgcctggggagatcttcaagtataagtggactgtgactgtggaggatggccctaccaagtctgaccccaggtgtctgacaaggtattacagcagctttgtgaacatggagagggacctggcctctggcctgattggccctctgctgatctgctacaaggagtctgtggaccagaggggcaaccagatcatgtctgacaagaggaatgtgatcctgttctctgtgtttgatgagaataggagctggtatctgactgagaacatccagagattcctgcccaatcctgctggggtgcagctggaggaccctgagtttcaggccagcaatatcatgcacagcatcaatggctatgtgtttgacagcctgcagctgtctgtgtgcctgcatgaggtggcctactggtacatcctgagcattggagcccagactgattttctgtctgtgttcttttctggctataccttcaagcacaagatggtgtatgaggacaccctgaccctgttccccttctctggggagactgtgttcatgtctatggagaatcctgggctgtggattctgggctgccacaactctgatttcaggaacaggggcatgactgccctgctgaaggtgagcagctgtgacaagaacactggggactactatgaggatagctatgaggacatttctgcttatctgctgtctaagaataatgccattgagcccaggagcttcagccagaatccccctgtgctgaagagacatcagagggagatcaccaggactaccctgcagtctgatcaggaggagattgactatgatgacacaatctctgtggagatgaagaaggaggattttgacatctatgatgaggatgagaaccagagccccagatcttttcagaagaagaccagacactacttcattgctgctgtggagaggctgtgggactatggcatgagcagcagccctcatgtgctgaggaacagggcccagtctggctctgtgccccagttcaagaaggtggtgttccaggagtttactgatggcagcttcacccagcccctgtacagaggggagctgaatgagcacctgggcctgctgggcccttatatcagggctgaggtggaggataacattatggtgactttcaggaaccaggcctctaggccctacagcttctatagcagcctgatctcttatgaggaggatcagaggcagggggctgagcccagaaagaactttgtgaagcctaatgagactaagacctacttctggaaggtccagcaccacatggcccccaccaaggatgagtttgattgcaaggcctgggcctatttctctgatgtggacctggagaaggatgtccattctggcctgattggccctctgctggtgtgccacactaacactctgaatcctgcccatggcaggcaggtgactgtccaggagtttgccctgttcttcactatctttgatgagaccaagagctggtactttactgagaacatggagagaaactgcagggctccttgcaatatccagatggaggaccccaccttcaaggagaactacaggtttcatgccatcaatgggtacatcatggacaccctgcctggcctggtgatggctcaggaccagagaatcagatggtatctgctgagcatgggcagcaatgagaatatccacagcatccacttctctggacatgtgttcactgtgaggaagaaggaggagtacaagatggctctgtataatctgtaccctggagtgtttgaaactgtggagatgctgccttctaaggctggcatctggagggtggagtgcctgattggggagcacctgcatgctggcatgagcaccctgttcctggtgtacagcaacaagtgtcagacccccctgggcatggcctctggacacatcagggacttccagatcacagcctctggccagtatggccagtgggcccccaagctggccaggctgcattattctggcagcatcaatgcctggtctaccaaggagccctttagctggatcaaggtggacctgctggcccccatgattatccatggcatcaagacccagggggccaggcagaagttctctagcctgtacatcagccagttcatcatcatgtactctctggatggcaagaagtggcagacctacaggggcaacagcactggcacactgatggtgttctttggcaatgtggacagctctggcatcaagcacaacatcttcaatccccccattatcgctaggtatattaggctgcatcccacccactacagcatcagatctaccctgagaatggagctgatgggctgtgacctgaactcttgcagcatgcccctgggcatggagtctaaggccatctctgatgcccagattactgccagcagctacttcaccaatatgtttgccacctggagcccttctaaggccaggctgcatctgcaggggaggagcaatgcctggaggcctcaggtgaacaaccctaaggagtggctgcaggtggatttccagaagaccatgaaggtgactggagtgaccacccagggagtcaagagcctgctgaccagcatgtatgtgaaggagtttctgatcagctctagccaggatggccaccagtggactctgttctttcagaatgggaaggtgaaggtgtttcagggcaatcaggactctttcacccctgtggtgaacagcctggacccccccctgctgaccagatacctgagaatccacccccagagctgggtgcaccagatcgccctgaggatggaggtgctgggctgtgaggctcaggatctgtactgagatatctctagagtcgacagtactggtgatcagcctcgactgtgccttctagttgccagccatctgttgtttgcccctcccccgtgccttccttgaccctggaaggtgccactcccactgtcctttcctaataaaatgaggaaattgcatcgcattgtctgagtaggtgtcattctattctggggggtggggtggggcaggacagcaagggggaggattgggaagacaatagcaggcatgctggggatgcggtgggctctatggaaccagctggggcccg

SEQ ID NO: 50 - protein, 1496 aa, synthetic construct
ATRRYYLGAVELSWDYMQSDLGELPVDARFPPRVPKSFPFNTSVVYKKTLFVEFTDHLFNIAKPRPPWMGLLGPTIQAEVYDTVVITLKNMASHPVSLHAVGVSYWKASEGAEYDDQTSQREKEDDKVFPGGSHTYVWQVLKENGPMASDPLCLTYSYLSHVDLVKDLNSGLIGALLVCREGSLAKEKTQTLHKFILLFAVFDEGKSWHSETKNSLMQDRDAASARAWPKMHTVNGYVNRSLPGLIGCHRKSVYWHVIGMGTTPEVHSIFLEGHTFLVRNHRQASLEISPITFLTAQTLLMDLGQFLLFCHISSHQHDGMEAYVKVDSCPEEPQLRMKNNEEAEDYDDDLTDSEMDVVRFDDDNSPSFIQIRSVAKKHPKTWVHYIAAEEEDWDYAPLVLAPDDRSYKSQYLNNGPQRIGRKYKKVRFMAYTDETFKTREAIQHESGILGPLLYGEVGDTLLIIFKNQASRPYNIYPHGITDVRPLYSRRLPKGVKHLKDFPILPGEIFKYKWTVTVEDGPTKSDPRCLTRYYSSFVNMERDLASGLIGPLLICYKESVDQRGNQIMSDKRNVILFSVFDENRSWYLTENIQRFLPNPAGVQLEDPEFQASNIMHSINGYVFDSLQLSVCLHEVAYWYILSIGAQTDFLSVFFSGYTFKHKMVYEDTLTLFPFSGETVFMSMENPGLWILGCHNSDFRNRGMTALLKVSSCDKNTGDYYEDSYEDISAYLLSKNNAIEPRSFSQNSRHPSTRQKQFNATNVSNNSNTSNDSNVSNKTSNNSNATNKTNNTNDSTNRTNQTNTSPPVLKHHQREITRTTLQSDQEEIDYDDTISVEMKKEDFDIYDEDENQSPRSFQKKTRHYFIAAVERLWDYGMSSSPHVLRNRAQSGSVPQFKKVVFQEFTDGSFTQPLYRGELNEHLGLLGPYIRAEVEDNIMVTFRNQASRPYSFYSSLISYEEDQRQGAEPRKNFVKPNETKTYFWKVQHHMAPTKDEFDCKAWAYFSDVDLEKDVHSGLIGPLLVCHTNTLNPAHGRQVTVQEFALFFTIFDETKSWYFTENMERNCRAPCNIQMEDPTFKENYRFHAINGYIMDTLPGLVMAQDQRIRWYLLSMGSNENIHSIHFSGHVFTVRKKEEYKMALYNLYPGVFETVEMLPSKAGIWRVECLIGEHLHAGMSTLFLVYSNKCQTPLGMASGHIRDFQITASGQYGQWAPKLARLHYSGSINAWSTKEPFSWIKVDLLAPMIIHGIKTQGARQKFSSLYISQFIIMYSLDGKKWQTYRGNSTGTLMVFFGNVDSSGIKHNIFNPPIIARYIRLHPTHYSIRSTLRMELMGCDLNSCSMPLGMESKAISDAQITASSYFTNMFATWSPSKARLHLQGRSNAWRPQVNNPKEWLQVDFQKTMKVTGVTTQGVKSLLTSMYVKEFLISSSQDGHQWTLFFQNGKVKVFQGNQDSFTPVVNSLDPPLLTRYLRIHPQSWVHQIALRMEVLGCEAQDLY

SEQ ID NO: 51 - protein, 1496 aa, synthetic construct
ATRRYYLGAVELSWDYMQSDLGELPVDARFPPRVPKSFPFNTSVVYKKTLFVEFTDHLFNIAKPRPPWMGLLGPTIQAEVYDTVVITLKNMASHPVSLHAVGVSYWKASEGAEYDDQTSQREKEDDKVFPGGSHTYVWQVLKENGPMASDPLCLTYSYLSHVDLVKDLNSGLIGALLVCREGSLAKEKTQTLHKFILLFAVFDEGKSWHSETKNSLMQDRDAASARAWPKMHTVNGYVNRSLPGLIGCHRKSVYWHVIGMGTTPEVHSIFLEGHTFLVRNHRQASLEISPITFLTAQTLLMDLGQFLLSCHISSHQHDGMEAYVKVDSCPEEPQLRMKNNEEAEDYDDDLTDSEMDVVRFDDDNSPSFIQIRSVAKKHPKTWVHYIAAEEEDWDYAPLVLAPDDRSYKSQYLNNGPQRIGRKYKKVRFMAYTDETFKTREAIQHESGILGPLLYGEVGDTLLIIFKNQASRPYNIYPHGITDVRPLYSRRLPKGVKHLKDFPILPGEIFKYKWTVTVEDGPTKSDPRCLTRYYSSFVNMERDLASGLIGPLLICYKESVDQRGNQIMSDKRNVILFSVFDENRSWYLTENIQRFLPNPAGVQLEDPEFQASNIMHSINGYVFDSLQLSVCLHEVAYWYILSIGAQTDFLSVFFSGYTFKHKMVYEDTLTLFPFSGETVFMSMENPGLWILGCHNSDFRNRGMTALLKVSSCDKNTGDYYEDSYEDISAYLLSKNNAIEPRSFSQNSRHPSTRQKQFNATNVSNNSNTSNDSNVSNKTSNNSNATNKTNNTNDSTNRTNQTNTSPPVLKRHQREITRTTLQSDQEEIDYDDTISVEMKKEDFDIYDEDENQSPRSFQKKTRHYFIAAVERLWDYGMSSSPHVLRNRAQSGSVPQFKKVVFQEFTDGSFTQPLYRGELNEHLGLLGPYIRAEVEDNIMVTFRNQASRPYSFYSSLISYEEDQRQGAEPRKNFVKPNETKTYFWKVQHHMAPTKDEFDCKAWAYFSDVDLEKDVHSGLIGPLLVCHTNTLNPAHGRQVTVQEFALFFTIFDETKSWYFTENMERNCRAPCNIQMEDPTFKENYRFHAINGYIMDTLPGLVMAQDQRIRWYLLSMGSNENIHSIHFSGHVFTVRKKEEYKMALYNLYPGVFETVEMLPSKAGIWRVECLIGEHLHAGMSTLFLVYSNKCQTPLGMASGHIRDFQITASGQYGQWAPKLARLHYSGSINAWSTKEPFSWIKVDLLAPMIIHGIKTQGARQKFSSLYISQFIIMYSLDGKKWQTYRGNSTGTLMVFFGNVDSSGIKHNIFNPPIIARYIRLHPTHYSIRSTLRMELMGCDLNSCSMPLGMESKAISDAQITASSYFTNMFATWSPSKARLHLQGRSNAWRPQVNNPKEWLQVDFQKTMKVTGVTTQGVKSLLTSMYVKEFLISSSQDGHQWTLFFQNGKVKVFQGNQDSFTPVVNSLDPPLLTRYLRIHPQSWVHQIALRMEVLGCEAQDLY

SEQ ID NO: 52 - protein, 1496 aa, synthetic construct
ATRRYYLGAVELSWDYMQSDLGELPVDARFPPRVPKSFPFNTSVVYKKTLFVEFTDHLFNIAKPRPPWMGLLGPTIQAEVYDTVVITLKNMASHPVSLHAVGVSYWKASEGAEYDDQTSQREKEDDKVFPGGSHTYVWQVLKENGPMASDPLCLTYSYLSHVDLVKDLNSGLIGALLVCREGSLAKEKTQTLHKFILLFAVFDEGKSWHSETKNSLMQDRDAASARAWPKMHTVNGYVNRSLPGLIGCHRKSVYWHVIGMGTTPEVHSIFLEGHTFLVRNHRQASLEISPITFLTAQTLLMDLGQFLLSCHISSHQHDGMEAYVKVDSCPEEPQLRMKNNEEAEDYDDDLTDSEMDVVRFDDDNSPSFIQIRSVAKKHPKTWVHYIAAEEEDWDYAPLVLAPDDRSYKSQYLNNGPQRIGRKYKKVRFMAYTDETFKTREAIQHESGILGPLLYGEVGDTLLIIFKNQASRPYNIYPHGITDVRPLYSRRLPKGVKHLKDFPILPGEIFKYKWTVTVEDGPTKSDPRCLTRYYSSFVNMERDLASGLIGPLLICYKESVDQRGNQIMSDKRNVILFSVFDENRSWYLTENIQRFLPNPAGVQLEDPEFQASNIMHSINGYVFDSLQLSVCLHEVAYWYILSIGAQTDFLSVFFSGYTFKHKMVYEDTLTLFPFSGETVFMSMENPGLWILGCHNSDFRNRGMTALLKVSSCDKNTGDYYEDSYEDISAYLLSKNNAIEPRSFSQNSRHPSTRQKQFNATNVSNNSNTSNDSNVSNKTSNNSNATNKTNNTNDSTNRTNQTNTSPPVLKHHQREITRTTLQSDQEEIDYDDTISVEMKKEDFDIYDEDENQSPRSFQKKTRHYFIAAVERLWDYGMSSSPHVLRNRAQSGSVPQFKKVVFQEFTDGSFTQPLYRGELNEHLGLLGPYIRAEVEDNIMVTFRNQASRPYSFYSSLISYEEDQRQGAEPRKNFVKPNETKTYFWKVQHHMAPTKDEFDCKAWAYFSDVDLEKDVHSGLIGPLLVCHTNTLNPAHGRQVTVQEFALFFTIFDETKSWYFTENMERNCRAPCNIQMEDPTFKENYRFHAINGYIMDTLPGLVMAQDQRIRWYLLSMGSNENIHSIHFSGHVFTVRKKEEYKMALYNLYPGVFETVEMLPSKAGIWRVECLIGEHLHAGMSTLFLVYSNKCQTPLGMASGHIRDFQITASGQYGQWAPKLARLHYSGSINAWSTKEPFSWIKVDLLAPMIIHGIKTQGARQKFSSLYISQFIIMYSLDGKKWQTYRGNSTGTLMVFFGNVDSSGIKHNIFNPPIIARYIRLHPTHYSIRSTLRMELMGCDLNSCSMPLGMESKAISDAQITASSYFTNMFATWSPSKARLHLQGRSNAWRPQVNNPKEWLQVDFQKTMKVTGVTTQGVKSLLTSMYVKEFLISSSQDGHQWTLFFQNGKVKVFQGNQDSFTPVVNSLDPPLLTRYLRIHPQSWVHQIALRMEVLGCEAQDLY

SEQ ID NO: 53 - protein, 1498 aa, synthetic construct
ATRRYYLGAVELSWDYMQSDLGELPVDARFPPRVPKSFPFNTSVVYKKTLFVEFTDHLFNIAKPRPPWMGLLGPTIQAEVYDTVVITLKNMASHPVSLHAVGVSYWKASEGAEYDDQTSQREKEDDKVFPGGSHTYVWQVLKENGPMASDPLCLTYSYLSHVDLVKDLNSGLIGALLVCREGSLAKEKTQTLHKFILLFAVFDEGKSWHSETKNSLMQDRDAASARAWPKMHTVNGYVNRSLPGLIGCHRKSVYWHVIGMGTTPEVHSIFLEGHTFLVRNHRQASLEISPITFLTAQTLLMDLGQFLLSCHISSHQHDGMEAYVKVDSCPEEPQLRMKNNEEAEDYDDDLTDSEMDVVRFDDDNSPSFIQIRSVAKKHPKTWVHYIAAEEEDWDYAPLVLAPDDRSYKSQYLNNGPQRIGRKYKKVRFMAYTDETFKTREAIQHESGILGPLLYGEVGDTLLIIFKNQASRPYNIYPHGITDVRPLYSRRLPKGVKHLKDFPILPGEIFKYKWTVTVEDGPTKSDPRCLTRYYSSFVNMERDLASGLIGPLLICYKESVDQRGNQIMSDKRNVILFSVFDENRSWYLTENIQRFLPNPAGVQLEDPEFQASNIMHSINGYVFDSLQLSVCLHEVAYWYILSIGAQTDFLSVFFSGYTFKHKMVYEDTLTLFPFSGETVFMSMENPGLWILGCHNSDFRNRGMTALLKVSSCDKNTGDYYEDSYEDISAYLLSKNNAIEPRSFSQNSRHPSTRQKQFNATNVSNNSNTSNDSNVSNKTSNNSNATNKTNNTNDSTNRTNQTNTSQQNFVTQRSKREITRTTLQSDQEEIDYDDTISVEMKKEDFDIYDEDENQSPRSFQKKTRHYFIAAVERLWDYGMSSSPHVLRNRAQSGSVPQFKKVVFQEFTDGSFTQPLYRGELNEHLGLLGPYIRAEVEDNIMVTFRNQASRPYSFYSSLISYEEDQRQGAEPRKNFVKPNETKTYFWKVQHHMAPTKDEFDCKAWAYFSDVDLEKDVHSGLIGPLLVCHTNTLNPAHGRQVTVQEFALFFTIFDETKSWYFTENMERNCRAPCNIQMEDPTFKENYRFHAINGYIMDTLPGLVMAQDQRIRWYLLSMGSNENIHSIHFSGHVFTVRKKEEYKMALYNLYPGVFETVEMLPSKAGIWRVECLIGEHLHAGMSTLFLVYSNKCQTPLGMASGHIRDFQITASGQYGQWAPKLARLHYSGSINAWSTKEPFSWIKVDLLAPMIIHGIKTQGARQKFSSLYISQFIIMYSLDGKKWQTYRGNSTGTLMVFFGNVDSSGIKHNIFNPPIIARYIRLHPTHYSIRSTLRMELMGCDLNSCSMPLGMESKAISDAQITASSYFTNMFATWSPSKARLHLQGRSNAWRPQVNNPKEWLQVDFQKTMKVTGVTTQGVKSLLTSMYVKEFLISSSQDGHQWTLFFQNGKVKVFQGNQDSFTPVVNSLDPPLLTRYLRIHPQSWVHQIALRMEVLGCEAQDLY

SEQ ID NO: 54 - DNA, 4497 bp, synthetic construct
  source 1..4497: mol_type = other DNA
gccaccaggaggtactacctgggggctgtggagctgagctgggactacatgcagtctgacctgggggagctgcctgtggatgctaggttcccccctagagtgcccaagtccttccccttcaacacttctgtggtgtacaagaagaccctgtttgtggagttcactgaccacctgtttaacattgccaagcccaggcccccttggatgggcctgctggggcccaccatccaggctgaggtgtatgacactgtggtgatcaccctgaagaacatggccagccatcctgtgagcctgcatgctgtgggggtgagctactggaaggccagcgagggggctgagtatgatgaccagactagccagagggagaaggaggatgacaaggtgtttcctggaggcagccacacctatgtgtggcaggtgctgaaggagaatggccccatggcctctgaccccctgtgcctgacctacagctacctgagccatgtggatctggtgaaggacctgaactctggcctgattggggctctgctggtgtgtagagagggcagcctggctaaggagaagacccagaccctgcataagttcatcctgctgtttgctgtgtttgatgagggcaagagctggcactctgagaccaagaacagcctgatgcaggatagggatgctgcctctgccagggcttggcccaagatgcacactgtgaatggctatgtgaataggagcctgcctggcctgattggctgccacaggaagtctgtgtactggcatgtgattggaatgggcacaacccctgaggtccatagcatcttcctggagggccacactttcctggtgaggaaccacagacaggcctctctggagattagccccatcaccttcctgactgctcagactctgctgatggacctgggccagttcctgctgagttgccatattagctctcaccagcatgatggcatggaggcctatgtgaaggtggacagctgccctgaggagcctcagctgaggatgaagaacaatgaggaggctgaagactatgatgatgacctgactgattctgagatggatgtggtgaggtttgatgatgacaatagccccagcttcattcagatcagatctgtggccaaaaagcaccccaagacctgggtgcattacattgctgctgaagaggaggactgggactatgcccctctggtgctggcccctgatgataggagctataagagccagtacctgaacaatgggccccagaggattggcagaaagtacaagaaggtgaggttcatggcttacactgatgaaaccttcaaaaccagggaggccatccagcatgagtctggcatcctgggccctctgctgtatggagaggtgggagacaccctgctgatcatcttcaagaaccaggccagcaggccctacaacatctatcctcatggcatcactgatgtgagacctctgtacagcaggaggctgcctaagggggtgaaacacctgaaggactttcccatcctgcctggggagatcttcaagtataagtggactgtgactgtggaggatggccctaccaagtctgaccccaggtgtctgacaaggtattacagcagctttgtgaacatggagagggacctggcctctggcctgattggccctctgctgatctgctacaaggagtctgtggaccagaggggcaaccagatcatgtctgacaagaggaatgtgatcctgttctctgtgtttgatgagaataggagctggtatctgactgagaacatccagagattcctgcccaatcctgctggggtgcagctggaggaccctgagtttcaggccagcaatatcatgcacagcatcaatggctatgtgtttgacagcctgcagctgtctgtgtgcctgcatgaggtggcctactggtacatcctgagcattggagcccagactgattttctgtctgtgttcttttctggctataccttcaagcacaagatggtgtatgaggacaccctgaccctgttccccttctctggggagactgtgttcatgtctatggagaatcctgggctgtggattctgggctgccacaactctgatttcaggaacaggggcatgactgccctgctgaaggtgagcagctgtgacaagaacactggggactactatgaggatagctatgaggacatttctgcttatctgctgtctaagaataatgccattgagcccaggagcttcagccagaattctagacaccctagcaccagacagaaacagtttaatgccactaatgtgtctaacaacagcaacaccagcaatgacagcaatgtgtctaacaagacatctaacaacagcaacgccacaaacaagaccaacaacacaaatgatagcacaaaccggaccaaccagaccaataccagccagcagaacttcgtgacccagagaagtaagagagagatcaccaggactaccctgcagtctgatcaggaggagattgactatgatgacacaatctctgtggagatgaagaaggaggattttgacatctatgatgaggatgagaaccagagccccagatcttttcagaagaagaccagacactacttcattgctgctgtggagaggctgtgggactatggcatgagcagcagccctcatgtgctgaggaacagggcccagtctggctctgtgccccagttcaagaaggtggtgttccaggagtttactgatggcagcttcacccagcccctgtacagaggggagctgaatgagcacctgggcctgctgggcccttatatcagggctgaggtggaggataacattatggtgactttcaggaaccaggcctctaggccctacagcttctatagcagcctgatctcttatgaggaggatcagaggcagggggctgagcccagaaagaactttgtgaagcctaatgagactaagacctacttctggaaggtccagcaccacatggcccccaccaaggatgagtttgattgcaaggcctgggcctatttctctgatgtggacctggagaaggatgtccattctggcctgattggccctctgctggtgtgccacactaacactctgaatcctgcccatggcaggcaggtgactgtccaggagtttgccctgttcttcactatctttgatgagaccaagagctggtactttactgagaacatggagagaaactgcagggctccttgcaatatccagatggaggaccccaccttcaaggagaactacaggtttcatgccatcaatgggtacatcatggacaccctgcctggcctggtgatggctcaggaccagagaatcagatggtatctgctgagcatgggcagcaatgagaatatccacagcatccacttctctggacatgtgttcactgtgaggaagaaggaggagtacaagatggctctgtataatctgtaccctggagtgtttgaaactgtggagatgctgccttctaaggctggcatctggagggtggagtgcctgattggggagcacctgcatgctggcatgagcaccctgttcctggtgtacagcaacaagtgtcagacccccctgggcatggcctctggacacatcagggacttccagatcacagcctctggccagtatggccagtgggcccccaagctggccaggctgcattattctggcagcatcaatgcctggtctaccaaggagccctttagctggatcaaggtggacctgctggcccccatgattatccatggcatcaagacccagggggccaggcagaagttctctagcctgtacatcagccagttcatcatcatgtactctctggatggcaagaagtggcagacctacaggggcaacagcactggcacactgatggtgttctttggcaatgtggacagctctggcatcaagcacaacatcttcaatccccccattatcgctaggtatattaggctgcatcccacccactacagcatcagatctaccctgagaatggagctgatgggctgtgacctgaactcttgcagcatgcccctgggcatggagtctaaggccatctctgatgcccagattactgccagcagctacttcaccaatatgtttgccacctggagcccttctaaggccaggctgcatctgcaggggaggagcaatgcctggaggcctcaggtgaacaaccctaaggagtggctgcaggtggatttccagaagaccatgaaggtgactggagtgaccacccagggagtcaagagcctgctgaccagcatgtatgtgaaggagtttctgatcagctctagccaggatggccaccagtggactctgttctttcagaatgggaaggtgaaggtgtttcagggcaatcaggactctttcacccctgtggtgaacagcctggacccccccctgctgaccagatacctgagaatccacccccagagctgggtgcaccagatcgccctgaggatggaggtgctgggctgtgaggctcaggatctgtactga

SEQ ID NO: 55 - DNA, 5934 bp, synthetic construct
  source 1..5934: mol_type = other DNA
ccccaactggggtaacctttgggctccccgggcgcgactagtgaattcgtcaatattggccattagccatattattcattggttatatagcataaatcaatattggctattggccattgcatacgttgtatctatatcataatatgtacatttatattggctcatgtccaatatgaccgccatgttggtgtggaaagtccccaggctccccagcaggcagaagtatgcaaagcatgcatctcaattagtcagcaaccaggcattgattattgactagttattaatagtaatcaattacggggtcattagttcatagcccatatatggagttccgcgttacataacttacggtaaatggcccgcctggctgaccgcccaacgacccccgcccattgacgtcaataatgacgtatgttcccatagtaacgccaatagggactttccattgacgtcaatgggtggagtatttacggtaaactgcccacttggcagtacatcaagtgtatcatatgccaagtccgccccctattgacgtcaatgacggtaaatggcccgcctggcattatgcccagtacatgaccttacgggactttcctacttggcagtacatctacgtattagtcatcgctattaccatggtgatgcggttttggcagtacaccaatgggcgtggatagcggtttgactcacggggatttccaagtctccaccccattgacgtcaatgggagtttgttttggcaccaaaatcaacgggactttccaaaatgtcgtaataaccccgccccgttgacgcaaatgggcggtaggcgtgtacggtgggaggtctatataagcagaggtcgtttagtgaaccgtcagatcactagtagctttattgcggtagtttatcacagttaaattgctaacgcagtcagtgctcgactgatcacaggtaagtatcaaggttacaagacaggtttaaggaggccaatagaaactgggcttgtcgagacagagaagattcttgcgtttctgataggcacctattggtcttactgacatccactttgcctttctctccacaggggtaccgaagccgctagcgctaccggtgccaccatgcagattgaactgagcacctgcttcttcctgtgtctgctgagattctgcttctctgccaccaggaggtactacctgggggctgtggagctgagctgggactacatgcagtctgacctgggggagctgcctgtggatgctaggttcccccctagagtgcccaagtccttccccttcaacacttctgtggtgtacaagaagaccctgtttgtggagttcactgaccacctgtttaacattgccaagcccaggcccccttggatgggcctgctggggcccaccatccaggctgaggtgtatgacactgtggtgatcaccctgaagaacatggccagccatcctgtgagcctgcatgctgtgggggtgagctactggaaggccagcgagggggctgagtatgatgaccagactagccagagggagaaggaggatgacaaggtgtttcctggaggcagccacacctatgtgtggcaggtgctgaaggagaatggccccatggcctctgaccccctgtgcctgacctacagctacctgagccatgtggatctggtgaaggacctgaactctggcctgattggggctctgctggtgtgtagagagggcagcctggctaaggagaagacccagaccctgcataagttcatcctgctgtttgctgtgtttgatgagggcaagagctggcactctgagaccaagaacagcctgatgcaggatagggatgctgcctctgccagggcttggcccaagatgcacactgtgaatggctatgtgaataggagcctgcctggcctgattggctgccacaggaagtctgtgtactggcatgtgattggaatgggcacaacccctgaggtccatagcatcttcctggagggccacactttcctggtgaggaaccacagacaggcctctctggagattagccccatcaccttcctgactgctcagactctgctgatggacctgggccagttcctgctgagttgccatattagctctcaccagcatgatggcatggaggcctatgtgaaggtggacagctgccctgaggagcctcagctgaggatgaagaacaatgaggaggctgaagactatgatgatgacctgactgattctgagatggatgtggtgaggtttgatgatgacaatagccccagcttcattcagatcagatctgtggccaaaaagcaccccaagacctgggtgcattacattgctgctgaagaggaggactgggactatgcccctctggtgctggcccctgatgataggagctataagagccagtacctgaacaatgggccccagaggattggcagaaagtacaagaaggtgaggttcatggcttacactgatgaaaccttcaaaaccagggaggccatccagcatgagtctggcatcctgggccctctgctgtatggagaggtgggagacaccctgctgatcatcttcaagaaccaggccagcaggccctacaacatctatcctcatggcatcactgatgtgagacctctgtacagcaggaggctgcctaagggggtgaaacacctgaaggactttcccatcctgcctggggagatcttcaagtataagtggactgtgactgtggaggatggccctaccaagtctgaccccaggtgtctgacaaggtattacagcagctttgtgaacatggagagggacctggcctctggcctgattggccctctgctgatctgctacaaggagtctgtggaccagaggggcaaccagatcatgtctgacaagaggaatgtgatcctgttctctgtgtttgatgagaataggagctggtatctgactgagaacatccagagattcctgcccaatcctgctggggtgcagctggaggaccctgagtttcaggccagcaatatcatgcacagcatcaatggctatgtgtttgacagcctgcagctgtctgtgtgcctgcatgaggtggcctactggtacatcctgagcattggagcccagactgattttctgtctgtgttcttttctggctataccttcaagcacaagatggtgtatgaggacaccctgaccctgttccccttctctggggagactgtgttcatgtctatggagaatcctgggctgtggattctgggctgccacaactctgatttcaggaacaggggcatgactgccctgctgaaggtgagcagctgtgacaagaacactggggactactatgaggatagctatgaggacatttctgcttatctgctgtctaagaataatgccattgagcccaggagcttcagccagaattctagacaccctagcaccagacagaaacagtttaatgccactaatgtgtctaacaacagcaacaccagcaatgacagcaatgtgtctaacaagacatctaacaacagcaacgccacaaacaagaccaacaacacaaatgatagcacaaaccggaccaaccagaccaataccagccagcagaacttcgtgacccagagaagtaagagagagatcaccaggactaccctgcagtctgatcaggaggagattgactatgatgacacaatctctgtggagatgaagaaggaggattttgacatctatgatgaggatgagaaccagagccccagatcttttcagaagaagaccagacactacttcattgctgctgtggagaggctgtgggactatggcatgagcagcagccctcatgtgctgaggaacagggcccagtctggctctgtgccccagttcaagaaggtggtgttccaggagtttactgatggcagcttcacccagcccctgtacagaggggagctgaatgagcacctgggcctgctgggcccttatatcagggctgaggtggaggataacattatggtgactttcaggaaccaggcctctaggccctacagcttctatagcagcctgatctcttatgaggaggatcagaggcagggggctgagcccagaaagaactttgtgaagcctaatgagactaagacctacttctggaaggtccagcaccacatggcccccaccaaggatgagtttgattgcaaggcctgggcctatttctctgatgtggacctggagaaggatgtccattctggcctgattggccctctgctggtgtgccacactaacactctgaatcctgcccatggcaggcaggtgactgtccaggagtttgccctgttcttcactatctttgatgagaccaagagctggtactttactgagaacatggagagaaactgcagggctccttgcaatatccagatggaggaccccaccttcaaggagaactacaggtttcatgccatcaatgggtacatcatggacaccctgcctggcctggtgatggctcaggaccagagaatcagatggtatctgctgagcatgggcagcaatgagaatatccacagcatccacttctctggacatgtgttcactgtgaggaagaaggaggagtacaagatggctctgtataatctgtaccctggagtgtttgaaactgtggagatgctgccttctaaggctggcatctggagggtggagtgcctgattggggagcacctgcatgctggcatgagcaccctgttcctggtgtacagcaacaagtgtcagacccccctgggcatggcctctggacacatcagggacttccagatcacagcctctggccagtatggccagtgggcccccaagctggccaggctgcattattctggcagcatcaatgcctggtctaccaaggagccctttagctggatcaaggtggacctgctggcccccatgattatccatggcatcaagacccagggggccaggcagaagttctctagcctgtacatcagccagttcatcatcatgtactctctggatggcaagaagtggcagacctacaggggcaacagcactggcacactgatggtgttctttggcaatgtggacagctctggcatcaagcacaacatcttcaatccccccattatcgctaggtatattaggctgcatcccacccactacagcatcagatctaccctgagaatggagctgatgggctgtgacctgaactcttgcagcatgcccctgggcatggagtctaaggccatctctgatgcccagattactgccagcagctacttcaccaatatgtttgccacctggagcccttctaaggccaggctgcatctgcaggggaggagcaatgcctggaggcctcaggtgaacaaccctaaggagtggctgcaggtggatttccagaagaccatgaaggtgactggagtgaccacccagggagtcaagagcctgctgaccagcatgtatgtgaaggagtttctgatcagctctagccaggatggccaccagtggactctgttctttcagaatgggaaggtgaaggtgtttcagggcaatcaggactctttcacccctgtggtgaacagcctggacccccccctgctgaccagatacctgagaatccacccccagagctgggtgcaccagatcgccctgaggatggaggtgctgggctgtgaggctcaggatctgtactgagatatctctagagtcgacagtactggtgatcagcctcgactgtgccttctagttgccagccatctgttgtttgcccctcccccgtgccttccttgaccctggaaggtgccactcccactgtcctttcctaataaaatgaggaaattgcatcgcattgtctgagtaggtgtcattctattctggggggtggggtggggcaggacagcaagggggaggattgggaagacaatagcaggcatgctggggatgcggtgggctctatggaaccagctggggcccg

SEQ ID NO: 56 - DNA, 4491 bp, synthetic construct
  source 1..4491: mol_type = other DNA
gccaccaggaggtactacctgggggctgtggagctgagctgggactacatgcagtctgacctgggggagctgcctgtggatgctaggttcccccctagagtgcccaagtccttccccttcaacacttctgtggtgtacaagaagaccctgtttgtggagttcactgaccacctgtttaacattgccaagcccaggcccccttggatgggcctgctggggcccaccatccaggctgaggtgtatgacactgtggtgatcaccctgaagaacatggccagccatcctgtgagcctgcatgctgtgggggtgagctactggaaggccagcgagggggctgagtatgatgaccagactagccagagggagaaggaggatgacaaggtgtttcctggaggcagccacacctatgtgtggcaggtgctgaaggagaatggccccatggcctctgaccccctgtgcctgacctacagctacctgagccatgtggatctggtgaaggacctgaactctggcctgattggggctctgctggtgtgtagagagggcagcctggctaaggagaagacccagaccctgcataagttcatcctgctgtttgctgtgtttgatgagggcaagagctggcactctgagaccaagaacagcctgatgcaggatagggatgctgcctctgccagggcttggcccaagatgcacactgtgaatggctatgtgaataggagcctgcctggcctgattggctgccacaggaagtctgtgtactggcatgtgattggaatgggcacaacccctgaggtccatagcatcttcctggagggccacactttcctggtgaggaaccacagacaggcctctctggagattagccccatcaccttcctgactgctcagactctgctgatggacctgggccagttcctgctgttttgccatattagctctcaccagcatgatggcatggaggcctatgtgaaggtggacagctgccctgaggagcctcagctgaggatgaagaacaatgaggaggctgaagactatgatgatgacctgactgattctgagatggatgtggtgaggtttgatgatgacaatagccccagcttcattcagatcagatctgtggccaaaaagcaccccaagacctgggtgcattacattgctgctgaagaggaggactgggactatgcccctctggtgctggcccctgatgataggagctataagagccagtacctgaacaatgggccccagaggattggcagaaagtacaagaaggtgaggttcatggcttacactgatgaaaccttcaaaaccagggaggccatccagcatgagtctggcatcctgggccctctgctgtatggagaggtgggagacaccctgctgatcatcttcaagaaccaggccagcaggccctacaacatctatcctcatggcatcactgatgtgagacctctgtacagcaggaggctgcctaagggggtgaaacacctgaaggactttcccatcctgcctggggagatcttcaagtataagtggactgtgactgtggaggatggccctaccaagtctgaccccaggtgtctgacaaggtattacagcagctttgtgaacatggagagggacctggcctctggcctgattggccctctgctgatctgctacaaggagtctgtggaccagaggggcaaccagatcatgtctgacaagaggaatgtgatcctgttctctgtgtttgatgagaataggagctggtatctgactgagaacatccagagattcctgcccaatcctgctggggtgcagctggaggaccctgagtttcaggccagcaatatcatgcacagcatcaatggctatgtgtttgacagcctgcagctgtctgtgtgcctgcatgaggtggcctactggtacatcctgagcattggagcccagactgattttctgtctgtgttcttttctggctataccttcaagcacaagatggtgtatgaggacaccctgaccctgttccccttctctggggagactgtgttcatgtctatggagaatcctgggctgtggattctgggctgccacaactctgatttcaggaacaggggcatgactgccctgctgaaggtgagcagctgtgacaagaacactggggactactatgaggatagctatgaggacatttctgcttatctgctgtctaagaataatgccattgagcccaggagcttcagccagaatagcagacaccctagcaccagacagaaacagtttaatgccactaatgtgagcaacaacagcaacaccagcaatgacagcaatgtgtctaacaagacatctaacaacagcaatgccacaaacaagaccaacaacacaaatgatagcacaaacaggaccaaccagaccaataccagcccccctgtgctgaagcaccatcagagggagatcaccaggactaccctgcagtctgatcaggaggagattgactatgatgacacaatctctgtggagatgaagaaggaggattttgacatctatgatgaggatgagaaccagagccccagatcttttcagaagaagaccagacactacttcattgctgctgtggagaggctgtgggactatggcatgagcagcagccctcatgtgctgaggaacagggcccagtctggctctgtgccccagttcaagaaggtggtgttccaggagtttactgatggcagcttcacccagcccctgtacagaggggagctgaatgagcacctgggcctgctgggcccttatatcagggctgaggtggaggataacattatggtgactttcaggaaccaggcctctaggccctacagcttctatagcagcctgatctcttatgaggaggatcagaggcagggggctgagcccagaaagaactttgtgaagcctaatgagactaagacctacttctggaaggtccagcaccacatggcccccaccaaggatgagtttgattgcaaggcctgggcctatttctctgatgtggacctggagaaggatgtccattctggcctgattggccctctgctggtgtgccacactaacactctgaatcctgcccatggcaggcaggtgactgtccaggagtttgccctgttcttcactatctttgatgagaccaagagctggtactttactgagaacatggagagaaactgcagggctccttgcaatatccagatggaggaccccaccttcaaggagaactacaggtttcatgccatcaatgggtacatcatggacaccctgcctggcctggtgatggctcaggaccagagaatcagatggtatctgctgagcatgggcagcaatgagaatatccacagcatccacttctctggacatgtgttcactgtgaggaagaaggaggagtacaagatggctctgtataatctgtaccctggagtgtttgaaactgtggagatgctgccttctaaggctggcatctggagggtggagtgcctgattggggagcacctgcatgctggcatgagcaccctgttcctggtgtacagcaacaagtgtcagacccccctgggcatggcctctggacacatcagggacttccagatcacagcctctggccagtatggccagtgggcccccaagctggccaggctgcattattctggcagcatcaatgcctggtctaccaaggagccctttagctggatcaaggtggacctgctggcccccatgattatccatggcatcaagacccagggggccaggcagaagttctctagcctgtacatcagccagttcatcatcatgtactctctggatggcaagaagtggcagacctacaggggcaacagcactggcacactgatggtgttctttggcaatgtggacagctctggcatcaagcacaacatcttcaatccccccattatcgctaggtatattaggctgcatcccacccactacagcatcagatctaccctgagaatggagctgatgggctgtgacctgaactcttgcagcatgcccctgggcatggagtctaaggccatctctgatgcccagattactgccagcagctacttcaccaatatgtttgccacctggagcccttctaaggccaggctgcatctgcaggggaggagcaatgcctggaggcctcaggtgaacaaccctaaggagtggctgcaggtggatttccagaagaccatgaaggtgactggagtgaccacccagggagtcaagagcctgctgaccagcatgtatgtgaaggagtttctgatcagctctagccaggatggccaccagtggactctgttctttcagaatgggaaggtgaaggtgtttcagggcaatcaggactctttcacccctgtggtgaacagcctggacccccccctgctgaccagatacctgagaatccacccccagagctgggtgcaccagatcgccctgaggatggaggtgctgggctgtgaggctcaggatctgtactga

SEQ ID NO: 57 - DNA, 5928 bp, synthetic construct
  source 1..5928: mol_type = other DNA
ccccaactggggtaacctttgggctccccgggcgcgactagtgaattcgtcaatattggccattagccatattattcattggttatatagcataaatcaatattggctattggccattgcatacgttgtatctatatcataatatgtacatttatattggctcatgtccaatatgaccgccatgttggtgtggaaagtccccaggctccccagcaggcagaagtatgcaaagcatgcatctcaattagtcagcaaccaggcattgattattgactagttattaatagtaatcaattacggggtcattagttcatagcccatatatggagttccgcgttacataacttacggtaaatggcccgcctggctgaccgcccaacgacccccgcccattgacgtcaataatgacgtatgttcccatagtaacgccaatagggactttccattgacgtcaatgggtggagtatttacggtaaactgcccacttggcagtacatcaagtgtatcatatgccaagtccgccccctattgacgtcaatgacggtaaatggcccgcctggcattatgcccagtacatgaccttacgggactttcctacttggcagtacatctacgtattagtcatcgctattaccatggtgatgcggttttggcagtacaccaatgggcgtggatagcggtttgactcacggggatttccaagtctccaccccattgacgtcaatgggagtttgttttggcaccaaaatcaacgggactttccaaaatgtcgtaataaccccgccccgttgacgcaaatgggcggtaggcgtgtacggtgggaggtctatataagcagaggtcgtttagtgaaccgtcagatcactagtagctttattgcggtagtttatcacagttaaattgctaacgcagtcagtgctcgactgatcacaggtaagtatcaaggttacaagacaggtttaaggaggccaatagaaactgggcttgtcgagacagagaagattcttgcgtttctgataggcacctattggtcttactgacatccactttgcctttctctccacaggggtaccgaagccgctagcgctaccggtgccaccatgcagattgaactgagcacctgcttcttcctgtgtctgctgagattctgcttctctgccaccaggaggtactacctgggggctgtggagctgagctgggactacatgcagtctgacctgggggagctgcctgtggatgctaggttcccccctagagtgcccaagtccttccccttcaacacttctgtggtgtacaagaagaccctgtttgtggagttcactgaccacctgtttaacattgccaagcccaggcccccttggatgggcctgctggggcccaccatccaggctgaggtgtatgacactgtggtgatcaccctgaagaacatggccagccatcctgtgagcctgcatgctgtgggggtgagctactggaaggccagcgagggggctgagtatgatgaccagactagccagagggagaaggaggatgacaaggtgtttcctggaggcagccacacctatgtgtggcaggtgctgaaggagaatggccccatggcctctgaccccctgtgcctgacctacagctacctgagccatgtggatctggtgaaggacctgaactctggcctgattggggctctgctggtgtgtagagagggcagcctggctaaggagaagacccagaccctgcataagttcatcctgctgtttgctgtgtttgatgagggcaagagctggcactctgagaccaagaacagcctgatgcaggatagggatgctgcctctgccagggcttggcccaagatgcacactgtgaatggctatgtgaataggagcctgcctggcctgattggctgccacaggaagtctgtgtactggcatgtgattggaatgggcacaacccctgaggtccatagcatcttcctggagggccacactttcctggtgaggaaccacagacaggcctctctggagattagccccatcaccttcctgactgctcagactctgctgatggacctgggccagttcctgctgttttgccatattagctctcaccagcatgatggcatggaggcctatgtgaaggtggacagctgccctgaggagcctcagctgaggatgaagaacaatgaggaggctgaagactatgatgatgacctgactgattctgagatggatgtggtgaggtttgatgatgacaatagccccagcttcattcagatcagatctgtggccaaaaagcaccccaagacctgggtgcattacattgctgctgaagaggaggactgggactatgcccctctggtgctggcccctgatgataggagctataagagccagtacctgaacaatgggccccagaggattggcagaaagtacaagaaggtgaggttcatggcttacactgatgaaaccttcaaaaccagggaggccatccagcatgagtctggcatcctgggccctctgctgtatggagaggtgggagacaccctgctgatcatcttcaagaaccaggccagcaggccctacaacatctatcctcatggcatcactgatgtgagacctctgtacagcaggaggctgcctaagggggtgaaacacctgaaggactttcccatcctgcctggggagatcttcaagtataagtggactgtgactgtggaggatggccctaccaagtctgaccccaggtgtctgacaaggtattacagcagctttgtgaacatggagagggacctggcctctggcctgattggccctctgctgatctgctacaaggagtctgtggaccagaggggcaaccagatcatgtctgacaagaggaatgtgatcctgttctctgtgtttgatgagaataggagctggtatctgactgagaacatccagagattcctgcccaatcctgctggggtgcagctggaggaccctgagtttcaggccagcaatatcatgcacagcatcaatggctatgtgtttgacagcctgcagctgtctgtgtgcctgcatgaggtggcctactggtacatcctgagcattggagcccagactgattttctgtctgtgttcttttctggctataccttcaagcacaagatggtgtatgaggacaccctgaccctgttccccttctctggggagactgtgttcatgtctatggagaatcctgggctgtggattctgggctgccacaactctgatttcaggaacaggggcatgactgccctgctgaaggtgagcagctgtgacaagaacactggggactactatgaggatagctatgaggacatttctgcttatctgctgtctaagaataatgccattgagcccaggagcttcagccagaatagcagacaccctagcaccagacagaaacagtttaatgccactaatgtgagcaacaacagcaacaccagcaatgacagcaatgtgtctaacaagacatctaacaacagcaatgccacaaacaagaccaacaacacaaatgatagcacaaacaggaccaaccagaccaataccagcccccctgtgctgaagcaccatcagagggagatcaccaggactaccctgcagtctgatcaggaggagattgactatgatgacacaatctctgtggagatgaagaaggaggattttgacatctatgatgaggatgagaaccagagccccagatcttttcagaagaagaccagacactacttcattgctgctgtggagaggctgtgggactatggcatgagcagcagccctcatgtgctgaggaacagggcccagtctggctctgtgccccagttcaagaaggtggtgttccaggagtttactgatggcagcttcacccagcccctgtacagaggggagctgaatgagcacctgggcctgctgggcccttatatcagggctgaggtggaggataacattatggtgactttcaggaaccaggcctctaggccctacagcttctatagcagcctgatctcttatgaggaggatcagaggcagggggctgagcccagaaagaactttgtgaagcctaatgagactaagacctacttctggaaggtccagcaccacatggcccccaccaaggatgagtttgattgcaaggcctgggcctatttctctgatgtggacctggagaaggatgtccattctggcctgattggccctctgctggtgtgccacactaacactctgaatcctgcccatggcaggcaggtgactgtccaggagtttgccctgttcttcactatctttgatgagaccaagagctggtactttactgagaacatggagagaaactgcagggctccttgcaatatccagatggaggaccccaccttcaaggagaactacaggtttcatgccatcaatgggtacatcatggacaccctgcctggcctggtgatggctcaggaccagagaatcagatggtatctgctgagcatgggcagcaatgagaatatccacagcatccacttctctggacatgtgttcactgtgaggaagaaggaggagtacaagatggctctgtataatctgtaccctggagtgtttgaaactgtggagatgctgccttctaaggctggcatctggagggtggagtgcctgattggggagcacctgcatgctggcatgagcaccctgttcctggtgtacagcaacaagtgtcagacccccctgggcatggcctctggacacatcagggacttccagatcacagcctctggccagtatggccagtgggcccccaagctggccaggctgcattattctggcagcatcaatgcctggtctaccaaggagccctttagctggatcaaggtggacctgctggcccccatgattatccatggcatcaagacccagggggccaggcagaagttctctagcctgtacatcagccagttcatcatcatgtactctctggatggcaagaagtggcagacctacaggggcaacagcactggcacactgatggtgttctttggcaatgtggacagctctggcatcaagcacaacatcttcaatccccccattatcgctaggtatattaggctgcatcccacccactacagcatcagatctaccctgagaatggagctgatgggctgtgacctgaactcttgcagcatgcccctgggcatggagtctaaggccatctctgatgcccagattactgccagcagctacttcaccaatatgtttgccacctggagcccttctaaggccaggctgcatctgcaggggaggagcaatgcctggaggcctcaggtgaacaaccctaaggagtggctgcaggtggatttccagaagaccatgaaggtgactggagtgaccacccagggagtcaagagcctgctgaccagcatgtatgtgaaggagtttctgatcagctctagccaggatggccaccagtggactctgttctttcagaatgggaaggtgaaggtgtttcagggcaatcaggactctttcacccctgtggtgaacagcctggacccccccctgctgaccagatacctgagaatccacccccagagctgggtgcaccagatcgccctgaggatggaggtgctgggctgtgaggctcaggatctgtactgagatatctctagagtcgacagtactggtgatcagcctcgactgtgccttctagttgccagccatctgttgtttgcccctcccccgtgccttccttgaccctggaaggtgccactcccactgtcctttcctaataaaatgaggaaattgcatcgcattgtctgagtaggtgtcattctattctggggggtggggtggggcaggacagcaagggggaggattgggaagacaatagcaggcatgctggggatgcggtgggctctatggaaccagctggggcccg

SEQ ID NO: 58 - DNA, 4491 bp, synthetic construct
  source 1..4491: mol_type = other DNA
gccaccaggaggtactacctgggggctgtggagctgagctgggactacatgcagtctgacctgggggagctgcctgtggatgctaggttcccccctagagtgcccaagtccttccccttcaacacttctgtggtgtacaagaagaccctgtttgtggagttcactgaccacctgtttaacattgccaagcccaggcccccttggatgggcctgctggggcccaccatccaggctgaggtgtatgacactgtggtgatcaccctgaagaacatggccagccatcctgtgagcctgcatgctgtgggggtgagctactggaaggccagcgagggggctgagtatgatgaccagactagccagagggagaaggaggatgacaaggtgtttcctggaggcagccacacctatgtgtggcaggtgctgaaggagaatggccccatggcctctgaccccctgtgcctgacctacagctacctgagccatgtggatctggtgaaggacctgaactctggcctgattggggctctgctggtgtgtagagagggcagcctggctaaggagaagacccagaccctgcataagttcatcctgctgtttgctgtgtttgatgagggcaagagctggcactctgagaccaagaacagcctgatgcaggatagggatgctgcctctgccagggcttggcccaagatgcacactgtgaatggctatgtgaataggagcctgcctggcctgattggctgccacaggaagtctgtgtactggcatgtgattggaatgggcacaacccctgaggtccatagcatcttcctggagggccacactttcctggtgaggaaccacagacaggcctctctggagattagccccatcaccttcctgactgctcagactctgctgatggacctgggccagttcctgctgagttgccatattagctctcaccagcatgatggcatggaggcctatgtgaaggtggacagctgccctgaggagcctcagctgaggatgaagaacaatgaggaggctgaagactatgatgatgacctgactgattctgagatggatgtggtgaggtttgatgatgacaatagccccagcttcattcagatcagatctgtggccaaaaagcaccccaagacctgggtgcattacattgctgctgaagaggaggactgggactatgcccctctggtgctggcccctgatgataggagctataagagccagtacctgaacaatgggccccagaggattggcagaaagtacaagaaggtgaggttcatggcttacactgatgaaaccttcaaaaccagggaggccatccagcatgagtctggcatcctgggccctctgctgtatggagaggtgggagacaccctgctgatcatcttcaagaaccaggccagcaggccctacaacatctatcctcatggcatcactgatgtgagacctctgtacagcaggaggctgcctaagggggtgaaacacctgaaggactttcccatcctgcctggggagatcttcaagtataagtggactgtgactgtggaggatggccctaccaagtctgaccccaggtgtctgacaaggtattacagcagctttgtgaacatggagagggacctggcctctggcctgattggccctctgctgatctgctacaaggagtctgtggaccagaggggcaaccagatcatgtctgacaagaggaatgtgatcctgttctctgtgtttgatgagaataggagctggtatctgactgagaacatccagagattcctgcccaatcctgctggggtgcagctggaggaccctgagtttcaggccagcaatatcatgcacagcatcaatggctatgtgtttgacagcctgcagctgtctgtgtgcctgcatgaggtggcctactggtacatcctgagcattggagcccagactgattttctgtctgtgttcttttctggctataccttcaagcacaagatggtgtatgaggacaccctgaccctgttccccttctctggggagactgtgttcatgtctatggagaatcctgggctgtggattctgggctgccacaactctgatttcaggaacaggggcatgactgccctgctgaaggtgagcagctgtgacaagaacactggggactactatgaggatagctatgaggacatttctgcttatctgctgtctaagaataatgccattgagcccaggagcttcagccagaatagcagacaccctagcaccagacagaaacagtttaatgccactaatgtgagcaacaacagcaacaccagcaatgacagcaatgtgtctaacaagacatctaacaacagcaatgccacaaacaagaccaacaacacaaatgatagcacaaacaggaccaaccagaccaataccagcccccctgtgctgaagcaccatcagagggagatcaccaggactaccctgcagtctgatcaggaggagattgactatgatgacacaatctctgtggagatgaagaaggaggattttgacatctatgatgaggatgagaaccagagccccagatcttttcagaagaagaccagacactacttcattgctgctgtggagaggctgtgggactatggcatgagcagcagccctcatgtgctgaggaacagggcccagtctggctctgtgccccagttcaagaaggtggtgttccaggagtttactgatggcagcttcacccagcccctgtacagaggggagctgaatgagcacctgggcctgctgggcccttatatcagggctgaggtggaggataacattatggtgactttcaggaaccaggcctctaggccctacagcttctatagcagcctgatctcttatgaggaggatcagaggcagggggctgagcccagaaagaactttgtgaagcctaatgagactaagacctacttctggaaggtccagcaccacatggcccccaccaaggatgagtttgattgcaaggcctgggcctatttctctgatgtggacctggagaaggatgtccattctggcctgattggccctctgctggtgtgccacactaacactctgaatcctgcccatggcaggcaggtgactgtccaggagtttgccctgttcttcactatctttgatgagaccaagagctggtactttactgagaacatggagagaaactgcagggctccttgcaatatccagatggaggaccccaccttcaaggagaactacaggtttcatgccatcaatgggtacatcatggacaccctgcctggcctggtgatggctcaggaccagagaatcagatggtatctgctgagcatgggcagcaatgagaatatccacagcatccacttctctggacatgtgttcactgtgaggaagaaggaggagtacaagatggctctgtataatctgtaccctggagtgtttgaaactgtggagatgctgccttctaaggctggcatctggagggtggagtgcctgattggggagcacctgcatgctggcatgagcaccctgttcctggtgtacagcaacaagtgtcagacccccctgggcatggcctctggacacatcagggacttccagatcacagcctctggccagtatggccagtgggcccccaagctggccaggctgcattattctggcagcatcaatgcctggtctaccaaggagccctttagctggatcaaggtggacctgctggcccccatgattatccatggcatcaagacccagggggccaggcagaagttctctagcctgtacatcagccagttcatcatcatgtactctctggatggcaagaagtggcagacctacaggggcaacagcactggcacactgatggtgttctttggcaatgtggacagctctggcatcaagcacaacatcttcaatccccccattatcgctaggtatattaggctgcatcccacccactacagcatcagatctaccctgagaatggagctgatgggctgtgacctgaactcttgcagcatgcccctgggcatggagtctaaggccatctctgatgcccagattactgccagcagctacttcaccaatatgtttgccacctggagcccttctaaggccaggctgcatctgcaggggaggagcaatgcctggaggcctcaggtgaacaaccctaaggagtggctgcaggtggatttccagaagaccatgaaggtgactggagtgaccacccagggagtcaagagcctgctgaccagcatgtatgtgaaggagtttctgatcagctctagccaggatggccaccagtggactctgttctttcagaatgggaaggtgaaggtgtttcagggcaatcaggactctttcacccctgtggtgaacagcctggacccccccctgctgaccagatacctgagaatccacccccagagctgggtgcaccagatcgccctgaggatggaggtgctgggctgtgaggctcaggatctgtactga

SEQ ID NO: 59 - DNA, 5928 bp, synthetic construct
  source 1..5928: mol_type = other DNA
ccccaactggggtaacctttgggctccccgggcgcgactagtgaattcgtcaatattggccattagccatattattcattggttatatagcataaatcaatattggctattggccattgcatacgttgtatctatatcataatatgtacatttatattggctcatgtccaatatgaccgccatgttggtgtggaaagtccccaggctccccagcaggcagaagtatgcaaagcatgcatctcaattagtcagcaaccaggcattgattattgactagttattaatagtaatcaattacggggtcattagttcatagcccatatatggagttccgcgttacataacttacggtaaatggcccgcctggctgaccgcccaacgacccccgcccattgacgtcaataatgacgtatgttcccatagtaacgccaatagggactttccattgacgtcaatgggtggagtatttacggtaaactgcccacttggcagtacatcaagtgtatcatatgccaagtccgccccctattgacgtcaatgacggtaaatggcccgcctggcattatgcccagtacatgaccttacgggactttcctacttggcagtacatctacgtattagtcatcgctattaccatggtgatgcggttttggcagtacaccaatgggcgtggatagcggtttgactcacggggatttccaagtctccaccccattgacgtcaatgggagtttgttttggcaccaaaatcaacgggactttccaaaatgtcgtaataaccccgccccgttgacgcaaatgggcggtaggcgtgtacggtgggaggtctatataagcagaggtcgtttagtgaaccgtcagatcactagtagctttattgcggtagtttatcacagttaaattgctaacgcagtcagtgctcgactgatcacaggtaagtatcaaggttacaagacaggtttaaggaggccaatagaaactgggcttgtcgagacagagaagattcttgcgtttctgataggcacctattggtcttactgacatccactttgcctttctctccacaggggtaccgaagccgctagcgctaccggtgccaccatgcagattgaactgagcacctgcttcttcctgtgtctgctgagattctgcttctctgccaccaggaggtactacctgggggctgtggagctgagctgggactacatgcagtctgacctgggggagctgcctgtggatgctaggttcccccctagagtgcccaagtccttccccttcaacacttctgtggtgtacaagaagaccctgtttgtggagttcactgaccacctgtttaacattgccaagcccaggcccccttggatgggcctgctggggcccaccatccaggctgaggtgtatgacactgtggtgatcaccctgaagaacatggccagccatcctgtgagcctgcatgctgtgggggtgagctactggaaggccagcgagggggctgagtatgatgaccagactagccagagggagaaggaggatgacaaggtgtttcctggaggcagccacacctatgtgtggcaggtgctgaaggagaatggccccatggcctctgaccccctgtgcctgacctacagctacctgagccatgtggatctggtgaaggacctgaactctggcctgattggggctctgctggtgtgtagagagggcagcctggctaaggagaagacccagaccctgcataagttcatcctgctgtttgctgtgtttgatgagggcaagagctggcactctgagaccaagaacagcctgatgcaggatagggatgctgcctctgccagggcttggcccaagatgcacactgtgaatggctatgtgaataggagcctgcctggcctgattggctgccacaggaagtctgtgtactggcatgtgattggaatgggcacaacccctgaggtccatagcatcttcctggagggccacactttcctggtgaggaaccacagacaggcctctctggagattagccccatcaccttcctgactgctcagactctgctgatggacctgggccagttcctgctgagttgccatattagctctcaccagcatgatggcatggaggcctatgtgaaggtggacagctgccctgaggagcctcagctgaggatgaagaacaatgaggaggctgaagactatgatgatgacctgactgattctgagatggatgtggtgaggtttgatgatgacaatagccccagcttcattcagatcagatctgtggccaaaaagcaccccaagacctgggtgcattacattgctgctgaagaggaggactgggactatgcccctctggtgctggcccctgatgataggagctataagagccagtacctgaacaatgggccccagaggattggcagaaagtacaagaaggtgaggttcatggcttacactgatgaaaccttcaaaaccagggaggccatccagcatgagtctggcatcctgggccctctgctgtatggagaggtgggagacaccctgctgatcatcttcaagaaccaggccagcaggccctacaacatctatcctcatggcatcactgatgtgagacctctgtacagcaggaggctgcctaagggggtgaaacacctgaaggactttcccatcctgcctggggagatcttcaagtataagtggactgtgactgtggaggatggccctaccaagtctgaccccaggtgtctgacaaggtattacagcagctttgtgaacatggagagggacctggcctctggcctgattggccctctgctgatctgctacaaggagtctgtggaccagaggggcaaccagatcatgtctgacaagaggaatgtgatcctgttctctgtgtttgatgagaataggagctggtatctgactgagaacatccagagattcctgcccaatcctgctggggtgcagctggaggaccctgagtttcaggccagcaatatcatgcacagcatcaatggctatgtgtttgacagcctgcagctgtctgtgtgcctgcatgaggtggcctactggtacatcctgagcattggagcccagactgattttctgtctgtgttcttttctggctataccttcaagcacaagatggtgtatgaggacaccctgaccctgttccccttctctggggagactgtgttcatgtctatggagaatcctgggctgtggattctgggctgccacaactctgatttcaggaacaggggcatgactgccctgctgaaggtgagcagctgtgacaagaacactggggactactatgaggatagctatgaggacatttctgcttatctgctgtctaagaataatgccattgagcccaggagcttcagccagaatagcagacaccctagcaccagacagaaacagtttaatgccactaatgtgagcaacaacagcaacaccagcaatgacagcaatgtgtctaacaagacatctaacaacagcaatgccacaaacaagaccaacaacacaaatgatagcacaaacaggaccaaccagaccaataccagcccccctgtgctgaagcaccatcagagggagatcaccaggactaccctgcagtctgatcaggaggagattgactatgatgacacaatctctgtggagatgaagaaggaggattttgacatctatgatgaggatgagaaccagagccccagatcttttcagaagaagaccagacactacttcattgctgctgtggagaggctgtgggactatggcatgagcagcagccctcatgtgctgaggaacagggcccagtctggctctgtgccccagttcaagaaggtggtgttccaggagtttactgatggcagcttcacccagcccctgtacagaggggagctgaatgagcacctgggcctgctgggcccttatatcagggctgaggtggaggataacattatggtgactttcaggaaccaggcctctaggccctacagcttctatagcagcctgatctcttatgaggaggatcagaggcagggggctgagcccagaaagaactttgtgaagcctaatgagactaagacctacttctggaaggtccagcaccacatggcccccaccaaggatgagtttgattgcaaggcctgggcctatttctctgatgtggacctggagaaggatgtccattctggcctgattggccctctgctggtgtgccacactaacactctgaatcctgcccatggcaggcaggtgactgtccaggagtttgccctgttcttcactatctttgatgagaccaagagctggtactttactgagaacatggagagaaactgcagggctccttgcaatatccagatggaggaccccaccttcaaggagaactacaggtttcatgccatcaatgggtacatcatggacaccctgcctggcctggtgatggctcaggaccagagaatcagatggtatctgctgagcatgggcagcaatgagaatatccacagcatccacttctctggacatgtgttcactgtgaggaagaaggaggagtacaagatggctctgtataatctgtaccctggagtgtttgaaactgtggagatgctgccttctaaggctggcatctggagggtggagtgcctgattggggagcacctgcatgctggcatgagcaccctgttcctggtgtacagcaacaagtgtcagacccccctgggcatggcctctggacacatcagggacttccagatcacagcctctggccagtatggccagtgggcccccaagctggccaggctgcattattctggcagcatcaatgcctggtctaccaaggagccctttagctggatcaaggtggacctgctggcccccatgattatccatggcatcaagacccagggggccaggcagaagttctctagcctgtacatcagccagttcatcatcatgtactctctggatggcaagaagtggcagacctacaggggcaacagcactggcacactgatggtgttctttggcaatgtggacagctctggcatcaagcacaacatcttcaatccccccattatcgctaggtatattaggctgcatcccacccactacagcatcagatctaccctgagaatggagctgatgggctgtgacctgaactcttgcagcatgcccctgggcatggagtctaaggccatctctgatgcccagattactgccagcagctacttcaccaatatgtttgccacctggagcccttctaaggccaggctgcatctgcaggggaggagcaatgcctggaggcctcaggtgaacaaccctaaggagtggctgcaggtggatttccagaagaccatgaaggtgactggagtgaccacccagggagtcaagagcctgctgaccagcatgtatgtgaaggagtttctgatcagctctagccaggatggccaccagtggactctgttctttcagaatgggaaggtgaaggtgtttcagggcaatcaggactctttcacccctgtggtgaacagcctggacccccccctgctgaccagatacctgagaatccacccccagagctgggtgcaccagatcgccctgaggatggaggtgctgggctgtgaggctcaggatctgtactgagatatctctagagtcgacagtactggtgatcagcctcgactgtgccttctagttgccagccatctgttgtttgcccctcccccgtgccttccttgaccctggaaggtgccactcccactgtcctttcctaataaaatgaggaaattgcatcgcattgtctgagtaggtgtcattctattctggggggtggggtggggcaggacagcaagggggaggattgggaagacaatagcaggcatgctggggatgcggtgggctctatggaaccagctggggcccg

SEQ ID NO: 60 - DNA, 4491 bp, synthetic construct
  source 1..4491: mol_type = other DNA
gccaccaggaggtactacctgggggctgtggagctgagctgggactacatgcagtctgacctgggggagctgcctgtggatgctaggttcccccctagagtgcccaagtccttccccttcaacacttctgtggtgtacaagaagaccctgtttgtggagttcactgaccacctgtttaacattgccaagcccaggcccccttggatgggcctgctggggcccaccatccaggctgaggtgtatgacactgtggtgatcaccctgaagaacatggccagccatcctgtgagcctgcatgctgtgggggtgagctactggaaggccagcgagggggctgagtatgatgaccagactagccagagggagaaggaggatgacaaggtgtttcctggaggcagccacacctatgtgtggcaggtgctgaaggagaatggccccatggcctctgaccccctgtgcctgacctacagctacctgagccatgtggatctggtgaaggacctgaactctggcctgattggggctctgctggtgtgtagagagggcagcctggctaaggagaagacccagaccctgcataagttcatcctgctgtttgctgtgtttgatgagggcaagagctggcactctgagaccaagaacagcctgatgcaggatagggatgctgcctctgccagggcttggcccaagatgcacactgtgaatggctatgtgaataggagcctgcctggcctgattggctgccacaggaagtctgtgtactggcatgtgattggaatgggcacaacccctgaggtccatagcatcttcctggagggccacactttcctggtgaggaaccacagacaggcctctctggagattagccccatcaccttcctgactgctcagactctgctgatggacctgggccagttcctgctgagttgccatattagctctcaccagcatgatggcatggaggcctatgtgaaggtggacagctgccctgaggagcctcagctgaggatgaagaacaatgaggaggctgaagactatgatgatgacctgactgattctgagatggatgtggtgaggtttgatgatgacaatagccccagcttcattcagatcagatctgtggccaaaaagcaccccaagacctgggtgcattacattgctgctgaagaggaggactgggactatgcccctctggtgctggcccctgatgataggagctataagagccagtacctgaacaatgggccccagaggattggcagaaagtacaagaaggtgaggttcatggcttacactgatgaaaccttcaaaaccagggaggccatccagcatgagtctggcatcctgggccctctgctgtatggagaggtgggagacaccctgctgatcatcttcaagaaccaggccagcaggccctacaacatctatcctcatggcatcactgatgtgagacctctgtacagcaggaggctgcctaagggggtgaaacacctgaaggactttcccatcctgcctggggagatcttcaagtataagtggactgtgactgtggaggatggccctaccaagtctgaccccaggtgtctgacaaggtattacagcagctttgtgaacatggagagggacctggcctctggcctgattggccctctgctgatctgctacaaggagtctgtggaccagaggggcaaccagatcatgtctgacaagaggaatgtgatcctgttctctgtgtttgatgagaataggagctggtatctgactgagaacatccagagattcctgcccaatcctgctggggtgcagctggaggaccctgagtttcaggccagcaatatcatgcacagcatcaatggctatgtgtttgacagcctgcagctgtctgtgtgcctgcatgaggtggcctactggtacatcctgagcattggagcccagactgattttctgtctgtgttcttttctggctataccttcaagcacaagatggtgtatgaggacaccctgaccctgttccccttctctggggagactgtgttcatgtctatggagaatcctgggctgtggattctgggctgccacaactctgatttcaggaacaggggcatgactgccctgctgaaggtgagcagctgtgacaagaacactggggactactatgaggatagctatgaggacatttctgcttatctgctgtctaagaataatgccattgagcccaggagcttcagccagaatagcagacaccctagcaccagacagaaacagtttaatgccactaatgtgagcaacaacagcaacaccagcaatgacagcaatgtgtctaacaagacatctaacaacagcaatgccacaaacaagaccaacaacacaaatgatagcacaaacaggaccaaccagaccaataccagcccccctgtgctgaagagacatcagagggagatcaccaggactaccctgcagtctgatcaggaggagattgactatgatgacacaatctctgtggagatgaagaaggaggattttgacatctatgatgaggatgagaaccagagccccagatcttttcagaagaagaccagacactacttcattgctgctgtggagaggctgtgggactatggcatgagcagcagccctcatgtgctgaggaacagggcccagtctggctctgtgccccagttcaagaaggtggtgttccaggagtttactgatggcagcttcacccagcccctgtacagaggggagctgaatgagcacctgggcctgctgggcccttatatcagggctgaggtggaggataacattatggtgactttcaggaaccaggcctctaggccctacagcttctatagcagcctgatctcttatgaggaggatcagaggcagggggctgagcccagaaagaactttgtgaagcctaatgagactaagacctacttctggaaggtccagcaccacatggcccccaccaaggatgagtttgattgcaaggcctgggcctatttctctgatgtggacctggagaaggatgtccattctggcctgattggccctctgctggtgtgccacactaacactctgaatcctgcccatggcaggcaggtgactgtccaggagtttgccctgttcttcactatctttgatgagaccaagagctggtactttactgagaacatggagagaaactgcagggctccttgcaatatccagatggaggaccccaccttcaaggagaactacaggtttcatgccatcaatgggtacatcatggacaccctgcctggcctggtgatggctcaggaccagagaatcagatggtatctgctgagcatgggcagcaatgagaatatccacagcatccacttctctggacatgtgttcactgtgaggaagaaggaggagtacaagatggctctgtataatctgtaccctggagtgtttgaaactgtggagatgctgccttctaaggctggcatctggagggtggagtgcctgattggggagcacctgcatgctggcatgagcaccctgttcctggtgtacagcaacaagtgtcagacccccctgggcatggcctctggacacatcagggacttccagatcacagcctctggccagtatggccagtgggcccccaagctggccaggctgcattattctggcagcatcaatgcctggtctaccaaggagccctttagctggatcaaggtggacctgctggcccccatgattatccatggcatcaagacccagggggccaggcagaagttctctagcctgtacatcagccagttcatcatcatgtactctctggatggcaagaagtggcagacctacaggggcaacagcactggcacactgatggtgttctttggcaatgtggacagctctggcatcaagcacaacatcttcaatccccccattatcgctaggtatattaggctgcatcccacccactacagcatcagatctaccctgagaatggagctgatgggctgtgacctgaactcttgcagcatgcccctgggcatggagtctaaggccatctctgatgcccagattactgccagcagctacttcaccaatatgtttgccacctggagcccttctaaggccaggctgcatctgcaggggaggagcaatgcctggaggcctcaggtgaacaaccctaaggagtggctgcaggtggatttccagaagaccatgaaggtgactggagtgaccacccagggagtcaagagcctgctgaccagcatgtatgtgaaggagtttctgatcagctctagccaggatggccaccagtggactctgttctttcagaatgggaaggtgaaggtgtttcagggcaatcaggactctttcacccctgtggtgaacagcctggacccccccctgctgaccagatacctgagaatccacccccagagctgggtgcaccagatcgccctgaggatggaggtgctgggctgtgaggctcaggatctgtactga

SEQ ID NO: 61 - DNA, 5928 bp, synthetic construct
  source 1..5928: mol_type = other DNA
ccccaactggggtaacctttgggctccccgggcgcgactagtgaattcgtcaatattggccattagccatattattcattggttatatagcataaatcaatattggctattggccattgcatacgttgtatctatatcataatatgtacatttatattggctcatgtccaatatgaccgccatgttggtgtggaaagtccccaggctccccagcaggcagaagtatgcaaagcatgcatctcaattagtcagcaaccaggcattgattattgactagttattaatagtaatcaattacggggtcattagttcatagcccatatatggagttccgcgttacataacttacggtaaatggcccgcctggctgaccgcccaacgacccccgcccattgacgtcaataatgacgtatgttcccatagtaacgccaatagggactttccattgacgtcaatgggtggagtatttacggtaaactgcccacttggcagtacatcaagtgtatcatatgccaagtccgccccctattgacgtcaatgacggtaaatggcccgcctggcattatgcccagtacatgaccttacgggactttcctacttggcagtacatctacgtattagtcatcgctattaccatggtgatgcggttttggcagtacaccaatgggcgtggatagcggtttgactcacggggatttccaagtctccaccccattgacgtcaatgggagtttgttttggcaccaaaatcaacgggactttccaaaatgtcgtaataaccccgccccgttgacgcaaatgggcggtaggcgtgtacggtgggaggtctatataagcagaggtcgtttagtgaaccgtcagatcactagtagctttattgcggtagtttatcacagttaaattgctaacgcagtcagtgctcgactgatcacaggtaagtatcaaggttacaagacaggtttaaggaggccaatagaaactgggcttgtcgagacagagaagattcttgcgtttctgataggcacctattggtcttactgacatccactttgcctttctctccacaggggtaccgaagccgctagcgctaccggtgccaccatgcagattgaactgagcacctgcttcttcctgtgtctgctgagattctgcttctctgccaccaggaggtactacctgggggctgtggagctgagctgggactacatgcagtctgacctgggggagctgcctgtggatgctaggttcccccctagagtgcccaagtccttccccttcaacacttctgtggtgtacaagaagaccctgtttgtggagttcactgaccacctgtttaacattgccaagcccaggcccccttggatgggcctgctggggcccaccatccaggctgaggtgtatgacactgtggtgatcaccctgaagaacatggccagccatcctgtgagcctgcatgctgtgggggtgagctactggaaggccagcgagggggctgagtatgatgaccagactagccagagggagaaggaggatgacaaggtgtttcctggaggcagccacacctatgtgtggcaggtgctgaaggagaatggccccatggcctctgaccccctgtgcctgacctacagctacctgagccatgtggatctggtgaaggacctgaactctggcctgattggggctctgctggtgtgtagagagggcagcctggctaaggagaagacccagaccctgcataagttcatcctgctgtttgctgtgtttgatgagggcaagagctggcactctgagaccaagaacagcctgatgcaggatagggatgctgcctctgccagggcttggcccaagatgcacactgtgaatggctatgtgaataggagcctgcctggcctgattggctgccacaggaagtctgtgtactggcatgtgattggaatgggcacaacccctgaggtccatagcatcttcctggagggccacactttcctggtgaggaaccacagacaggcctctctggagattagccccatcaccttcctgactgctcagactctgctgatggacctgggccagttcctgctgagttgccatattagctctcaccagcatgatggcatggaggcctatgtgaaggtggacagctgccctgaggagcctcagctgaggatgaagaacaatgaggaggctgaagactatgatgatgacctgactgattctgagatggatgtggtgaggtttgatgatgacaatagccccagcttcattcagatcagatctgtggccaaaaagcaccccaagacctgggtgcattacattgctgctgaagaggaggactgggactatgcccctctggtgctggcccctgatgataggagctataagagccagtacctgaacaatgggccccagaggattggcagaaagtacaagaaggtgaggttcatggcttacactgatgaaaccttcaaaaccagggaggccatccagcatgagtctggcatcctgggccctctgctgtatggagaggtgggagacaccctgctgatcatcttcaagaaccaggccagcaggccctacaacatctatcctcatggcatcactgatgtgagacctctgtacagcaggaggctgcctaagggggtgaaacacctgaaggactttcccatcctgcctggggagatcttcaagtataagtggactgtgactgtggaggatggccctaccaagtctgaccccaggtgtctgacaaggtattacagcagctttgtgaacatggagagggacctggcctctggcctgattggccctctgctgatctgctacaaggagtctgtggaccagaggggcaaccagatcatgtctgacaagaggaatgtgatcctgttctctgtgtttgatgagaataggagctggtatctgactgagaacatccagagattcctgcccaatcctgctggggtgcagctggaggaccctgagtttcaggccagcaatatcatgcacagcatcaatggctatgtgtttgacagcctgcagctgtctgtgtgcctgcatgaggtggcctactggtacatcctgagcattggagcccagactgattttctgtctgtgttcttttctggctataccttcaagcacaagatggtgtatgaggacaccctgaccctgttccccttctctggggagactgtgttcatgtctatggagaatcctgggctgtggattctgggctgccacaactctgatttcaggaacaggggcatgactgccctgctgaaggtgagcagctgtgacaagaacactggggactactatgaggatagctatgaggacatttctgcttatctgctgtctaagaataatgccattgagcccaggagcttcagccagaatagcagacaccctagcaccagacagaaacagtttaatgccactaatgtgagcaacaacagcaacaccagcaatgacagcaatgtgtctaacaagacatctaacaacagcaatgccacaaacaagaccaacaacacaaatgatagcacaaacaggaccaaccagaccaataccagcccccctgtgctgaagagacatcagagggagatcaccaggactaccctgcagtctgatcaggaggagattgactatgatgacacaatctctgtggagatgaagaaggaggattttgacatctatgatgaggatgagaaccagagccccagatcttttcagaagaagaccagacactacttcattgctgctgtggagaggctgtgggactatggcatgagcagcagccctcatgtgctgaggaacagggcccagtctggctctgtgccccagttcaagaaggtggtgttccaggagtttactgatggcagcttcacccagcccctgtacagaggggagctgaatgagcacctgggcctgctgggcccttatatcagggctgaggtggaggataacattatggtgactttcaggaaccaggcctctaggccctacagcttctatagcagcctgatctcttatgaggaggatcagaggcagggggctgagcccagaaagaactttgtgaagcctaatgagactaagacctacttctggaaggtccagcaccacatggcccccaccaaggatgagtttgattgcaaggcctgggcctatttctctgatgtggacctggagaaggatgtccattctggcctgattggccctctgctggtgtgccacactaacactctgaatcctgcccatggcaggcaggtgactgtccaggagtttgccctgttcttcactatctttgatgagaccaagagctggtactttactgagaacatggagagaaactgcagggctccttgcaatatccagatggaggaccccaccttcaaggagaactacaggtttcatgccatcaatgggtacatcatggacaccctgcctggcctggtgatggctcaggaccagagaatcagatggtatctgctgagcatgggcagcaatgagaatatccacagcatccacttctctggacatgtgttcactgtgaggaagaaggaggagtacaagatggctctgtataatctgtaccctggagtgtttgaaactgtggagatgctgccttctaaggctggcatctggagggtggagtgcctgattggggagcacctgcatgctggcatgagcaccctgttcctggtgtacagcaacaagtgtcagacccccctgggcatggcctctggacacatcagggacttccagatcacagcctctggccagtatggccagtgggcccccaagctggccaggctgcattattctggcagcatcaatgcctggtctaccaaggagccctttagctggatcaaggtggacctgctggcccccatgattatccatggcatcaagacccagggggccaggcagaagttctctagcctgtacatcagccagttcatcatcatgtactctctggatggcaagaagtggcagacctacaggggcaacagcactggcacactgatggtgttctttggcaatgtggacagctctggcatcaagcacaacatcttcaatccccccattatcgctaggtatattaggctgcatcccacccactacagcatcagatctaccctgagaatggagctgatgggctgtgacctgaactcttgcagcatgcccctgggcatggagtctaaggccatctctgatgcccagattactgccagcagctacttcaccaatatgtttgccacctggagcccttctaaggccaggctgcatctgcaggggaggagcaatgcctggaggcctcaggtgaacaaccctaaggagtggctgcaggtggatttccagaagaccatgaaggtgactggagtgaccacccagggagtcaagagcctgctgaccagcatgtatgtgaaggagtttctgatcagctctagccaggatggccaccagtggactctgttctttcagaatgggaaggtgaaggtgtttcagggcaatcaggactctttcacccctgtggtgaacagcctggacccccccctgctgaccagatacctgagaatccacccccagagctgggtgcaccagatcgccctgaggatggaggtgctgggctgtgaggctcaggatctgtactgagatatctctagagtcgacagtactggtgatcagcctcgactgtgccttctagttgccagccatctgttgtttgcccctcccccgtgccttccttgaccctggaaggtgccactcccactgtcctttcctaataaaatgaggaaattgcatcgcattgtctgagtaggtgtcattctattctggggggtggggtggggcaggacagcaagggggaggattgggaagacaatagcaggcatgctggggatgcggtgggctctatggaaccagctggggcccg

SEQ ID NO: 62 - protein, 14 aa, synthetic construct
SFSQNPPVLKRHQR